European Patent Specification EP 4 320 276 B1, published April 23, 2025. Title: METHODS FOR DISEASE DETECTION. Applicant: UNIVERSAL DIAGNOSTICS, S.L. The sequence listing filed with the application follows.

SEQUENCE LISTING (469 sequences)

SEQ ID NO: 1 - DNA, 181 bp, Homo sapiens
acgggggggctgttcaccaggaaggggcagggctgcagcctcagcctcccctccagatgccggcagcaccagcctctgcctgcatggggccgcgaggtttgcagtgacatcccccgagcttcctgacctgccccggacacggagcacggctcccaggggccgcacaggcacccgctggcct

SEQ ID NO: 2 - DNA, 181 bp, Homo sapiens
tggaggcgtggggaccccatctccaaatacagccacattgggggttagggctccccacgtgaatttaggggacacttcagttcgtcccggcggggactggggacgccgggctgtgtgctgtgtcctgtgggagagtttgttcaccctgctggaggctccctgatgagccctggcgtctgct

SEQ ID NO: 3 - DNA, 481 bp, Homo sapiens
gcaattagggatccttggggggcttgggctggtaattaaggtgatgtataattagagtttcaacaaaaattatccgggattaaaaatcttttgaataatttcgtttaaaattttcaaatagcgttaaatacaatttatcaggttttgaatcaaacccgtgtaacgagtcttggaagctgcagctcccgtcgccggcgcgggaggaccaggagcagctccggcgacttccccgtgcgggaaggaaacttcgcgagcgaagccagctggctggggcctcgccgcggtgcagcggcggccgcgggctcagaatcgagccaccgagggctgcagacggcgtgggccgggtcggggagcggggcctgggggaccccgggccggccggtagtctcggccgacttcccactccccgcgcacaaagtcgcggccaactaccgcggagcagcgcccgcgtccacaccgcgcagcctggcgccccgaccct

SEQ ID NO: 4 - DNA, 481 bp, Homo sapiens
gcaaccaaaaggagacattttgacatggagacatatacagggaatatgccctgtgaacatgaagatggccatatgcaagcccaggagagaagcctggaagagaccgtttcctcacagcgctcagaaggaaagaaccctgccaacatcttgctttcagatgcccccaggattgtcagacaataagatctgttattgacgccaccgggttggtgatacttaggtacagcagccctagcaaacgaatacacccccatgagaactaagctccctgagagcggtaagctgccttgtcttgctcacagctgacaagaacacgcctgtacggtcacttagcacctagtactgccatttaaccgtttcactagtatgtatgaaccggagagcctgtcaagggaagagctgaatcttttatcttttgtaacgactacccagtgaaagaaaccgcgggtatgcaataaaaacctgttgaatcgattaaacc

SEQ ID NO: 5 - DNA, 241 bp, Homo sapiens
cgggaggggcggagccgacgggatgcgcgccaggccccgcccctcctccgggcccgcccccggcctggccattggccgcagagctcgggggcgtggtcgagctggggctgggggcgcccgcggtgcccgcccgcgagtctcgctgcctccctcccggggctgcgggcccggcggccgggctggctgggccgcgcttgggttcccgcgccggctcccgcacccgcaatggggaactcacacc

SEQ ID NO: 6 - DNA, 181 bp, Homo sapiens
ccacgtcggcctgcgtaaagcccagcttgatgcgccgctgcttgaactgcttggcgaactgctccaggtcgtccgagctgggcgcatcctcgtccgagtgctcgcccaccgatgagccgccgccgcccgcgcccgggtgcaggtgcgccgccgccgcgtgcaggccgcccgcgtgtgcatg

SEQ ID NO: 7 - DNA, 703 bp, Homo sapiens
tgcgcaccttgacggctccttagggacagaccagccgcaggcaagaggggcaggtgggcaggattcatcccgagtttccaatatatttaatctctaaacctgataagtacaatgcgcgcatagtctaatttttttccattttgtccctttttttgcttgttttgaatgtttttcacgttaataccgaggtcacctacagattacaattaataacttagaattccattttataacattatacactggcttgtatatatatatgtatagattatatatagatttatacatatataaaaacacactgcaccaaggaaacccatgcttatcggcataagcaacaaagagagcgacaaataccgcaacgaggaaagtgcaccttaaaacttgtttcctttttttttttttacaattgtatcgatatatatgtgtgtcccaaagactcagtgccaagagatttatacatcctaaatttatatttgttagagcgaatatttaaattttttaaaagtgagggctggggagacacagaaaagactctcggattatcctgccatccactgagagccggatgagcacagctaaggagccgcaggagcctgcgctgctgtcgcagcctctgaattctcatgaattcccagccttttggaaagggggccgggtgaggctggaagagggatccggaggtaggagatgaggacccagg

SEQ ID NO: 8 - DNA, 361 bp, Homo sapiens
aaccaccaccttggatttcagatcgaggaaaggaagccaaagcaaaggtgtggttacacaggacatccatagacaaatcgttgcctctctaagtgggcctgagctttgcggctccagaagcgcgaggcgcggttggtgcggacgcgggggcgtgggagtcatcgctctccccgcagccctggccgagctctctgctgtcctcccgagtttgggccagagaccacggctcactccctaacgccctcgcaaggacggctgcccgtcgggccaagggcgccccgggctggaggccggagcaagacggccccgcgggactcgggagccttggtaaggcggaggctcagaccccgttcacgaaaac

SEQ ID NO: 9 - DNA, 426 bp, Homo sapiens
cttgacgaccgcagcaagatggagacgctgccaggcttgctgcagcggcccgaccccggggcgcttagcgcagcgcagctggagcagctgcgaaaattcaaggtgggtgcgcccgcgcccccatccagcgtccaccaaagtgtagctgccccaggactggggccccagactgggaagagagccgccgagagaaggggagcgggagcctgttccctgataaagtggggagggcgcaggggagacccccggcggacctctaggcgtctgatcccagcacagagcgcgacgggcatctgagagtgcaggaagaactaactcagggactcggccagagaaatgggccgaaattactgccagacacatccgaccttagtaaaggcccctcatcctgaacaagcggcagaatgatattttatctgtaagaag

SEQ ID NO: 10 - DNA, 541 bp, Homo sapiens
gcgcccttcggcagaagcagcaaaccgccggcaagcccagcgaggagggctgccggggtctgggcttgggaattggctggcacccagcggaaagggacgtgagctgagcggcgggggagaagagtgcgcaggtcagagggcggcgcgcagcggcgctccgcgaggtccccacgccgggcgatatggggtgcctgctgtttctgctgctctgggcgctcctccaggcttggggaagcgctgaaggtgggtggaacgagggcgcttgagtgcactcgcgggagggcggagagagggagctgggtagggacggggagggcaacgcctgatggggactggtgagacccgggacgcactggcgcgatctaggtagaaaactcgctgctccctggctccggggagaggcagcgcggcacagagttcgctggcatcagccgcctcctgaagctcatctcctcttgtttctttcttccttctctttatgctggctgctctcccggccacttgctacacgcctccaatcttcattctctcccagtcccgc

SEQ ID NO: 11 - DNA, 301 bp, Homo sapiens
tgggcagggtggactcagaggttgggaagctgctcctgagaggagaagcctctgtctctacacaggaacctacctgacacatgaggcaaaaggctccgacgatgctccagacgcggacacggccatcatcaatgcagaaggcgggcagtcaggaggggacgacaagaaggaatatttcatctagaggcgcctgcccacttcctgcgccccccaggggccctgtggggactgctggggccgtcaccaacccggacttgtacagagcaaccgcagggccgcccctcccgcttgctccccagcc

SEQ ID NO: 12 - DNA, 721 bp, Homo sapiens
gccaggcaacacgaagggactcgcccagggccccccagggctcggtgctggccctgatgccccgtgcctccccatctcccgaggggccactcattcggcaaacctttattaagcccctccaggacccccgacgccgcctaggcgcccagcgacgcgcggcaggtggcagcagctcgggcccccgccgcactccaggcgcccgcagcgctcgccctgacgcggccgccatggcgcaggagaacgcggccttctcgcccgggcaggaggagccgccgcggcgccgcggccgccagcgctacgtggagaaggatggccggtgcaacgtgcagcagggcaacgtgcgcgagacataccgctacctgacggacctgttcaccacgctggtggacctgcagtggcgcctcagcctgttgttcttcgtcctggcctacgcgctcacctggctcttcttcggcgccatctggtggctgatcgcctacggccgcggcgacctggagcacctggaggacaccgcgtggacgccgtgcgtcaacaacctcaacggcttcgtggccgccttcctcttctccatcgagaccgagaccaccatcggctacgggcaccgcgtcatcaccgaccagtgccccgagggcatcgtgctgctgctgctgcaggccatcctgggctccatggtgaacgccttcatggtgggctgcatgttcgtcaagatctcgcagcccaa

SEQ ID NO: 13 - DNA, 181 bp, Homo sapiens
aggggctcgtggggagggggcggagcccaggcctggagagccggggactttcctgggcccgggcgggggccttaatgatcccaggggagccggttgaagccggagacggggagcttgtgttggaggtggggggagaggcgtggaaggatcggagtctggaggtattggaagccaagggtgt

SEQ ID NO: 14 - DNA, 241 bp, Homo sapiens
ttagcgctcttaagattgggcctcccagtttgaggaaggggcgggctgctgtctacctctgtgaatctgccctggaccaccccgggagagaaggagggctccggggaatctcgcacattccaggcaaaggctcccgggccgcagcctctgtgccacacccttggcccgggccaggtgtgcgccctcctcgctgcgagggggagcgggcggctgcggggagcgattttccagcccggtttgt

SEQ ID NO: 15 - DNA, 421 bp, Homo sapiens
caagaacaggtgggaagaaaaacagcagcctgatccgtcttgcttttcccttttctccatgcagccagcacttttccttctcactctccccgcacgcccacgcccacccgcttctgcaccgagaacctcgaggcgcgcacgcacgtggaggtgacgccaagcccagcggcgaggtcggggctgggggtggggggagccggcgtcccgcgggcccccgaggccggggagctccgccagcgcattgtgcgagcgagctgaatgcagccgaggggcgagcgcgcgggctcgcacggattagccgtgctttcccatgagccacaaaagaatgcccgaatctgggacatctgtcatcaaggggcaggctgctcaggatgcaaggtaaccagagctttcctcggactgcttcagtctttggggacgt

SEQ ID NO: 16 - DNA, 181 bp, Homo sapiens
tggaaacgctccccagacgacgctcgccgggcccgtgggaggccgcgggagcttggggggacttcccaaagcctgagccccctagcgatgcgcggggtgggcgggggaaagaccctgagggctgcgcgcgctgcgttcgcgaggtccggccgtcagtgcgccccgacctttcagtgtccgc

SEQ ID NO: 17 - DNA, 1016 bp, Homo sapiens
ggtcgcgcagaggcgctgggggctgtggaagccccgcggccgcctcccgtgggcaccggtgtcgctggccgcggggaggccttctcggggcggagcggcccacccggcggggatggggactcctcgtggcggccgctgacggacggcccaactttaggttgaggggcgcggggtgtgcgggacccggcggcggagctgggctctgggccacgaccgccagccgcggctgccccgagagtccccgcacgcgcagtggctttccaacgcggcctcttcccatttctcacttgactccccttgcgcattaaattgtcgagaaacctttggccagtgggtcttcaaagctaaaccaaatggctgtccttgcagtccttggctacctgagatcccttaattctgaaccatccgcacctgggaggggaagttgaaaggagcgctggagctgagcccgcatccttaaggatcccattcactgcttatgatggtagagctttgaattagatgtcaggctgttcacgtcatccagactctggttttcagctctgtgctgagacagtgttttgatacgtatcagaggatgatgttcctatgggacaataacttgctgtatgttctgagatactagactgcgttcatattgtagcaccatcatcgtataaaacgggcgcctttgaaaggtttcagtaaacaccttcctcaggaacatccgccagcacttaaattgtacttcactttcactttgacgtttgttgtttgtgaatcttgtgcacaatttaaagtgagtcgtctaaacagcacaggatcacgtggtgcggggcattgagcaactggggaggaaagcagagacttgaacctgctggagtctagttggtctgcgtttttatgttggagaaccatcctggttccagcttattttgctttcgtaaatatgatgcattttttaaatgctttcatttgatacggtctatctggactgtaagattgagtctagccatgcatggaatgtgtttacttct

SEQ ID NO: 18 - DNA, 1546 bp, Homo sapiens
ctctgtactgtacttaactggtgagacgccacctcccgcccacatcttcctgtttttcagtctcccatttccgaccataagctcctccaaggcttttgcccagacccctagacgactgttctggacccagtttataaagactgcctggctggccaggaaatcccccagaggcctccttccgtgtccccgggccaaatctgtgaagagaaaacggaaggctaccatgtcacgaaaaactatgatcaaataaattattatgccttttctcctattgatctgccttttgtcaactgattttcagtgaaccttcggagagccatggggaagttttccctttccccctacagggctctgaatctgaaggtaagagtgagcctatagggggaaccttctggctccctcacaggaactgactgagcaggagttggaaaagccacttggattcccatttcctcaactccccgccaataccaaggcgtctgtttttacaggctctttcgtggtgttctgggcacattcaacttccaatgcagctgagagggtcgggaacagttagagaacaggggtggcagccgcccgggaggctgcaaggcgctcgcccgcaacgcacaggcgcgcgcggcgcacccggcctccggcctccccaggtcgggcctggcagctgcgggaaggaggtcagcgcagccgccacacttcgcccgggcgctggcccgacccgaccgccggcgactctctggcagcgcccggagaccgccagcccctgggccgcccgtccgcagagccccctccgccccgggaccctcgcgcgcagctcaagttgggagccccgctccgcaggcgagcgcgcgcccaccacccacacccactgccactcatgcacaccgcgggtccggagatgcccccgagcgttttaaaatccagaaacatcacatggtagccacatccggcggctgttacctgctcgcagcacccagaccctcgccctggtttcccgggagcccgcaaacccggcacgcgggctgcgcgccctcccgcaagccaccgctcagcgccagcgcgccggcaagccgcctaccttaggggtctgcacttcaggtcccgtcggcacctccaacttcctcttggttacccagaagaacagcagcaccgtgatccagagcaccccgaagactggcagaaccagccgacgagtcaggcgccgcatggtcccctttgccgcttcctctccgcggcgctacgtcccgggggcaccccccggcggtcagggttggcggggcaggagtcctggcgagcgcctcgctctggggagctctagacccaggatccggttggaggggcggcaggatcctgcaaggcgcccttcccgcttcgaagagaagcgagcctgggtggggggtgcagggcgacccgaaacgtggcagggaaggaccgagggcagccaagctggacgcccgctccagcgggagaagcgcggtggctgccgagatgttccccacgccgccaccgcggctgccgccgccgccgccgccgccttgcccgctgccgc

SEQ ID NO: 19 - DNA, 181 bp, Homo sapiens
agaggccgcgctttccagcgtggagaccggacggtgcggccgtgctccggctcaggccctccgcgcggtaggaaacggcgagggccgtcccggggagcagcctcacttcgcagctttgctcgccttggtagggaaatggccttgggcggaggcgggggacaggcagggaacggagtggcca

SEQ ID NO: 20 - DNA, 661 bp, Homo sapiens
gcgccgagggtggagggagaaggggcttttgagatcatcctggagaggaaactgaggcctgggggttgtgggtggaaaacaggaaggaaccggtagcccttggcacgtattcttagaggagaaaacggaggctcacaaaggtcagatcacagagccggccagtgttggagcacaggcggcccggggtgagcgccagaggtgggctttcttccctcactgaaagccgggagggagagagagagagagaacgggggccggcggagaagagggcgagacgaaagtaagcaaagggacattagaagggaaggcagagccgagggacgcggaccgagcggccgagcagtggaaagggcggcaggtgaaaggcacagagaggaaagatgcgcgggggacgcgccgctcacctatggttgacaccacggtgcccacgaagtagaaggcgccggggaagtcccagcgcgggcgcagcgcgtcggcgcggacgccggcggccagcgcggcctcgtagtgccggaggaaggcgcgcagctctggctcggccacgccgtgcgcagcgctgaagttgcgcagcgtggcgccccagcgcgcccgcgcctccgcctcgccggggctctcgagcgccgagaagactgtggcacccgccaccaggtagaggccgatg

SEQ ID NO: 21 - DNA, 181 bp, Homo sapiens
gccgatggggcgcggctccttggagcatgcgcacacaaactttccgctaggaatcaagcgagcatgcgcacacagatgttagggttcgggcgagctatttggagcctgcgcagtcagatccgaggacatgttgacgtcgtccgagagtcttaaaatcctgctctggccggattccagactc

SEQ ID NO: 22 - DNA, 301 bp, Homo sapiens
ctgggttgggagcctgggcagggtgggtgtcaagtggctctggcaactggaccccttcggggttgccctcaggatcaggatgaaaagggggaagtcaggctggagcagcagcgcggttcacgcagagagcaccccaggcagccacgaactggcttgctccgttcagatttctcttaaacagcagttttccgtttctgttctatggcctctgagggaatttcccaaattaaccttcactaagctttcctgagggactgtttttgagcgctgatgggggaatttcccccttttgaccacactg

SEQ ID NO: 23 - DNA, 181 bp, Homo sapiens
aatcttcacctcaaccttgtaggaggagccggtgagcagcttgatggtgcggttctggccgaagcgctgcccgtccaccttgtaaaagaccgggccgtcattaggctggatgcgcagcgcgatggagaggcgcacgaggcccggcaggtcccccatgtctgggcgagggtctggcgcggcg

SEQ ID NO: 24 - DNA, 541 bp, Homo sapiens
aggttgaggtgaaccccaagccccacgcggagaggtgccgcaacccggcgcgcggacctggcaggaagaccggcacgaagtggctgaagtacatgatggagttgctcagggccgagcagaaatagtagccctcgttctctcggcggaagtcgctcagggtgaggacgaaggtgtcccccaacctcttgcccgagaaccgctgggtgtccagcccctcggccgccttgggcttgttttgggagaggtataggaggaaggtgggactggcggcggcgccgcgcggctggaagagccacgagcagcccgacgtcgggttggacagcagcacctggcacttcagctccactgtctcgcccaggttccaggtccgatccagcggcgacacccggaactggctcggcctggcggcgtctgcaggcggcaagcagcgaggctgagcccgcagtcccgcgccccccgccccccgcccgccccatcccctgccttcccgggcgtctcaaactcacggagcagcaaggccagcggcaggagcaaggcggtc

SEQ ID NO: 25 - DNA, 541 bp, Homo sapiens
ggggcgacgcagtggcgaagtcgggctgtgggcccggcggcggcaccaggcggagaagcgccactcaaccccatccctgggctgcagagggcccagcgcggagggctccgcgcgtcgggagccggtggaagaggagaagagcgcgcgggcgacagtcatacaggccttggggcagggcgcgcctcgcgctccagggagccacgccagcccgctgcgcctccgcagcaaccgccgcctgcacgtggcggggcgagagagctgctagggcggtttctccgcctcgggcctgttgggcggggccggctaaggtgcgcgtgctcgctggtcctaacggttctgttgggcgtttctgctgagaggcgggaggggctgagagtctgtgcgaaggtaggtggacagactgcattgcttgttgttgcgcttcggaggcggcgatccccgaaggcgagctgaaatacggctggagcgttcccaggctacagtttgtagccgacgattgtggaagactaggagccggagaggtggcccaccctcagggagc

SEQ ID NO: 26 - DNA, 1201 bp, Homo sapiens
ggtctgcgcggagtctgagcggcgctcgtcccgtcccaaggccgacgccagcacgccgtcatggcccccgcagcggcgacggggggcagcaccctgcccagtggcttctcggtcttcaccaccttgcccgacttgctcttcatctttgagtttgtgagtggctcctggccggggaagggacggggtgggctgagccgtgcgctctctcgggcgcccagcacagctgtcggacgggatccgctagctgcgcaggttctgggagcatcggggcagcaggcgcagggcggggactaagccagggaagtcccctcccacctccggtcctttgtgcccttctagaccaacagaatgaggggaacagtctacaggactatggaggaaaaactgggttcccaactggggtcagatgtaggcagcggggcagggggggacggctcttggttcgctggtcccaaagctgcgcgcggggcccacttgacgcgcgcagcgccaccgaagctcccgccgcgctttgcgcggttgggtagaagtgcgcagcttttacaagggagaaggtttcgttaaaaaagaaaaaaaaatcagcaagagaaacattagtattaccaaccgagatttggagatgagagggagctgaatccggtttattttcttctggccttttaaagtttctggcgagggaacgtatttgcgaccaattcgatctggaaatgaggccatcgtttgcttggccgcagtccttctgccccgtgtgcggggtgggggtggaggagatggggggtggggggtggggggtggcggcgagagcgatccgcgcgcctcgactgaccttgggcaggcccggggcctctgcacctgcggtcggtcccgccttgcacgcacggtctctgcctgaggctgcaggaaagcgcttcctactgagaactcctgataagcgctcacggtgtcgcgaagccgaagtgacctccctcagcctcaactccccgggggccgctggccttcacctgggaggggtgtgccctgtatgtcctgtgggtgcggtccgtcaccgcctgagggacaccttttccggcaccccaccctcagaagtgtcagcgtggagagttgggcgggaaagaaaatgtcggagcctggctgtttaaaaattggaccccaggttgttattgcctgattggagggggagggtgtgaataccaaagggagc

SEQ ID NO: 27 - DNA, 421 bp, Homo sapiens
aattctgcttggtctgtggtaaatgccctttctgagaagcaaccatgaccttctcaagaatacttcagaggcacttttgctccttctccactaaccgacatcctgttttgctggaacacatggggcagagcgcacacagctttgttcctgcacccgccctcagagctttgccacctgttttcaggctgcctctgcctccaaaccctgcggagccctccctgccccgtgctttgaagcagtttctttggaagctgctgcacaggggttaacaacaagcaacaactcaggtcgcattcttgtcaacggaagggagggccaggtggaaccgccaagggggccatttctggctttgctggaggctgtcagcttctggtgggagccacagcctgagggcagccaggatggctctgctgggagggac

SEQ ID NO: 28 - DNA, 601 bp, Homo sapiens
ggcggcgcgctgcgagcggctgagaccgcgggcgggggcgggcgcctggcttgggcagcgtcctcagcgcggtgtgggcggcgagccccgcagggctgcaatcgttccggggtgggggccgggacaggcaccgcgggcgcaatctgagcccctgcccacgcgcagcggcctctcagtcccgccggcttaggtaacccaggtcgctgcggtaacgcagtgaccgcgctccaggtccgcgtctcttgcgatgcttcccccactcgcctgagggctcctgcgcgactgcgcgcgcgtcctctgcctgccgcctccccgcagaggtgccggggccctgggagcaggtggccttggccgcgggctgctggcgcgccggcaccgcggcacctgctcttccccagaggcctggccgcccccacaacctgtggctccgcttaagcaagaacccaggaaaagtcaccaaacgcatcacgcatctctagcttcgacttaggaaattgtcctaaatgactggggaggctgaagtgggcacccagaggccccgcctcagcgagcttcttctcttaactctaggctgaggcctttgagaactcattttaacaga

SEQ ID NO: 29 - DNA, 301 bp, Homo sapiens
tttctaggacttaccggtttctcacaccctctccccaccatcaaaatcatggtttcagaggcattaggccaaaaaactgcaaaagggagcctccttctgggaagtctccggcccttccgcggctcccggcgtctccagcagagggctctcggctgtgccgactcaggacagctgctgcgacggggccggctacgcttgtcagagcagcagctggtgattttggacttgcctttgctggcaggggagcgctatcgagggttcattttatccagcttgaggaaagaaaggtcggagtgtaggg

SEQ ID NO: 30 - DNA, 301 bp, Homo sapiens
tgagccgagagggccactgagccccagcctcagcgacacagctagaccctgtcaaggaaaggggaaggaaggaaagggaaagcaaagaaaagaaaacaaaaaagcagaagcaaacgggcaagaggccagcgtgtggtcccgggctggcctcagtagtaaagatgctcggaggattgattgatttgccggattctgcgcggtttcccagcctgtgcctggttgcagtgccctccctgtggtcgctggctgcccggacccatacccagccccacgcctgccctgccctcttcccagccagagt

SEQ ID NO: 31 - DNA, 181 bp, Homo sapiens
ggcgccctcggctctccccttcgggcctccggggaagcgtccccgctaggggtggggtcttgggactccctggggcttccggagctgacccgtggggggtctgctgccctcagttcctgctgaccaaagtcctgccggatctggcgcctacgaggacgtggcgggtggagctcagaccggt

SEQ ID NO: 32 - DNA, 181 bp, Homo sapiens
actttaagcctcgctgaggcgcagacccggttcccctctcctgccttcgcagtctctctgccacccccgcccccgccccgggatcctgcgcgatccagcgcctgggcccccgccctgccccaggcggacgctcccgaagcccggccggagacccggcgggccgggcgcgagcggagcggga

SEQ ID NO: 33 - DNA, 371 bp, Homo sapiens
accagaagagcagcatgaggagccccgccgggcggcgaggggtcgcccagcctgtcctcatcctgagctggcgcaagccttccggccgggtcctcgggcgcacgcggctcccgccccgcctgctgagcgcggcctgccccgcccgcacctctgtctaggcctctgggggcgccccggccccgcccccgccgccctcggccaatcagacgtgcgtctcctcggccccggggcggagcgggccaggtgtgggaaatgaacagggctgggcgctagatacctgcgtggggtaggacccgcgaggaagaggtacgtgcggatcggtgggagagccaggcaccagacaggctcctgcactggagggttcggtcccc

SEQ ID NO: 34 - DNA, 481 bp, Homo sapiens
ggggttgaggtcctcgtccgggagacaggaggacaaggatccccgcctctcgtggggtgccagcggcatgagattattacacgtggtggagaaaatgcagcgcagtaaggggagagagcacccacctctccaaccccctgccctgccgcgactccaggctccgctcctgggtgggggtttattttctcttggcatcacgggacagaagaatcgatgcataccctttccggctattcagaccttgcggggtatgaagttttaaagaggggtgggggcaccggcaggtgcagagtaacattctttttttgttcttgaaagcaaagtgtgagggacccggtggagctgtcgaatcccttgctgaaattcacagctctctgcccccgcagtcgctcgctcaaggtctgtgttagagaaggtcatttgggaggctgctttcgtcttaatacctgcttctcgggaaaagatctttacgctaaaaata

SEQ ID NO: 35 - DNA, 361 bp, Homo sapiens
cgaagagggaggaagaagagagtgccttacaccaaactgcagcttaaagaactggagaacgagtatgccattaacaaattcattaacaaggacaagcggcggcgtatctcggctgctacgaacctatctgagagacaagtgaccatttggtttcagaaccgaagagtgaaggacaagaaaattgtctccaagctcaaagatactgtctcctgatgtggtccaggttggccacagacagcttagaagccattcggttgtctccaaaaggcctttggaaagacttgaatatgtatttaattccccccaccccctgccaatggtggcaaattttgtgaattgtttttctctcttccccttatct

SEQ ID NO: 36 - DNA, 181 bp, Homo sapiens
tgaaataatcatgtccagaaatgtatcaaaggccagagggattatcccacttaatagctccacagatgcgcccagaagaatgtggacgcgcgacaggacgggctgaaaggctgcaggaggaagcaggcagccccggctcctggctttaccatttcggttgctttcctaaaaggctacatgc

SEQ ID NO: 37 - DNA, 301 bp, Homo sapiens
tttggggcgtgagttttcttcgggctttttttcccctcttttaattccccgagcgcaatttggggcgcatgcgtccacgagacgccccgctaccgccctctaagggtgaagcagggactccagccagtcctcaaaatcccagggcaccggaggctggcagccgggctgggggagggcggggaggggaaagccctggagccacagagcacgaggttgggctgaatctattcgtaccttttattggcttcactgcgcgaggaaattaaagatcctcccccacccctacaggccttcaaagcag

SEQ ID NO: 38 - DNA, 181 bp, Homo sapiens
gggaggaaatccgacttcaccttgggctcagagttgcaaggaaggtcactgtgggatcagcctgagcccaaaaggatgggctaatgggagcggccgcaggtgcacgcgcgctcggccgctcccattagtgttacgtctgccgggggaagaaggtggggtggggggttgggggcgccgggag

SEQ ID NO: 39 - DNA, 661 bp, Homo sapiens
gcccagctagagtttccaaaaaagttagaataacttcctctcccggagacctcggttttgcacaagccggccttgaaatcagagcctttccagcaactccgagagcgtgtgctcggcgaccgcgggcttggccagcggcgcgcgctcggcgccccggcgcccccagccccacgcgcgccgggcgggcgccatggaggagggctccagctcgcccgtgtcccccgtggacagcctgggcaccagcgaggaggagctcgagaggcagcccaagcgcttcggccggaagcggcgctacagcaagaagtcgagcgaagatggcagcccgaccccgggcaagcgcggcaagaagggcagccccagcgcgcagtccttcgaggagctgcagagccagcgcatcctggccaacgtgcgcgagcgccagcgcacccagtcgctcaacgaggccttcgcggcgctgcgcaagatcatccccacgctgccctctgacaagctgagcaagatccagacgctcaagctggccgccaggtacatagacttcctctaccaggtcctgcagagcgacgagatggacaataagatgaccagctgcagctacgtggcccacgagcgcctcagctacgccttctccgtgtggcgcatggagggcgcgtggtccatgtcc

SEQ ID NO: 40 - DNA, 301 bp, Homo sapiens
cattttaattgtccaaaactaattgcccttttacaagtctgtgatataagaggcaggaaagcaatgtggagacagaggtgatttccattaacagaggcctggcagcaggcaggcactcaccgacgcttttcagggaagtccgtctcctgattaatgtgcttccgggggcagacagcggatgcgtctccttgctcagggatggggtgcatgggggcatggtctgaggttttgtgcaggttgtttgaggtttccttagccctcttgctgagaaaggcaggaagaggacagtggagtgtttctg

SEQ ID NO: 41 - DNA, 550 bp, Homo sapiens
tctatagtggccaaggggtccagttgtcccctgagtccggaggggtgggcctaagaagggggcagctctcccccattaagcaccataagccgagtggtacagagcttgtgcccaaccccagcagagaagcactaagggggggttggtgccctccttggccacatcctctggaccagagggtataaacagccacacagtggtcacttcttgataggagagagagttaggctgcgggaagttcccccgttcaaggtcgtgcctcatgggggcccaggtgacagccaggccggggttgattttattgtgtattcaccagcctgagcgtccttaggggtggcaggcagggaggtcgaggtcactgatgctggtgctctcagcatgtagttatgcaggagagtcactgctctgtattggacagaggctgatggaaaagggtggtttgtggatcgcagtactcaagcattcctggaaaaggggactctgagaccagcccactaagaatcatgctgttcaggagatcagccttcaagagaaccagttttcaaagccc

SEQ ID NO: 42 - DNA, 419 bp, Homo sapiens
gctgaagacacaaatgtttacaatgaccacagcgatgacgggatccgagagaaaggcaaggcggaaggggtgaggccggaagccgaagtgccgcagggagttagcggcgtctcggttgccatggagaccaggagctccaaaacgcggaggtctttagcgtcccggaccaacgagtgccaggggacaatgtgggcgccaacttcgccaccagccgggtccagcagccccagccagcccacctggaagtcctccttgtattcctccctcgcctactctgaggccttccactacagcttcgcagcccggccccgccgcctcacgcagcttgcgctggcgcagcgtcccgagcctcagctgcttcgtctgcgcccctcctcgctgcgcacccaagatatctcgcacttgctcaccggcgtctt

SEQ ID NO: 43 - DNA, 541 bp, Homo sapiens
ataacgcgtaatggagttaagatgcagattctggagccagactgtctgagttcaaaggctcctaatagctgggctccttaacctctctgtgcctcacttcctcgtccggaaattgaagctaataagagcactgacttccctgggcggcggttgaaggctacctgtgtggatctgggcacagcgaagagcggagccttaacagggtgagcacgccggttgcgcgctctccagagcagcccagcatctcccgccagcctcgctgcccgctccgccccggcgcaggggccccaagcccacaggcaacgccagcgcgctcccaaccgctggagacagaaacaatgtgcgcgcgcacacggcccacgtgcacgcgcgcacgcccacgcggcatacaggcgcgcacgtgcacacgcgcgcctgcacagctctgcggctctgctccggccccacaggcccatcttaaagtgtttcgtgctctaacttaccaaacacgtggcagccggcagaacgaaaaggaaaataaatgaactgcgacgaaataaag

SEQ ID NO: 44 - DNA, 421 bp, Homo sapiens
agtttgaaagaatccagtgtagaaacagacttctccgtccaatttggttttaatcagtaatcatataagtatacccacataaccacctaagtggagagcagacgcccagattcacggtccccacgtgttgctggagttggcgcagacgcgtgtgcgggcatagcggcggacgtgacaccgcattttctccgaattcctgccatctagggtggtgccgccccaagagggggccgtggggaggtggggtaataggctgcgcaatccacttgctctgggggagcttagggttcagagcagagcgcaactccggggggctgtcgcacagccccattctcccacaccagaagagcaatgctccttatggatgattaatagccgggcttctcctgaccatgcggcgcgtccctgccggcaccactta

SEQ ID NO: 45 - DNA, 181 bp, Homo sapiens
ctgcgggctgagctcgccccctcccccgacttctttgcggggcattttctcttgctggtgtattacgtgtcatttctcacggggcattgccggccgcttttctgcaactgtcctttcggatttggtgatctggtccggcacagaggctctcctaggaggtggtgcccatgcatattcattc

SEQ ID NO: 46 - DNA, 181 bp, Homo sapiens
ggcgccggagtggggagcaggcaatcccccaggctcggagaaatcttttatcccgaaatccagggtgtcccccggtcaggatcgactcggcgccgcgttggcttcctcgctcaaccctgacatcccggtccccaccagtcaccgcagccgggcggactccgaaggcagcggccgctgggga

SEQ ID NO: 47 - DNA, 421 bp, Homo sapiens
aaggctataacactggtccagcctgagagaagcccaagtggggttcactgccctctgagccacagatttaagggggagggtgtggaaactgccggctgctgaggtccaaactcaccgaaggtactgaccgccgcggctcctctcttcacagcgtctgccggaggcctccgtttactccggttaccgagacaacgccacccctcttccagggaggcggaaccagggcgggccgtggggcgcatgcgcggccggcgtccagctctccgggaacccggtacctatccgccctttggtcgggccttctccgcctcatgacactggttcaaagccaaacagaaaagcccgacgagtttattatcccctaaaggacgtcatgtagataattaaatgacatgaataccgtcgaagatacctgcctgat

SEQ ID NO: 48 - DNA, 325 bp, Homo sapiens
ccttcctcctccgggcagcttctctcagtggcagctgtgttccccatggtttgtcctggatgtctcccttgtgccatccttgcaagcccgcggccagcgcctccacccacgctccggccttgctcccactcccaccgctctgccacctcccacctcagcctcccaccttggtgtggagggaccagcgtcgaagacaaaggaatctctgacgagaaccggccagtccgggagggacggcggggaagggggtgctgctctggcggagccctcacttcactcgcttcccctcgagcgcccctctaggctggggcccggccgctctggg

SEQ ID NO: 49 - DNA, 1201 bp, Homo sapiens
gttcaattccagccccttaaagcagaaggctccctccctcggcatcagtgcaggctctcccacctcattactgttctgtgtctttgggaatcgtagagtctgtggcccccacgtcctaggtgtctcggcaccctggacccaggcgcctccgagattctatatcgcttctgacccctaccttcaagcctggcaggctccccgcggaaccctgctgagacccggagacaatcgggccgtgcttctccctcctccacgaacagccacggtttatttggagcggccggggccggcggcctgacaactggtaaatccgtttcgttaggcacaatttgtctgcaatttgtcagcccggctgggaaacgctccccagacgcctcggctgccgcacgggccctacctggttctcgaatcctgcctgctcataaacgaatcctagcacggggtgcctgcgtagacctggagctcaccaccagatgttcccgacctcgggagaggaggctttttccaaaacaacgaatttccttccttgttttccggtaaaggagcgttcgccacacacggggtccctgaacgcggggcctttcccctcgtggttggagcaacgcggagttcaagcctggccgccacagaataattttaaatgccccgttttcagacagatccagaacgccgtctacgcctaccggcggcagatcttcaagcccgcggcggccccattcttattgaaatcccactaaacggattccgactccggcttggggcggggggagacttccagacccggcgctctcccccacacgcaccccagtcacacaggataaagggctgcggggcgcagcgcgcgggggcgcaagcaggagcgagctgggttaagccgcgaaaagccggcgcacgggaccagccggcaggtgcagccgccgctcggcggcccggctcggacgcatccgccgcggtggcctggggattgggggcggccgagacaaaggccccagttcgggggccgggaggcgggggtgctttgcgaggctctgggaatgccagggtctcgtggcctgtggctccgagaaatgggaagacaagaggcccgaggcgggcctgctgtgcccaggtaaccaaatactccctctggttaaagtccctataaccagggtttccggtctctggcagggccaaggcgagccccaaaggtaggggccacagg

SEQ ID NO: 50 - DNA, 601 bp, Homo sapiens
gttgttgtgagtattgcactctgtttttcctgtttcttcagtatttatttcacaaggacagacagagaatgtgtgatttgaggtgattagaaagctgatattattgagggcgacaccgtgagagagacagagagacagaggcggagagaaacccgaaaccccgttacagctaggagcctctgaaactgacagctggttttcctttgcttgtctgcctgctagacgtggacatttttcatttacggttctgcacgttacctcggatgcctgcttggctttccttaaagggagattcatttctctgagagatgatgtggatggtattagcagaaaagcccagaacaccagaaaggtgctgagaaaagcggggcccgcaagacagagcaggttctatcctgtggggcacttgtcttccttgcgaccgtcctttctgccgttcctcacccttcaccttgcctttgtttcatattgtgtaacagtcagtatcttgcgattgcaatttggtgaagatgaatacttgttcaaccatttttcaaaagctcttatgacgggagccatagtggtgtatttatatatattcatagctcttctttatgtcact

SEQ ID NO: 51 - DNA, 481 bp, Homo sapiens
tttccctcctcggcccagctgaacgaggctcaatgcctcaaagatgcagagctgcctcggtggacatgctctgtggctgatattataattttcataatgcgcttttatgtcgcgccagactcctccggtgaggagcccgcagagctgctgaaaggggctttgagaggcccgggcgcgcggctgctgcgagctgcgcgccccccgccggcctgagtggcaccgcgtgcccctgccggggcgcggctcctgcactgcgggcgcgcaggcggcggcgggctctgccggcgccccttattagcatgcaccctgggtgcgcctggcctgctcccgctgcttccgggcctctctgcgcccctccgagtctctgccatccgcctgggtgcgaggtccctggccttgctcctggtcaaactccattccgctccagctcaggctttagggaaggtcaaggtgttaaaatgtgggcagaacattccggaag

SEQ ID NO: 52 - DNA, 661 bp, Homo sapiens
agaagtggagagaagaagaaacaaatggaggaagaaggagaaagggaaaaagcagacggaaaaagtgaagtagtacgagggcgtcccagcggggcggcccgagaagctccagcttcttcccgagcggccgccgctatcccccgggggggcgtctggccccactccggaccacgcccgagcgatcctggtcgccgactgccacagccgtgcttcccggcgcgggatccaagccgcggagccacctgttaggcgcgcgccgtcggaagcccaggcgcggcggcgctggagaatcctctcgaagtttccgggtgcgcggggaggccccaggtgcgccccgacatcccgacacggcccagcacgggtaagtgtcggcggccccccgcttctccttcctgggtcccctcccgctgcccccggccgtggcgggaaggaaagttgtgcggagagttggtacctgcgctgagctccaggctggcgctgtcgctacccgtgccgccggtgccggcggccgccgccgcgcctgggccatacctgacgacagcggcgaacgaagacgacgaggaggcggcgggggacgcgggcggcggctgcgccggagtcctcaagtggccctgggatgtggcgggcgtgcaggacggcgacgacgacgaagcggcggcgg

SEQ ID NO: 53 - DNA, 1261 bp, Homo sapiens
gtgctgatagcgcaccccagcacggaggaaagcctcacagtctacgcccttgcccctggggagaggggcccccaccgcgtccaccaagcgcccgtacttgggcagggggccgtcctcgtgaggaagtggggtaagccggcacctgcgggtggccgtggctccagacttcagggaggcgaagtccagcactctcctgtctatggcgcggctccagcttcgcagcttctccactaccaaaggcctgttacgcgtcaccagctccagctgggagaagaccaagtccaccgccagcgtgaagggcagcaccagagtgtgagtcggggcgtcgtagcgcagctgcagcagcacccgggcgcgtccggggctgtgggagccgaagtgagtgtactggacttggcggggcccgaaggtgcaggggaagcggcgcggggagagcgcgcccttgagccgcggcagggcgtccagtaccgtgacttcgcaccggtcccccggctgcactccaatcaccagatcccggagcgggtcgagccaaagggaacgacccaggggcacccggagtccagggttggcaatcagcacgctggggccgtcggggcgagtgccgtcaagcgcaccccgggcgggcaggtaaagcgccgggtcgggctcggtcccaagtgaggatgcccgtccctgcagcgcggggcgactcaagagcaggcaggcgagcgccacaaggagctgccggggcgtcccagtcgggtgccgagaagcccccgccatggccacggatggctcctggcgttgggattcccggggtggggtgccctgtgcaaagagggatctgctgagcggcaggtgcaggcagtggaagcagtagctgctgtccagtcggtagccgacttgcggatccagcaagagccagcggctgcgcttcggctgctgcaggtaacggcagcgggggaaggggctctgcccacttcctgctcagccccggtcgcaagtctctctctgctggcttctggggaccccagatacgcgcccagcgcggcgagacttagcgagggtgcagcgctgtcccctccgctcctgggcgcttcacccagcctaccttacacaccttctcgccgggagccgtggccgccgcactgctgcccgcgctgccagactccgaccagctgtctggatactctcttccccaggtgccacaaagggattgtccctcagggttgggagagagacggtgactgtactcgggtcagtcctgcgtctgtgagattga

SEQ ID NO: 54 - DNA, 181 bp, Homo sapiens
agggaccgggagcggcaggggctgcacatgacctggggcgcgggaaggagcccgctgccgtctaggcccgcgaagggccccggcagccgccgacttctgaggaaaagcagaacggtgtttggtttactaaagtagccgcctcctaccactcttcctccccagccccgctctctgctcccca

SEQ ID NO: 55 - DNA, 181 bp, Homo sapiens
agcatgtgtggaagaggcaggcattattagcagcgcgtccgcctcggccacctccctgctcccgcctcggccacctccctgctcccgccccggccctgggggcctctgttcagcctccaccagctcagtcgcccacggagactcccgaactcttaaatcccagccctgtagtcaaaaccac

SEQ ID NO: 56 - DNA, 721 bp, Homo sapiens
cttgcacacatgccttcagcccctggtaccgtcttctctccccgggtcgcgacactgactcgtcaacgttaatgggggtccgcgactgctgcggggacgagggcgcagagcagcccccgccacgggccggtccacgcaggggccgagaaagtggcggagaggcggtggccgaggcccaggggcgagcgcgggctgagctggtccctgctgcgttcacgagcgacacccaccccttcgctgcggacgccccgcgggcgccaggctgggggccctgcgaccgacccctcccgcccccgaggtaccgccgggcccgcctggcaggcagcgcgtcccgcgagctggagggccgagtttcgcggggccgtggggcgtgtgggtgaaggcgacacctcggatgcgggacgcatgaatggtggcagagcaggggtcgggatccgttcatgggttgggagagagatgcttttgtgagcacgggaaagtagcgctgccggagaacagctctgaggcgggatcaaaagccgccggcgaagccccgccgaggaacacggccgctgcccggggcggctcgcgagcgtgcgtgtgtggaggggaggatgccgccccgcggggtcttcggagggtgccgggagcgggttctcagtgcagttcccccgtcttcgctgggggcacggctgctcacaggccccggcccgcgtgtgtggagcggggcgagggggtgagg

SEQ ID NO: 57 - DNA, 181 bp, Homo sapiens
gctattactgtcaagtacccttgactctttatttttgcccttttatctattacaactaattcgagttcttttgcccttttcagtctaagacgtgggctttctgcaaagcctccccctgccagcgagctctcggagcgcggagcctttagaaattgaggggtttactgtcaaaatgaaaatt

SEQ ID NO: 58 - DNA, 601 bp, Homo sapiens
gccttcgggaagtcctgcaggagccgcgttccaggagggcagctggcagccgccccaggcccccgggccgcctgcaggtgattaggctaatgagctgccccgggggcgcggagaccggcctggcgagcggattacccggcgcccagctgctgccggcggagactcccaggagctccggagaggaaccctccgaaggtgacttcagaactggaggtaggaaatcggcttctcaggcgaaagcctcaggttttctgatctgatccaggtcgggtgcagactggggctgaatccacaaatgtggagatttagccacagcctcggaggcgcggagcggccacctaagcgtctgcccttctcgtctcccggatcactggggtgtgttgtttttaaagtgggggatttgcgtgttgagagacggtttgtgttcctcgggaggagtaagtgacttggagctggtttgtcaatggctggacggaaggaggcgccccggctgtgtgtgacgggcagggaaggggtgcccagaggggacaggtaatagggggttccggagccacggcggtttcagaaccttggggcctgtgccgttgaagccccggtaggg

SEQ ID NO: 59 - DNA, 361 bp, Homo sapiens
ctcgaggctgaggatggtggctatggcttcggggagcggggggacgcggacgtgtaatcgccagtgtggcccattttacggtagggtagaatctgagggaaggcggactgagatgccggtatagcgccgatccctcctccctctagtcagggattaggagcactgcgatgagggaatcccgtctctgctcccccttggcgctcacgcgcctggaatgtgagtggtgcaatcccggcaaagctccccgagaccccagtgccacgcggatgagaccgaaggggagcggagttgagccaggcgccgggctagtccacaacttggcatggccgagcacctgggcgctggtcgtaggggacagcgc

SEQ ID NO: 60 - DNA, 601 bp, Homo sapiens
tcctgaatccagctttgtgcttttacacaacataacagaaatggcatctttcacaaagcctaactttgacctccaacactttaactttgggtttaaccagtacaccaccttcggaagttagcacataaaaatacaggtaagtcaaatgcactacggatacagaaaggacgaggaacaggtttaaaggggagttgaagcagaggggcacgaaatcacctggcaggtcacctctccgaaggaaaaacatttcaagctccctcccatcccccaggtaacctctggcctcagaactcactgccctgcgtggggcagaagttctgggcgctggagtccgcgtcccccaggacacgagggtgacccaagggcgcgcggagagcggcgggacccggagcggcgctctccggggtcactcccctaggacgctccgcagagctgggagcgctgccccaccccgcccgggccgcccctggggaccccgctcggggctccgcggctcccctgctccgcgccgcgcccacccgcccccaggactcacggtacgctcccgcgccgctatcttgccatcccctgccgccggctctgtagcctcggccgccgcccc

SEQ ID NO: 61 - DNA, 301 bp, Homo sapiens
ccgacctaaccacactccagtctcttctaggtcgtcaccgctctgcaccaaacaaatgagtcctgtttcaccactagggtgccgaggtggatggtggatgctggcccccgcccctggcagcgctcagcccttagaaaccagagccagctgacaacacgcgaaacacacaggcacagcgaaaacgccgagccgacgctcattccctctgccccctccctctgctctctgtaacaaggaggacacgtacacagcctttacacacttaaaagcccttgcgactccctctgaattcttagttact

SEQ ID NO: 62 - DNA, 181 bp, Homo sapiens
tggtttcccctgcgtgcgggatcgcacagcgcctgtttccttgcttcccaagggggtggtgtggaggggaagggggaatgatttttcttgcgtctcccggaagctgtgctgttagacacaattacctcagctaggtcactgagaccaaatcatacgggacgcttaatgaaggaccgcattc

SEQ ID NO: 63 - DNA, 961 bp, Homo sapiens
tgcggctcggtcaggcgcgtgggggaagggcagggcaagtggggtgatcatgatcatttttagcccagggtcagtagagtagggcacagaagtcagacaaatctgccagagtttcaggagcgccagctacatggccagatcctgcccgggtggcctcatttctctgggtccccgcactccttgggaggtctgatgaaagcttggggtcttctccattccccagaacactgcagagaggagttttattttgcttacaattcaggagtccgggcaggcagagcgggcccaggttaaggacgccttctagagctggggatgacaggatttgtcagtggaaaagcgttggcttctcacggccctagctggtacagggaaccgcgggcgggaagctgggcgggacgcgtggacttgctgagaatggggatgtggagggcttggctctttgcggagtgcgggttggcaagaggcgcttggagtagaataaaggcggcgcagggccaaaaactacctaaagacacagctcccgcaggcgcgcccaaggtgcggaggaaacgctccatgtatggggacaaaatagtgtctgtccagaacgtacatcttgggtgctcaaacccgacagtgtgccgtctgagacgccgacgcaagtgaagtcaagcattggcctgatgttgggacttttcctgtccctcatcaaagccacactcccaggacctggggcctccatgctggggagagaggtgagccccgcagggcagcccaggaggcgcgcaacgccctgaccccggcttctaggcgccagccgtcagtaacaggcctgggctgccacgccgaaatcacgcctcgagtttctgagccagggactactgggggtctggaattgttagtctagtctgtggaggatgccttttcttaaatgtggggcgttcaaggcccaggaaacctcgtccccccacctcttcac

SEQ ID NO: 64 - DNA, 181 bp, Homo sapiens
ctccaagccgacgcgccctgttttatgccttgagtaggcgggagccttgcaggtctgtgggtttctttctcaaaggaaaattgctgggctcgtgaggaacagcctcgggcacttgctctacttggaaagggtgaagagcgcgggctttggaaccctaggcgcgcccgcaatcccagctctg

SEQ ID NO: 65 - DNA, 721 bp, Homo sapiens
aaataagtcgtgaacatttctgtcttttaaaactgtgactccttggactctagccttctctgggaggccgggaggctgcgcgcgggacggattttgcaggcgcacgcgtcccagcaggtcgcagcccgtgggtccctcgctgtccttcctgaaccccgcttaggcgagactctagcgggtgaccctggctccttccctgtcctctctgccgtccccttcttgtgcggtttccatccgttcattcattcgttcgacctctcattcattccgaacttcctcctgctgcgtcttctttcgtgttcaccacactcttctacctccccgcccctcccaacccccacttttcttgccaaatgtcaatgatttgggacagctcccagccgtgaattaataaagaccgaggttctgttgcaggaaagggcagacattagggaacaaatacgttcaatttcaattccacagtcaacaaatagtcatttttggaccgaggttaatgtgttcaaaacgcgtccctcaggcacgaccaccgtcttttttttccctccaaacctctcaaagtaaggttatttcctaccgggaaaacagagtcccaaatcttgtccgattaaaatttctatctcaaaaacaactctctctcctgctctctaaaaattcaaaggtttattgcaaaatgccacattcacttatttccaacatttaaggaatttgctgccattagaaa

SEQ ID NO: 66 - DNA, 241 bp, Homo sapiens
gatctccctctaatggtagaaacttttcccttttccagctctttaccaacagcctaatcgcctcattagcatatcaacaatagtccaattgctcgccagtaccacaatctgccgccggccgctccgacacaggtataaaggcctctctacgccgcgaacttgcttctagagcgcactccagcctgcgaactgataaaaccttcctcgagctccgccgcgaggccctgccccaacaccccct

SEQ ID NO: 67 - DNA, 440 bp, Homo sapiens
gagatagagtgagaactccgtctcaaaaaaaaaaaaaaaaaatacctccttcttctctcaaaactctccaatggcttccaccctgggtcatcaacatggcctggaagagccgtactctggatacccgagggcgcggccccagcgccgcgacgccccgcccctctggctgctccgctctgggatgcacttccgacgccctctaggcttgggagttccgcgcctctcggtgtcgcctggggggcgtgctccggttggcgcactgattcccagttgggtaggggaggcttgactgagctcccacccggaatttcaccttagacctttaaagaccttgctccggcctcccgcgccagcgctaacacctagtcctctttagtggagttccggcggaaggggatggcgggcacccgacggtggtctcctcccagatggcgaatttc

SEQ ID NO: 68 - DNA, 721 bp, Homo sapiens
aataagaaagttgaggagcaaaacgacgtgtctaacgtcacacattgagctaaagacagatgggatctgacatgcattgtcagcacaaatacagcgcttttaaaaatcatacggattttgtgtcgtgaggcactcaggactcagctgatctcggcgttcagtcgtgcgtgattttggatttgcacctcgcccttgggcaagtgcagaatcctggggttatacaaagcacatcacagttaacccctttgtcccagtccgcagaatgagagctcggagcccggccatgggtggctcggttatataggcaggaaaatcaaggaacccaggtgtgagcaggggcgtttgtggcgcggagagagctcctgtccttgccgtccacctatttctcaggcttggcccctggcgtgtagaaaaccgcatctccggaaaacccagaaagttacgtcgcccaggtactctcttgtcattctccgggatgtaaaagactcagggtctcttcacggatcactgaaaccgccttctccgaggcctccagggtgactaaagagagggtgggtgttctgtgttctcccgccggtgtgttcctcttcatgtccaaccgcttgtgtctgtgcccgctagggtctcgggggtttttataggcacaggatgggggcgtggcgggccagggtggtcttgggaaatgcaacatttgggcgcggaggaagaagtgcccctcctc

SEQ ID NO: 69 - DNA, 181 bp, Homo sapiens
tgcattgcattatactatagcagcaactatacttttaaatgattcgaatcttgaggtttcaaactgaaccgtcttgtgccttttgcccggcgggcatttctgcggggaccgcgggtcaccttctgaatttttaccttcataaacagcaaggactgcgctctttcgcacggcgccccgtttt

SEQ ID NO: 70 - DNA, 601 bp, Homo sapiens
cccaccccagctccttcctccctctgtcattggtcacagaacaagtcagtcatgatccagattgaaggagaaacctggagcaaaatggccccagcgcttccccacctgagagggatcagctgaggccccgcccccccatccctgggagaaccgggctggtcactctggggtcggggcggggcacacctgtgcccggagtctgaggtcactcaccggctgaccctggtggtggtgcgggcccaggaacctcaggcccctcagtaacacattccctgcggtcttcgagaactttcctcagggcgcccacagccctgtgccatcttctccacccgcgcttcacgctctgattctcgccgcggctgtggaagctcaggaatcgcgtgtcgcccacgaaggcgccgcggaggaactcagggcccacgtggtgaaggcggagcccggcggccttcaagtacccggggtgcgggcctgggctccgggaacccgcacattgcgggcgggagaggcgcagggtgcctgggacgccgccccgctcgcctctctcctggacgccgtcgccctgcctccccgcggggacacagcctccctcccacgtcccgcc

SEQ ID NO: 71 - DNA, 421 bp, Homo sapiens
gagttcctctttgaccagacggcctatgcattgggccagctgagccctagatcattcctcctttatcaaagttttaatcctctctgaggtcccgtgcactcacctcgcagctctcttgggagcccttcctgactgctgcgtttcctcccgtctgctggggccagctccgggccttggcgtatgccgcctgcttccctttttataggctccacctgcctcactaaacatctttaagcctctgaaatcagaggccgtgtcttgtgcctcttaaccctttactgagcccagcacattgtgagtactctaagaatgtctacggagtgactgacgaaccaggaagatggaggagatgggttcctgcactccctgtgctcgcccctggagagctcctgtgatatggaagagaatcccaggctcctgg

SEQ ID NO: 72 - DNA, 421 bp, Homo sapiens
cgacgaggagggcggtgctgagcccatagcaagtctgtggatgccccctggtggccctaaatagaatggcttcaatggatggaaatttaacgtgctcgcatccccagcacgttaaattacccagaaaagtaagagaaaaagaacagacacatcagaaatgtctctggccaaacctttcaagtacgaatcaaggcaagatatggcgatgaacaagcagagaaaagtggactgcaaaggaagcagtaattaatctgtcagagaagggagggctccttcctgcttccggaccatgttggatgtgagtctagatgcgagacatctattatagagataatagaagaggttagcggaaccaaggatggttcacttttcttctttagaaataccattaatgctgatcgtcttcgccgccgcctgcgtg

SEQ ID NO: 73 - DNA, 181 bp, Homo sapiens
aggacatggagcaaattagcatcacacaaatgacgatgctgcaaatgagcggtgtacagggttggcgggtgttgcaggcaggtttcctgtcgttggcgccacgtgctgcagaaagaggacccctccccctgcgggccgccgctgcgcccgtgcatccgtcacaggtacaattcgcaccgga

SEQ ID NO: 74 - DNA, 241 bp, Homo sapiens
cgtcctaggggacaggtgtccatcctcactttcctgatagaagaccgcccccctagataagcgggcggcctccgtgcccatataaggccggcttgggctccacgccggcctcccgcccgcagcccgcctgcctggcagggcctttgcattcctcccgccagctgtctccccgctaggggcgggggtgtagtttagcccggccctccgggctgggtcgccagggagtagaaagggagcactc

SEQ ID NO: 75 - DNA, 481 bp, Homo sapiens
cggcggcggcggcggcgggaggagacgcaggtcacgcccccttcccaccacctcccgccgccgacggggcgcgcgcgccgaggagcccgggacaggtgactcctagaggactgcgtctgcgcctcccccggcgggagtcccttcttcgcggcctctgccgccccctgcgtcccctcctgggcttccgagagtctgactcagccaagccggcatcgcttcgcctcctacaacacaccccgagcgcgagaagaaattacaggattgcaggggcacggctaatgcgctctaattacccaccgccgctgtcatccgcggcgctccgcggcgctgggccaacgcgccgtaattaagacgccgctccccggtcccggaaccctcccttcgccaccctccacccacccacctcgcggtccccaggaccactggctgccaactcctgccgccctctgggactgcccctcagtcccaggagagctatgag

SEQ ID NO: 76 - DNA, 721 bp, Homo sapiens
gcgcgtgcacacgtggtggcttttatttcttcgcacgtgttcgtggtcttccttctggagcctctcccctcccccagccccacttctctcatctctacagcttgaaccttttccccgaggacacccaatgaactgcccggtagcttcaggctcccggggcgagagccaggcagacgcgggacttaggctgcgcggataattgggagcaattaggtcccaagatacgtaaacttcaaccgaacggggcgcccgggagctagggaatgcaaagggaggacaggcgcccgtgtgaggcttgagagtatactggagaggttaggaggtgatggcggggtaggacggggagaagtgagggggcatcgagggctaggtcctcagtcctaggggcggagtaggggaagctgctacttggagagagctgctaggttttaagcgcgcccggaaacacgcctcgccaccacccagccaccaccaacggaaaatctgtcagtgcatgtagcccttcctgccacggagaaggtggccaaggtctagaggaggccagcaggccaggcgaagcaacgctcccgcgctgcagggggcggggaggcagcggggaacctggggcgcaggaacgcgggcggaggtgcgatagcagaagcgcaaatgggtcgcctctgacagagatcgggcagtgggttaagtccccgtttgtggcgcggagtcaaagagtgtgtgtgtg

SEQ ID NO: 77 - DNA, 1021 bp, Homo sapiens
gggcccctaaagccactcacctcgatttctgcggatccaaaggtggaaagacactgtcccgatcaggagcatcgcaagggtctggagaaagggccatccataaatgaagatcaggactccgtattctgagactgtttcaatcacaaataagactcggaacagcctctggaaggccgacagcatttcgcgtttctggcctgggaaagtaagggtgcgctaaggcacgagtagtacagctcctcccgccaccgcagagcccgccggcgggaagagaccagacaccgacggagaagcgaagttcaggacgcgaaggaaagggccacttcgggtcggggtcaacccagactggaccaatgcacagtctaggtggattaacgcgccaccgcgagaagtgggcacgggaccacatgcggctggcaagacgtcccagggctcaagctccaggctcggtcaccaaacaacggtgataacatccacaacgccacgtaaaccatctttgggccttgatcgttttccaataaccgactgaactgagggcgtgaccaaacgacaagaaccggaggagaggacccggagaacggagcagcatcccgccgcccgcctccaggaaagcccgaggcactgtagcaggagggtctgggctccgcgccttaattacaccgccctggacccgcctcttccgccgctcgctcctctgaccggcacccgaaggtgctgtcccgcccacggactcgctcacactccgtttcttcgatcctttagacgactttttaccgttcagggatgctctccgttaccgcctctgccatttggttgccctccctgcggtccaagggcctggaacactccccagggctgccaggccagcgctttccaggggctccagcctacagcgccgccacctggggctggagccagaaacgcaggggccgggggctcaccggctgccaagtagagggcgtcgaaaatggggctgggtgtgtaagaatgcttgtgatttttgcacactgattttgtatcc

SEQ ID NO: 78 - DNA, 1176 bp, Homo sapiens
gatgaaggagctagatagaagaaaagattagcagggttctgtcaaagcgaccaggaggctgaagaaacctcctgtaccttcagctgcccctgaagccctccttcctccccagcccgctctccatacaaaataggactaaatgttaaaaggaatcctgtgcacggggaagagggaggcgagctcgggagatgtgggagcacagggtggggcggctcctgcgaggagctcctggctgcacaggctccatctgatatgtcagctcccgcatccgagagctgatgagagatggagggagctcagaagaaaaccctgcgagtgtcgggggaggggaggccttaacattcggatcagattaaccagtgctcaaccgcagtgcccgcgccggcccctccgctgatccgcagcatccgaaagccgcagggcgcgggggcctgtggggccgggcccgggagctgcgagaccaggggccggtgaccccccgcgggggaccgagcgaggatggggaagtcagcggctttacctgcgatggaccaggtccagcggtagaactctaccgtgtcgttgagtgccgtggacactacgtttaggacactacccggctccgagtccaggagccccatcgcggcgatgagcgggcgctggcggcaggagaaagcggagacccagagagagggctgaccccggaggcggtggcggccgacggggcgagcggcggccgggaacccctctaacggcggcggcccggctgcgtcttctcctgctcctcaaggcgccgcggcggcggggatgcggcagaaggcagggccaagcggaaggcgtcgtcaaggttcccgggagaaagacgaggaggtggaggaggcccagccgccagcacagtgcgctgcaccagtctgcagcctcgcgcagccgcccctccaatctcctcagccggcgtcacgtggccgcgcgcgggggcggggggccggccgcccctcctccctccctccctccctagtattgggactcgctggcgtagggatgctgcgctcaagggtgcgacgccaactgggctcgcgcaggcgcgcgccgtcgagcgggagcgggacacctgggctcctccttggcccctccccgcacaagtcgcctcattagccttccccgcccctgtcccgggcatcggcccctgcggaggagttc

SEQ ID NO: 79 - DNA, 901 bp, Homo sapiens
cagcccctgcggtcctcaaagttggccccctgggagggggcggcagggagcaggatgaaggatttgttgtaggaggaggattcacacatctgggcgaagggaggggcagcgccgctgctgggacgcggcgcggacccgcatcattgcgcgcagcagccgctgcagcagccgccggggaccgcggagccgggacgcccccgctcggcccgcgccccgctccccgccccacccccgcccgccgggcccagcaacgcagggtgcctaggagccgcgggctgcgcagggaggcgggcagcggccctcgcgcgcttctgccgcccccggagccggcgcgcggcgagcgcagggcgagcgcgcgtcgggcggcggccgcgctggggggcgtgaggcgagcggcgcggagagcggcaggggcgaaacttcgcgggccagatgcccgagggcgcggcggcgctgccaggctgccgctgctgcccctgcgggccccgagcgcgcctccgcaggcggcactgcccgcggcgcggcgtgtgcaccgagcgagtgaaggtatgtgtggcgggcgcggctggagctgccgccgccgccgccgccgcgccagcaggtcctaatgcctgtcacttcccaggacgctggcagcagcagcagcccggagcccccgagccctcggcaggtttgcgtgtccttccccgcgatctgattggataaagtgggggctcgacggtggccgacgtgggacagtctggctgtggcaggggtctcggaaaccatgggttattgcagtggcaggtgcacgcttatctttatctgtggcatgcaactggtaagtgacacttgggtccccttattctgtaatgtgtctttgagatagtgggcaggggagtgcagcaaagggtctgccatt

SEQ ID NO: 80 - DNA, 541 bp, Homo sapiens
actgccgacttctatagatcaaggacttcattggtgcagctgaggaaattcttccaaacaagtctaaatgttggaaatccaccaaactgcagagaaagacctcttgcctccgtattctttcttcatctgtaaaaatgttgacttctgcttttcagactacgcgcacagcctctttatttcctactgcggcttcattccctcacggaacactgacgccatcgcgaaggaagcatttcgagcacgactgacgctccccttattatttgctaagccgctgcgctcgggtctggctacgatttgctttcagaataacgggaaggtgcaacaagatcgcttccctagaggcgcgtcgcccgcgtggcccggaccccccacgcccgcccgccgccccgtgggtgcgcacgcgtgtccgcgcaggcttcccgcctggcgagtgcaaggctcctctccgccgtgctgctttccagcctctcagcaaatcacgaacaccgaaagaagccacggcggcgacgggaggggcgtcgcgcgtgcttccctcggc

SEQ ID NO: 81 - DNA, 301 bp, Homo sapiens
tggctcaaaatattcaaaattttttccagagtttggccttttcttcagcactgggaattgtgatccaaagcttttcctgatgaggcacaaagttggagaaacaaaacgcaaactaagcaacaatgaaacagaacagagtgaatctgctgtagctcaagagaggacgtagctgcccccactccgcatccccgggctcgggtttgccttgctgacctctgctgccacctggtgccgcacagagaaactgaggagaaaccacatcagtctccttcagcctcagcttcacatctgtggtgggtca

SEQ ID NO: 82 - DNA, 541 bp, Homo sapiens
gggcgggagggttggggtgtgggtggctccctaagtcgacactcgtgcggctgcggttccagccccctccccccgccactcaggggcgggaagtggcgggtgggagtcacccaagcgtgactgcccgaggcccctcctgccgcggcgaggaagctccataaaagccctgtcgcgacccgctctctgcaccccatccgctggctctcacccctcggagacgctcgcccgacagcatagtacttgccgcccagccacgcccgcgcgccagccaccgtgagtgctacgacccgtctgtctaggggtgggagcgaacggggcgcccgcgaacttgctagagacgcagcctcccgctctgtggagccctggggccctgggatgatcgcgctccactccccagcggactatgccggctccgcgccccgacgcggaccagccctcttggcggctaaattccacttgttcctctgctcccctctgattgtccacggcccttctcccgggcccttcccgctgggcggttcttctgagttaccttttagca

SEQ ID NO: 83 - DNA, 181 bp, Homo sapiens
gaggacagaagggggcgctgccgggccagtgcggaggctgcagccgcccactgcagaacgcgcccttggttgggtctggcgagctgcccgcgtagtggagtggtgttagggctcccaagtagaaagaacctgttccctacgtaggtgtcggttgtacttaagagcatcatttggtcgctcg

SEQ ID NO: 84 - DNA, 481 bp, Homo sapiens
ccaaaaaagagttcgcggcggggctctccgagcatgacattgttgtgggataatttggcgaagggagcagatagccctttctggctgacatttcttgtgcaaaacatgctgaatacgattagcaatccccccgcaccgcggcgggcgcccgcagccaatcccgagccagagtttccgcgcgaccactcccagtttggtttcgtaggcgcggggccgctctccgagggcgccctcagagcccgcgattgatataaatatgtaatctgtattgatgggccaggagacgcaccccgacaccttggcccgaaggccgggagctgtgggggctgccccaacgtggctggtggggggcctggccattgggctcgccccgcccctacccggacgtgagccccataccggggtcccttagaagggcccttgggccccgcgcagttaacaagtggggtgtttatggtgcgcgcccagtctgccttgggtg

SEQ ID NO: 85 - DNA, 181 bp, Homo sapiens
gaaagcggatccggttggactccagatgtaggtagagcaggttgcccaagggagcgaagaccgcgtccggcagcgcccccagggcgttcccgtccagccgcagcttgactagactctccaggccctcgaaggagccgcggcttaggcggctgatctcgttcccgttggcgtagaggatgcg

SEQ ID NO: 86 - DNA, 301 bp, Homo sapiens
ccactctttcaaattctcatttgtagctcccggaactcagaagacagtcgacccccaaaactgtccaggaagtaatcggtttccggcttttggacaatggtccctcgcttaacgaatgctaacgaatgctcccttagctgggagctgcagggaccggtcccggcaggtctaaccaaccgtccgcaggcgccgtggtcgagagcagagccgagacggcggggcagggtgccaagcggagggcacagcctggcagccaccgttggcggcaggagagaatgggagaagggagacccgcttctca

SEQ ID NO: 87 - DNA, 301 bp, Homo sapiens
cgggactattaacctggaaccccaagagggggagaaaagcggacaagggacacgtttcctgcttcgagatgaaggtcttgttggctgggtgccctggcctgcccgggcggacgcgtgggacctgcgtggatggcgcacgctgcagccaaacaggctgcccgagggctcttcctgagcgcagttcctccggtgtttaaaaacaaactcaaactaagtgagagtttctctttggaatcgcttcacttgggaaaatgatccagccttccaccagcaactgtgcactgtcccctctggtgactgc

SEQ ID NO: 88 - DNA, 181 bp, Homo sapiens
tccagggacgtgaagctgagcgtacagcgggcgctcccagacactggggaaagtgctttacgatgtcccgagtccctccagtctcgccagcggggcgagcgtgagggtgccccgaccgaccagcggccccgggtgcagggtggcgggcccggcggcgcgcgtccccctccccctcctggcg

SEQ ID NO: 89 - DNA, 181 bp, Homo sapiens
ctcacctttcctggggctgcgtccccgcgggacgccaggttcccggtttcttctaggtcgccctggttcctggcagctcctggtgccacgcggtcctctacggtctcctctgacctgagagggacagtgagatggggctggcggggatgggggtccccgcgctgttggaaagcagcggggc

SEQ ID NO: 90 - DNA, 481 bp, Homo sapiens
gtgctagggacccgggggagggcaaggacgtaaaggaaagagacccctcttcctcaggatctgggggttcatttgtagattctctcaagcctacaatatgggttctcccctcctccgccactagtgctcgccctttcgcgcgcgtgggggacgggcgaggggacccctcggcccccaccgcgcaaggggctgcgcggctgcttgggccacttgttattttttgcgcacaggcttggatattgggcgtttagtcagtaatttagctttggaaattggtgaaacgttagactgtgccctggtattgtttaacgtatccaacctaaagggaagtgggacagttaccttgggacctattgttcggtacttcgggtcctggaaagcgagatttgggtgttcagtctcgaggtctctgaatcttcccgctgctggagagaaatgcgcgctgtggagttgtctggacatttaggaatgtctctcgaac

SEQ ID NO: 91 - DNA, 181 bp, Homo sapiens
ctgcaaactgtgtaagagggagaggaattccccgccaagttgaaaagttgaacctgcctcccaaactttctcctgtagtccagacggggacgccctgagggagcgtttgtgtcagtaatgggaaatctgcaagctagacggaaatgacctgctagtgattgcgctgtaaagaagccggaat

SEQ ID NO: 92 - DNA, 1321 bp, Homo sapiens
ctagaaccctaaaaactcctttggcctccagaaagaccccggtgcagctctctaccctaacccctaagcccctctcaagtgagagcctctcagttagtactcagttgccacgtctcgcaggaactttggagcaagttttcagctcccaggtgtccaacctttaaaaggaaaagcataataatactaacctttctttcacgaccacgcgaaacgcaaaggatgtggagtggggaggggaggaaaaaaaaaggggcggccagccaaatcaaagcttgggagacattttgacagtgcgcttgaaataatgctcttaatttttggaaggttttcaagaagggggtggggggcacgtgggagaaccacaactttctcctgtctgtcactcaagcggccagagagggctccaacctccagctcccgcggcaacacacagtgggaaattgcttcaagatacagtggggctctattctttctctacccctgccccgcctttcccgagcagtgaacttcacagagagggtggtaagggagggttatcctgggtgtcaaaaatctgtgcatagcctgagatcagaagagttaaccccaggccctagacccagcccagcggccaaactggcaccccgtgctgatcagcccccgcatccccatatctgcatccccatatctacctccccagtcgggggtggtgaggtttgggggaggggggcgacactaccatatgcatccaccacctaagtccagcccaggctggcttcaatgaaagctggcaaatccggcgaatctcgcagaaattttcttcgaacttaattcaattttaaagtggatttttactattaaaaacgctgccgagcaacacattgaattaatctgactgtacggttttaattacagtgagggtttctctacaaatctgtacaagacagtggctggttcttggaggatctctgcctcctgaattccattatcgggcccctggttccctgcagacggcagctcgtgggagccagctgcggtgcgagcgttcagtcgccctctgcttctgccgggcctcctggctcctgtccctcctcccttccttcatcccagccccatggagagcccaggattcctgcctgtcatttgagactgctgaactgatatcctgaaacgctacccttgctttttaaactcttgggccccagacttttgagccccctgagcatcgttcttaaagtggctcgttttgtctgggagggtgacctcttgtgtagtgttttttgaagggttctcctgcttcgacttagcagctgttagagtgggcagcgtgatgcccagtctg

SEQ ID NO: 93 - DNA, 421 bp, Homo sapiens
tatgattttctagaacagcaaaacacagtagtcccaaaaaagagagtaagagagagcagcccatctaatagagtgtcccggaggccagcgccagcgggtgctgtaaggagcccggcggcggcaggtgggaattgattgagctggctgcacttgtgtaccaggatgcagagttctccaggtagctggacgctggggactggttggaggtcggagggtgggcatgagggtggtggctgagcgagcgggacgagccctggggctcccacaccgctggagactgcggcgagttacacgccattgggtcgctggagctgggactgtgctccgggggcatctccccgtttttcatgatcttcttgatcttggatcttttgttctgaaaccagattttcacctgagttggggaacaaaggcacacgtt

SEQ ID NO: 94 - DNA, 781 bp, Homo sapiens
ctccactaactttattctcgctccctggaccaagcgcatcgctggggccagggttgtcatggttcttgtttccaaggccccttggaagaaggaaagggatgagaaaggtgcgctggcgggcgcacccggcggcggcgagcgcggaggtgctgcggtacctaccatggtattcttgtcccggaacgtagtaggtggggttgcccgcaatatgcagggaaatgagcacctcgccctgctccccatccccttccagctccccgtggtgggtgcacaggaaaaagaagggcgaaaagcgggggtaatagccagccgccgcgcgcgccctcagcgtcgcccccagcaacagcgctaggaggaaagtctgccgggcccagccactgcgctccatgccgccgccgccgccgccgccgccgcgcgccctacgcgccgctcgctcattcagttttggagacgccgggacggaggagccacgcggagagaaggcgagaagaaggcggacgggagcggaacgggctcgggagcgggcctgggagcgggcccccgccgagaagttccgcgggagacggcggctcccaaagttactttgggccgcgggagcgcgggaccggggctgcgggcgccgagagcgcgtcgtctgccgcctccgtgcgccgccgccgcctctgcgcgacgcccctcggccaggcctgggaaagcgcccgccccgctccacaccttcttaaagccccgggcgccgcgtcccccccgccgccgccacacgtgtcccggccgctcccccgcc

SEQ ID NO: 95 - DNA, 181 bp, Homo sapiens
gggctctgctcttctttaaggagtcccacagggcctggcccgcccctgacctcgcaacccttgagattagtaacgggatgagtgaggatccgggtggcccctgcgtggcagccagtaagagtctcagccttcccggttcgggaaaggggaagaatgcaggaggggtaggatttctttcctg

SEQ ID NO: 96 - DNA, 361 bp, Homo sapiens
ctaattacccctcttaattaaagtctttagcagttgtttcattgttttggcaagaaaacaggagagacgtgcagttagaaacaccagagcccgagctcacagcggagccgctgattaacacttgaagcatttcaaggacctggcacccgccacagtttggttttcatccatgtttcctccttgaatggaagtatattcgtctataaacatacatacacatgtaaaaacacggaggctccgtttgccagctgtgtacaagtcagtatgtgccgtcaggatgcaaacaatagatacctgtctatctatgattgtaatgcgtttgaggagatgtacattgcatacagctactggatacgttgtt

SEQ ID NO: 97 - DNA, 1261 bp, Homo sapiens
atgtttcatgtcctattgtcattctcatccggctaggcacttctcggggacgctgtgtggtgttgaggttttacagggaaaatgctaaccttggcgcctcctgaattatcaactagctacggggtgcccagatttttctcccgagttccagacccagggcaccccgaggcggcgcctggccgaggagctccgcactgcgccttgttaacagctgggtccgggcaaactcgcgccacctaattctctgccctctaccggcttgagatgcttattcctcagggagggcaagaatcgaaacgattgagaccaactatttacaagtgaggcaaccgggctacaggtgcctcgagggaaaggaggctgggtctgcgctcccacaccttgccgacggctccacgtccctgtctgcgcccgaggtccaccggtctgtgaagcccactttccccgcctccctctcgcgttgtgccgcttggggcgcccgctaggacccaaaatgcggactggtgggccgcccatcaagggttgcccgcggtagggcgggggctcccgtgagctgctcccaaaccccactcgcaggatgctgccctgacgcccagggccaacccggggagccaaggcccccggtctctgcaaggccgaccccagcccgctggggaccctgcaagcccgcgcgtggctcccagcacgccgggcgtccgcggggcgagctgctcagggtcactcggggtccctcgccaatacaggccgcgcggagagtgtgaggcgagccccgggcccgcgcccccacgagcacctaccttccaggtacccaaccccaggatgggcatcttggcgccgttgttgagcaggagacggcttgccatggctgctgcgctccccagacccccgcccagtacggtgcggccttggccgcggcgcgtacctttaaatagcccgtgaggtcggcagaaagggcgcctgcggttggcgcgccgctgcgcgaaggagccttctgattggttgcgctgggggtgccgcggcggccttccccaagggtcggcggggatgcttcttccgcctggtcctagtggcagcggattctttccgcccccaacgctcgcccgcgccccgcgtggcagaaaggagttcctcagctgctgtatctggtgggaaagcgaatgctttagcgaaaataacaggcatcccataaatacatagactagaaataagttttggtttcattaagagcccagaagaatgcctttgttgtccaaccccagtt

SEQ ID NO: 98 - DNA, 301 bp, Homo sapiens
ttgcagcctgttcctgttttttaaaagtatttataaaagctgaatgtcaattttctacttagagttataaatagaagcagatgctctggtttgttgatcagcacgctgtgttcttacaggggaagtcaaagaatccgaagtgtgcttggagcatagaactagcgcaagagggcgctagtgaggcggtgcggcgcgggcggccaggagctagggtttgaaaacagacttcggtttgagccctgaatctgccacttagaagctgtgtgcccttgggaagcgataataatacatttaccaaagt

SEQ ID NO: 99 - DNA, 950 bp, Homo sapiens
actccgcagccgctctcagctcagtcctaggtggaaacgcctgtagcttgcaaggtagcgcctgtggctttctggggaaaaaaagatcaaatgcctcccaagacaccagcgacccaaaccggggatgcagggagctcgcttggcccctttgaaggccgactccgcaataagcagtttttcctttaaataaccgtagtggatttgagagaattttccatggctgaaaagagaaacaggagctgtaggcaacatccctaaatttataataatgcatgtaaacatgctacataccacatatatgtatatgtgcataaatatggatgtggttgggcacatacctatctagacaccattgacttgcctggtcaaagaataagacttagacatttcgtgcctgggaaatggtgcagtttatctttaaggagactagaaaaataagagatgaggctcacgttgcacggatgacatcactagcttttggctgcgcgctcggtgttctcgtctgtgggttttagccaaggctgcagctacccgcgccggacgagagagcgcggcagcagcttcctccggcgcccgcacccgggcaatgcgatttccccagtcccctgggcgcagcctgggctctcgcgcctcccgggcaccagccgagcctgcgaggcctcggagccgccgcggctagaggaggaggcgacgaggggaagccgagtgacccagcctccctcccccaccctctccccattcatctcggcgaccaccgcgcgccgggagccggatcgtgggacgccgaggccaggacgggattctctgcacgctgtcgagtgagccggcatctcggcgcccgggtgggctgcgaagaaaatggtgcaatctgagagcgactgagcccagctgggcagagcagacggggtgccagagtgccaagggctcaggtgcctggagaaaggggcgga

SEQ ID NO: 100 - DNA, 344 bp, Homo sapiens
ggagtgcggagcgcggtggtgcgagagggcttggagggggcgctcaggcagggcgtgggtttccctcagattcaatgatcctgctgggctcggtggagcggtcggaactgcaggccctcctgcagcgccacctgtgtcctgagcgcaggctgcgcgcagcccaagagatggcgcggaagttgtcggagctgccttacgacgggaaggcgcggctggctggggaggggctccccggcgcgcctccaggccggcccgagtccttcgcctttgtggatgaggatgaggacgaagacctctctggcaagagcgaggtgaccgcgccgggaagggctagggagtgggat

SEQ ID NO: 101 - DNA, 421 bp, Homo sapiens
gggatgacctaaagtccagctatcaaaatgcgccgcgttttcagaaaaactactgccacgatttaacctaaaaagcttcatctgtattttctgccacagtttgcttccgtttccttcagtcactattccctggcgaagtctccacgcgctcccgttcgccggggaacttagggtatccgggcttccctaaattgacaagcgggggccggcgccttcgcccgccttcgctggccgccgcttggtttgttcttcttctccttcggggacttctccgcccgcgcccgcgcccgcgccccagctttcgtcccgctgtgcggagatgccacccagctccaccgcaggaccgcggagcgagaggcggcagacgcgctccgggggccgccggtcaagaggaagatgaagggcgcgacgacttcgcggt

SEQ ID NO: 102 - DNA, 301 bp, Homo sapiens
ctcgaggcggtcgggacgctttgtccccaaagtcccatgagaagggaggagggtggatcgaaagcgccaaaaatcaatcagaaatcgtccccgtagtttgtgcgcgtgcaaaggttctcgcagctacactgccagaatagaacgtgctcctccgcttttataccccggaaaaaaggcgtggtcagttgtactcccttcccgcagtcacttccaggcactcaggctgggtctcccccagcacctccaggagggcccaggttgtgtgggtgggtgcatggacggacaggaactggctctttcc

SEQ ID NO: 103 - DNA, 181 bp, Homo sapiens
ggtgcaggagagcacacgctgactgtgaataagtgtgtcagttcttaaggtccagcaacacaaagcgaaaagttagtggaggactacgagcgcgatctcgacagagggcgctgggtggtcagtggctccagcaaccacgcggctggggtgcgccgggaagggagctggatgttttagcctc

SEQ ID NO: 104 - DNA, 181 bp, Homo sapiens
gggcctgggaggctgcgccttcttcccgcgaatcccgaaaactgcgcggcaaaggcgggttccgcagaagtcgcgcgtgacccggggcgccgccctcctcggggcccattcggatctgccgcccgtcctctccagagcgccccctggcgccctctaggccatcttgattccaccgccgcag

SEQ ID NO: 105 - DNA, 1921 bp, Homo sapiens
cgtgtcctgccctcctccctccagcgctgccccaagtgcccggccgccccctcggacctccttttccaggggcttttccgtgttccccgtattcacacgacttctctgcctgtggatgtctcatgaccctctagagcagcgactttttcctccctcattccttccactcccctcgggcatctaagtagcaggaacctgactgtccaaagttgatttgggagcagccggctgcccttctaaaatgatctaggaaaggtgccagtaacataagccgccgcctgctgaaactggcgcttcctcagccactcgctgcggccagcgtgaaaggggaggggaaaggggcattcctggcacggtcaggtgtctacggacagcaatcttagttaattctcaaaaccccggaagatccagaaatggggtgctgacagggacctaacctgtccaccacccctcggtcggtgggactgaaacccatgtctttgagctgctttaccagtttatttccaaaaagtcctcctacacctgggaagggacatagaaagctgatcccattgccagccggatttctttacttaactctcaaccgtggtaaatctaattcgcttacgacctctttccgagagctgggaatctgcagagatgctctgttttctgctgtactaatctcaggcttcccaaagcgagtgcctcgcccagctcctaggggaatccacggagccccaggcgcagggcaaaggatggggcgggatggggacatcgtacctgcgctccgggagccgctgggagtccggccggccccggccgcggggaggaaaagcaacggcttgggctccttatccgtgacgcgcgctcccctgcgcccccggggcctcccgtgggctccgtgcggggacaaagccagcgccagcaggaagagtgcgggcaaaggggcgccgggcttaaggggccgcatgttcgcaagccgggaggagagagcgggagactccgggaggatcccgacgcaggtccggagggtgcgcggcccaagagaaggccagcgggaccacagcgcggctacgcggccggccgcagtcttcaccgcgcgcctgcccttgtctacgtcccgggggtcggctggagctgcactgggactcggtcctcagtgtgccgaagcctaagcgctgcggggcgcggggcgggaacgggaggcggtgcctggggccacggggtcgtcccccaggatgagggcgtgtcccagcgcgcgggaccctcggaagtccgcgctgggccgggcgggcaccagcctcggactcagcgggtctcagggctccctgcgcaacgcctgcctcggatccggaccccgggctcgctctctggtcgccgtccccgggaggacccagtagggtaactgccgcgtcgccccggcggttctccctgggctctgtctcccgccgcctccaccccccgagcctcggggtccgtcacggcttcccctggctggcggggtcagtagaacccgcggcgcctaggtccggacggaaaaaagcagggccggggtgcggcctggatgagcggagatctccgcgccttgggctcaaaggtgcggggtgcgctctgctgccgagcccctgctcgctcaggaacactggccacgccgtcacgccagccgcccctgccccaggtctggaggcccgacctgctctcctaggcgcagcaccgcgttctcttccgcgtgggggagcggcgggcggaagaggtctggggctgggcaccggggacacgcgcccagctcccctggcctccctggggggagtggccggtttcagtgcttccccaggtgaaatcgccaaggttgaccagtgcgcccaaaaaagcagccggctggatttttcttcaaattagggaactcttataaagagttttagtgttaacaacttaaaaa

SEQ ID NO: 106 - DNA, 361 bp, Homo sapiens
ccctgtgtgaaccaacgggcgggcaaggcgctgcagggagggactccaaagacacacgcgcgcagccctcctcccgcccgcagcccttcagctgctacagtggccacagctattccgaggtctattccggcctcgccgccgtggcgaggcttgcgcatgcgcactgggcgcctgaataatggctcaggcgccggccctgcctgcgttgcccgcaggccggagtcccccaccctgctgcgggtttatcgctccagctcatgctcatactcctttgtaccatgggattttacttacaaaacaagttcaacgataaaataattaagaattttaggagtgcaggggccgggcgcggtggctcacg

SEQ ID NO: 107 - DNA, 541 bp, Homo sapiens
ataccccataaatactgattggctattacgcgcataacgtgagatcaaaaggagttcctacaaagacccttaaatcctccagacttcttaagcttaggaaagatttttgcttggttttcggttttctttttcttattttgagcagcagaccagcgtgactccacagtttcaaagagcaagcgtctatatttgtgtgacccggggccgagctggggaaggggaagcagagcagcgctgacgcagtcaggtccctggtgcaggtgccagctccccacagcgcgccgaactccccagtatgagcgaacctcaagtcactgccctcgcgcttgtcgagcgaactctcaaggcttgcaggtcgtctccaggagtcagagaggtccggactccggggattcctgctccgcggagaactggggagcccccgttcctgtgccactctcaggtggggtgactttgggctctgggaaggagagctgtgtccgtgtcacgagggggccccggcaggtggcgagcagcaccgaagcgcgggccaggacgctcg

SEQ ID NO: 108 - DNA, 181 bp, Homo sapiens
aataattacagtcagtttcacttaagggggagatcagcccggtgctcttcggccgccccgggaggaaaagggcggggagtgggggcaggtcggccgggcagtccagcttgcccggcccagggcctgaccaccccggctccccatctggctggtgcatggcgcggggaagggggcgcgccag

SEQ ID NO: 109 - DNA, 751 bp, Homo sapiens
gaatgttgttccttaagagaggattagagtttttccttcccccttttcctgcctatgacatggtgatgaaatgtgaagagctggaaatcacaaagcccaccgaggtggctgcgggtctgcctccgaagttatcagtgtaatcgggcctctgtgtatgcctgcacgtgtattttcatgattggaagattaggagcacggatttgttcctgcaagtctcctcttttgttgtcatgagagtgttatgttaacgcttgtgataacgataagacagaaactattgaaaagggtgcagtggtggtgtgaaggattaatcctttgcttgcttcacatctgaacaggaatctccacacaaatgtcccacatgtggaagaacctttaatcagagaagtaatctgaaaactcaccttctcacccatacagacatcaagccctacagctgcgagcagtgcggcaaagtgttcaggcgaaactgtgatctgcggcggcacagcctgactcacaccccgcggcaggacttctagagaagcccaggatctgtcccgtgccgccgctgctcccctccccagacacctctccacgtctcctacccagggggtcgcatccctagcccttcactgaccccagctcttcccttgctgcagccgcacctgcagctccagggagttaactcttcttctgggggactgagaactgtagaaagccacacactactacatcccttcacaaagagtatatgctagtttcttgtaga

SEQ ID NO: 110 - DNA, 452 bp, Homo sapiens
tgacaggccgagcgactgcagtaggagggggcgggcccggctctcggtccgcccccacgccgggctcggggtgggggctcggggcctattacgggatggaagctccgggtgtcgcgggggcgggaggaattaagggagggagagaggcgcgcgggtgaaaggcgcattgatgcagcctgcggcggcctcggagcgcggcggagccagacgctgaccacgttcctctcctcggtctcctccgcctccagctccgcgctgcccggcagccgggagccatgcgaccccagggccccgccgcctccccgcagcggctccgcggcctcctgctgctcctgctgctgcagctgcccgcgccgtcgagcgcctctgagatccccaaggggaagcaaaaggcgcagctccggcagagggaggtggtggacctggtgagtccgagggagccgagccgggac

SEQ ID NO: 111 - DNA, 301 bp, Homo sapiens
tcagaggattgtaaaccacttaagaaaaggaaacagaacttggggaggcggtggcggcgagagtaaacaactcccagggggcccgtctgcagcgcctaggggaggggagaggccgggagccgcctccgggggtctcgcggggccgccgctgggacagatgagtcggagacaggccaagccggaacctcgctgggtaaggaacaggaccggagcgcgctccgggtgggagaggcttgcgctcctgcagccccttcccagggcctgcgctgactcatggcgcgcactggagcccctgcagtcg

SEQ ID NO: 112 - DNA, 531 bp, Homo sapiens
atgagctacagggaagatggttaggaggacagagagaagaacaacgacgacaaaaaaaaaatgcatgtcagataagaaatacgtcctaaagagacaagtttagatgaggaggtggggcggcgaacatgagtgcggaccgcacgacttagccctgagcgcccgattggcgcccggctcgccgagctcccagcgcgtctcgctccggctccccgcgcctccagggtacagaaaacagagtgttttgtagagctccagggtcctaaaggtggggactggggacccgcaaaagctggggtggagagcacagccctgaccatctgagcccccggagccagggcgtgagtgagcgcctccacacgccacccctgaagcccaccacgcacctttggcagagagggacccacctcgcttactgcgtctccatcggttgccttggcagtggctgtaatccatgcagttcagaatgatgagggcaaaggagaaaaggcgaaactgcatctgggcggtcgggcgggggagagacgcctctca

SEQ ID NO: 113 - DNA, 181 bp, Homo sapiens
ggaatcccagatggggcccagacagtggcaaaagagggaggaagagagggagaaagggagcagcggctgctactgcaaacagttccccttcgcagctctgcgctcagctcgcccatcagtgtgccactgcctctccgtcctcctcctcggagctgggcgcaggggggcgcccgggaggcgg

SEQ ID NO: 114 - DNA, 301 bp, Homo sapiens
cggtaattacgagaaaatacccagtctcgccatcagttttgctaaccggtacttgaaaatgggaaacggggaacttatccaacctccaatttgtcacagttgtatagctttcgtattaattctgtacagacgtgaaataggtgggtacgtagcaacgtgctgggcataaattaagcaacaatggccacgcgaggtctcgtccgccgcggagctccagtggtgggcactgccaccttgccatccctagcccccaccgcccttcgcagagtccagtccgggaggctgacggtgcgctggcttt

SEQ ID NO: 115 - DNA, 541 bp, Homo sapiens
caggacacctggatgacaaccaggtccctgctctggaaaccgttaggagtagaggattctcagagggggtggaggcagggtgtgcgtactccaggtggcttattaccgcggggccggggccgtggtaatttgggaaaccatagtcaatatagctattgttttcaaatagcagactagggaaactgaccctggacaatgtcttcctggcaggcgggaacacgcagaatttggagtgaaacggaaaggggcatggggtcgccaaggtggtgaaacgccgcattaaggcgcttcaagatagctggagttttgcttgggaaactcagagggatctcgcccggccggcacaatggcgtttctgaacccatgcccagcccactgggggcagtccttgctgcttgcagaggccagacgcttcttgcaacttctaagcggcgagagctgccaccttgccaatgactcaaccgtttgcctatgccctctgggctgtgccaccagccgcagccgccctgctcccccacccacccttctccccaggctccgc

SEQ ID NO: 116 - DNA, 721 bp, Homo sapiens
attcactttcaaccctccaggggaggagggggtgcgggtggggaggggagacggctcccagctccacctcgcgcgcggcgcggccagtgcactcggctccgggagaggcgagcagcgccggtgagccccgcagcagcgcacccggccgcggagccccgcgatggagtgagtatccccgagccgcgccgccagctgctctcctctcggcatgttgccatggtgaccgcggcggcaggcagatcccgctcgggtccgcgtccaggatgggtgtttaatttcagccccgtgtgtacgcctggtgtttctatagcagccgccgcggcggcaggaggcaaggggtgggagccccgggtggcgtggtttttgcggctgccccttggctagcagggcctggggggcgagtgaggggagtagatgatgttgctaaggacggaggcatattctaggctttcctatctctgccccaagcttccgcttatcggggagttggccgcaatagccatgacttccgattcctaaccatgtcagcattattggactgcagttaaaaaaagagggagggggtcactgcggatcggaagcaaacgcggttcagtgtgaagcgtgtaatggaaggatgagttagtgggtaatatgagccagggctgcaatgtcctggctactagaaaccatcagaagacccaaaagaattgatttgttcctggggtattggagaaataag

SEQ ID NO: 117 - DNA, 630 bp, Homo sapiens
aagagctgagctgggtctgctggtcctcggactgtccttggctcctctccttgctcttacgcagctggcataaggggccactccttcaatagggaccaccccccggcgccgtcgctgcctcctggcctgctgcccatgcctgcatcgtctctgagaccccttagcaaccaaggacactaactctccaggtgcagacgacgacaccccaggcacagagatggacccgcctacccaagttcacaagagatcagaatcagagctaggactggaatctagcatcctgaggcttgacgaaatcctccttaaatccacccttgccctggaggccgggatcccctaagccaagagaaaagcggtgcagctccagcagctgcaacttcctggctgggctggtccggctgcctggactgtcccggagagtctgtgactggcccgtccagaaggaaagcggcctcccgggccctcctccgttccaatcccttacctctctcgggctccaccaccgtcctgccgacccagtttcaggggacctgcctgtgaattctttgttccaaacccagggagccccctgtctccattgcgccctggcccacctccaggccgttctgccagcccaagctgctgctcaca

SEQ ID NO: 118 - DNA, 181 bp, Homo sapiens
cggggggccctgaccccctgccttactctccgggcccgccgcagtagcagtagcattgctgctggttggtgcgatggggcgagtcccactcgagctcctcgggctggtaggacagcaccatcttcacggcctgcagcgtcctggcgatggcgcccttcttcagcgcgccgcctttctgggg

SEQ ID NO: 119 - DNA, 481 bp, Homo sapiens
ggaggacagaagatgttacactttactcagggaacagaggcgggcaactggccctgtgactgcagccaacagctttaagaacacagtcctttctgcttcaaggttagggagacgttctcgcctctttcttctttgcagttattattcaagaggcttcccccgaccccagtccccagcaccatcctcagagcttcagaccatacattgacagtgagcaaagggggccccaggcaggcgggtctggggccaaggagggcggctcccctgcgcggatccttccctggtggctcccaaatccggcgttttctctgccgcctctccctcgggggagactcggaaaggctgcaaaaatctgggcgcccgttcgctcgcttgtcaagaagcaaactgtcttcacattctccaagagcaacatccctgcctaggaagaggaaggaagaggcaaaataaataaaaccagttaatgttgtagttaacttgc

SEQ ID NO: 120 - DNA, 181 bp, Homo sapiens
ctcagtcacttgcacaacgcatatcgctagtaagcgttgctggtgggatcacactcagcacttcataggcaaagaaaatcccaggagtgccgaggaaacgctgtcaagatgtcaaaaatacgcggtaagacgtcagcccggtgagcatcctccgcactgcggaccgcccggggtcggggtc

SEQ ID NO: 121 - DNA, 301 bp, Homo sapiens
cctcaatgtccacagtcactcgccactgcctgggtctctaccctcggccacctcactgacttacttcttgatggcaaacacagttaacccaatggtggtgttctggagcctgaactgctcgttgaggatgtcgatgttgaatgtgccctcccagacaatgggagccagccaaggggtaccacgaggacatccttcctactgcacatggagagaggcgtgcggtcacatggagctggcagggtgccacccacatgcgcctctggcacacggccgcccccacctggaaactccactcagcttc

SEQ ID NO: 122 - DNA, 332 bp, Homo sapiens
taccgccctgcgcagccaggctggctggcaggctgcagcgggaagcgcctgtgggtcctcggcgctgactgcagagctgggtggaggcagcggaaccaaaactgctgtgtcactgcacgctgcagctgttgccagggtgaccgggtgagtttcccacgcttgcccgggcggcagcgtgcgggccggcgggtggggcggaggggtgtgcagagaggccagtggtgtcgtgccacccgatgcccgggggtgtccactcccctctcctgggtcacgtgaccagggcccctgccctgcggtgttgtggggtgtatgtgtggttcttgggggggtcc

SEQ ID NO: 123 - DNA, 361 bp, Homo sapiens
tggcaacgcagccgcctcagggcagtgtgacttcctgatggtggtgactcaggacaacaaaagcgagaggccctgagagtcaggcgggcaccacagggccttgctgaggcagccggggactcccgctccctctgctgacaccattggtggccagtgagtcagaggcagaggtgccagagaccccgcccgaagggaggagatctgagagcctgcagccacaggctcctccaggactcgagcaccggggccgcacagagagccctttctctcctgggcaggccaggcggggatcccccagcgccctaacctgctctgtgaccacggcaatgtggccttggggatgtgccctgcctctctgggt

SEQ ID NO: 124 - DNA, 181 bp, Homo sapiens
ccgtggtggagttcaagcggaaggaggtgcttgtccgcgcgtgctgtggtctacccagtgtctgtctccggccacagttcgtttctcggtcggtttagtgtccgtgtagccacccaaccgtgtggccgaccattcgcgctttcatttgtccttcgcctccgtctgcgccgtctgtcctagg

SEQ ID NO: 125 - DNA, 241 bp, Homo sapiens
gttccgtcacacgcatttagagccagaagcagcatggcaaatcatcattttaaagctgaggaaaccactagcctgcaagatgacatgactcaggcagtcatgccaccaagataggaacggatatcggtcaccatggcagccaaaattgctgggtcctgtccaaccagcaagtacagaggaacttgagggaaacatggatttagggcaaatcaagctgtggtttgtgggcctatctcctttg

SEQ ID NO: 126 - DNA, 181 bp, Homo sapiens
agggtgaggtgcggtgaatagccgtatccggaaaccgagcgtgccccgggcttctttcccgccgccagaccccgcacagccgccctgggacgtttttcgaggcttgggacctaagacgggtccccggaccctgctgggaaaccagggggcgtttttcgtccctctctgaggccattatcca

SEQ ID NO: 127 - DNA, 181 bp, Homo sapiens
gggagggggcgcagagggtcgcgggggagccggcagtgaccgcgcctggggtgtgtcttacagactcgagttgccgcgtcgggctgggcgcgccgccgggtcccatggagctggaggggcagtggtggcgaggacagctggccgccgatattcaccaagcgcttcgctacaaggtaactcc

SEQ ID NO: 128 - DNA, 481 bp, Homo sapiens
cggcctggctgccccatcaaagcctccaagtgcccccacggggtcgaggaggactcagggttcccctggaatgcctgaagccggcttgcctcaggcagcctgaagggaagaccacacctcgtccagcataaggcggctagcagctacgccgcgcgcggggctggctcccggagctctctgccacccagcgctgtgcccgggaactcggcttcccaggggaggaagagccagcccgcggggctcttccccagcctggaagcgtaggcactcggccgaggccagtggcttcccaggcccgggtctcagcctggctgactgggagactctcccgatagcccggcacatccctcctcacccgctccgccccctccaggccccagaggccccctcccctgacagctgacctccagtgcgcccccaacactttctctgccagctgctggctgtcgcccccacacatcagctcccacctctccgccac

SEQ ID NO: 129 - DNA, 1561 bp, Homo sapiens
gaggccatgctgcaaacccagacttttcaggctgcatctcagatataccgaagtgtgtacccgctacgcacagtgcggtgatgcctggccacctccagcctccagcggggacctcctgcccaggtggagtctgaatgcccaccgccaccagcccacgcgcgcagtgggcgtacacgtggtgacctgcctgcggctgggttcccagctccggctcctcctccctccagctctcgctcggcttcctgcagtatcacgtgcagctgcgctgggtgcaggatggcggcggccgcggcggcggcagcagcggtgggtgtcaggctccgggactgctgcagccgaggcgctgtgctcctgctcttcttttccctgtctcctcggcccccggccgccgccgcctggctgctgggcctgcggcccgaggacactgctggaggccgcgtgtccctggaggggggcaccctgcgcgccgccgaaggcaccagcttcctcctgcgtgtctatttccagccaggaccgccggccaccgccgcaccggtgccctcaccgaccctcaactcgggggagaatggcaccggcgactgggctccgcggctcgtgttcatcgaggagcccccgggcggtggcggcgtggcccccagcgcggtccccactcgccccccgggaccgcagcgctgcagggagcagagcgactgggcatcggacgtggaagtcctggggcccttgcgtcccgggggcgtggcaggctcggccctggtccaggtgcgagtgcgggagctgcgcaagggcgaagcggagcggggcggcgcgggcggtggcgggaagctcttttcactctgcgcctgggatgggcgcgcgtggcaccaccacggcgccgccggcggcttcctgctgcgcgttcgcccgcggttgtacggcccaggcggggacctgctgccccctgcgtggctgcgggcgctcggggcgctcctgctgctagccttgtcggccctgttcagcggcctgcgcctgagcctgctgtcgctggacccggtggagttacgggtgctgcggaacagcggctcggccgccgagcaggagcaggcgcgccgcgtgcaggccgttcgcggcagggggacccatctgctctgcaccctactcctgggccaagccggagccaacgcggccctggctggctggctgtacacctcgctgccgccgggcttcgggggcaccggggaagactacagcgaagaggggatccacttcccgtggctgccggcgctcgtgtgcaccggcgcggtattcctgggcgccgaaatctgcccctactcagtgtgttcgcggcacgggctggccatcgcctcgcacagcgtgtgcctgacccggcttctgatggcagccgccttccccgtgtgctacccgctgggccgcctgctggactgggcgctgcgccaggagataagcaccttctacacgcgggagaagttgctggagacgttgcgggccgcagacccctacagtgacctggtgaaggaggagctcaacatcatacagggtgccctggagctgcgcaccaaagttg

SEQ ID NO: 130 - DNA, 541 bp, Homo sapiens
cggccgagcgcgccgccctggccaaggcgctcaaaatgaccgatgcgcaggtcaaaacctggttccagaaccggcggacaaagtggaggtgagcaagcggggcgggccggccgcccgcgagcggcgcggtctcaggcagctctcggttcattggcctctcgtggggcgcacatactttttccgctcgcggtttctgatcctttcggaggagcgagctcccgctaggcttgcggggagctggaagcaaccgaggccgatagctgggatggggctgaagagccctggctctgttttaccggaggcttcagggctttctggttggcacactctctgccggtgtagacgcggcaggtctattccgccgcttgggcaaacaggcgggttagtgcactccacgcagtccaggctccagggatctgtgagtcctggggagctttttgtttgcgcaaactcttgcttatggaatcctgctctgtcctggagactggatgcagaacagcccgcaccttgttgcagcgctccagccgggctcccggcagag

SEQ ID NO: 131 - DNA, 541 bp, Homo sapiens
catgtgcgtgttttccaggggccgctgacacggggatggaggtgagggctggagaggtctgaagagggttcctaaagtccaagggggtgtctgttgggttcaacccgagacgctgaacgcaagcaaataaataaataaacggtactttccgagcgtcgcgagcggagcctgcagctgcctggagtccgagccctcggtggcggcggcggcagctccctagccagccctggcgccgaaagagccccttctcccgggaagttggcctccccctcctcgcgtcagccagcgagctcgctcagccgccggccctccccactccgatcgccaatccctagccccagtcgccgccctccttctccccgggactcgtctccctccagaggccgccaagccagggggaaccgatgtcccgactggggctgaaacccggttcctgcgcccctaccccctacccgccgcgcgtcctcggctccctcctgggcgtccgctcctctcacactctcgcccggtgcccaggactcgggcgcttccgcaccccagc

SEQ ID NO: 132 - DNA, 410 bp, Homo sapiens
gccgggagaacagagaccaggacggcctcagcgcggaagccctgtccagggcccgaacgtgggtgcgggctgggggcgcagcggcagaaacgcggccttagacgcgcgcggggggccggtgtcccccccgcccccacggcaccgggagccgctcgctcatccatcccgcagaccgggcggtgagatgactccgagccccgcgcacggcggccgcgagcaaacgctccgacgtctgtggtgacgtctcgtattgatttagggacacggggcggctgtggctgtggcccacggctcgtggggagcccgagtctgtgcgcagggaacgccgctgcgtggcctctctcgggcctgtgccgcggaggaaggcggcgcccggggttcggggccggggtctcacgtccgccccctcg

SEQ ID NO: 133 - DNA, 541 bp, Homo sapiens
gtggtgtcgccgcgcaggtccagggtggcgcgtggctgctgagcccccgcctgtgcgacgccctcatggccatggacgtcatgctgtgcaccgcctccatcttcaacctgtgcgccatcagcgtggacaggtgcgccgccctccccgcccgcgccccggcgcccccgcgccccgcccgccgccctcaccgcggcctgtgcgctgtccggcgccccctcggcgctccccgcaggttcgtggccgtggccgtgccgctgcgctacaaccggcagggtgggagccgccggcagctgctgctcatcggcgccacgtggctgctgtccgcggcggtggcggcgcccgtactgtgcggcctcaacgacgtgcgcggccgcgaccccgccgtgtgccgcctggaggaccgcgactacgtggtctactcgtccgtgtgctccttcttcctaccctgcccgctcatgctgctgctctactgggccacgttccgcggcctgcagcgctgggaggtggcacgtcgcgccaagctgcacggccgcgcgccccg

SEQ ID NO: 134 - DNA, 481 bp, Homo sapiens
aaatgttccccttcccttgacgctatagcttagatgggagggagccactgctgaggaaacacctccttaacccaaagacagagggttccccaggcgggggtgtgggaactcggaggtgggggtgagggaaggccaacctccacgcttcggcccggaggttcccccgcctcttcctgcacgactggattccttctccatccgcgcctccggcccggtccctgccccgccaaatccgcgcatcggtttcccatcccatagcgcagataggtagggcaggtacacagggaggtgttcgaatgatccccgtttcacagaagacgaaactgaggctgggaggcctggggactggcccggctgcagcgccgccgttagccgaaggtgggagccggcgcggtcacgcgcatggagcgtggatcgcgacgatttcgggggagggggcaagggcgctccgcaggccctgagccggccggggggtggggtc

SEQ ID NO: 135 - DNA, 241 bp, Homo sapiens
taagtttatcgcgccaacggtaagatgtcgctctggacgcgtgcacctgctctcgcaatcaccgactgcggtcagcatcttccttagagcagcgccccgggccacttggatcccggtctcaatttactaagcgaacccagaggatgccccgagtcctggaccgcagagccgctcgcgagaggcaccggggctgtaaccgcgcaacctcgtgccgcgggcggaggcgagggaggattccccg

SEQ ID NO: 136 - DNA, 481 bp, Homo sapiens
tcgaggctgagctctgtgccgagcccactgtattttcaccggaaaatgcgagactttcatttctacctctcgaatgcccagtctttgagtcctgcagcccccgggtcgcccgggtcccggagccggcgggtgtgaacggggccaaagccctccaggccgggcgtgtcagccccgcccccgaggctctttgcatattcatgaccttggcgggcatgcgcaccgcggcggcggcggcggcggggctcccgggccgccaggcgaccgggcgggccggcgtcgaccttccccgacccaggcatcctcaaccgcggcctcctcctcccttgtcttgatggaaagggcttggcgtcccccccactcccaaccacctgagagcctcgcgctggaaggactttggtaattatttgtttcagttgagctgttttcagtctaggctaggctgagtcttgtaatgagtatggatttgccagtaaataagtcc

SEQ ID NO: 137 - DNA, 478 bp, Homo sapiens
ccggcagggctcctcgcccacctcgagacccgggacgggggcctaggggacccaggacgtccccagtgccgttagcggctttcagggggcccggagcgcctcggggagggatgggaccccgggggcggggagggggggcagactgcgctcaccgcgccttggcatcctcccccgggctccagcaaacttttctttgttcgctgcagtgccgccctacaccgtggtctatttcccagttcgaggtaggagcatgtgtctggcagggaagggaggcaggggctggggctgcagcccacagcccctcgcccacccggagagatccgaacccccttatccctccgtcgtgtggcttttaccccgggcctccttcctgttccccgcctctcccgccatgcctgctccccgccccagtgttgtgtgaaatcttcggaggaacctgtttccctgttccctccctgcactcctgacccctccccgg

SEQ ID NO: 138 - DNA, 181 bp, Homo sapiens
ccagccccggcggacccgcccccggcccggcccagcgtccccaggggctcccggcccaccccgtccgttctggagcgagagttcactccccgggctgactgctccaagccccctttattagaagcattccttgtggaaaaacaggaaacactgacctgtaaaacaaaacgcttattaaaat

SEQ ID NO: 139 - DNA, 181 bp, Homo sapiens
ctccccaccacttggtctgagaggggctggggccggaaggccagggaatctctggtggatttgggggttcatattgctcagggtaccagccgatgcgttttgaggggcgggagtcgaggaattagaatcgcctttaaccctcaagagttgcgccttcagcctcgggatcccagatgcgtcg

SEQ ID NO: 140 - DNA, 181 bp, Homo sapiens
agcccagagtccggcctaccacggcggccactcctcgggcagtgacgacgaccgagacggtgagggcggccaccgctggggagggaggcccgggctcaggcctggaagctccctattggatcaggactgcaggcctgacagtgatgggttaaatctaagcagcatgaactcagcaggggtt

SEQ ID NO: 141 - DNA, 346 bp, Homo sapiens
gtcaccccaccctgcggcacagtgtatcccactgaggcccctcggtcgctcccactcgtcgtgccctcacctagtcaggtcccgcagccgcgcctcctccccgcgcaggtaccgcctcagcagccccagcagccggcgctcgggcgccagggcgcgcgccacgctggtcagcgccgagaacgtgtcgccccgagccgcagccctttctgggtctcctgtcccgagcgccagcaccgccagcagcgccgccagccgcgccccaggacccatagccagcgctcgcgaacttcccctcagacagtcctggccgcgcggcggcagccgctcccgccctcgcctgccccgc

SEQ ID NO: 142 - DNA, 181 bp, Homo sapiens
gcgcaagtccccacggtttccagacggggcgcgcagagcccagctccctactcccacatgctgctccacgatcactgcgctcgggaggatcggggaggatccgggaggactagcttggtatttgcagcgcccacccctcccccactccccctcggttccacagtctcacggagagcgcgcc

SEQ ID NO: 143 - DNA, 181 bp, Homo sapiens
agcgactagagacagcgtcgctccaagaaaaagccgggttctgctcccgggaccgacgccgcgccgccctgcgctctcgccgcctgcgctcgccctgcgctggcccgggtcgctgtgctaatcgccgagctctccccaaacttcctgcatgctgaactttccgagcgcgtgtgggtgccgc

SEQ ID NO: 144 - DNA, 181 bp, Homo sapiens
cgacacccggcgtgccctcgggagccggcgtctgtgccccgagccgcccaccccgccgcgcctgtgacgccgggctctgccccccgtggacgcccgcagccctccagccgtcagagccctctcagacgcaccccatcgcggccccgtccccactgctccgcggagagctccctctgccctt

SEQ ID NO: 145 - DNA, 961 bp, Homo sapiens
gcagggggcggggccgagggcccggggagggggctccaggcgatttcagagtcgcgagtcggggccgggatttcgcagggaaagcccagcggttgcagctgcggcggatccctcggcactgtccgccgcgcgccggggcagcccagggccggcggcagctccgcaaagtcgcggaacgagaggaggcggagcgccggccaagtggtggggctcagcgctggggctgggctgggctgggagaggtgtgcccagggagcctggatcccggtgcccttctccctcgtgtggagcggccagtgcggccagaggcgagctgacggcctggaaagagaaatcaaattgcagcctccccaaagacgctgagttacgcgggcgagccggttcccggggatcgttcgcgagcgcgcagagagccgcgccgcgccgcagagccctcccggggccgccggccagaagcggggcgccgtccgacaggcagcagcccctgggcgcggggttcggccgcgagtgagcccctgtgcagagagggggcgtgcaaggctccgccggcccccccgcagcccgcgcccgacttgggcgccccctccgtcccattctgggagcgatgccccccgctcctcgcaccccccgggaacgccgcgagcatggagaagtcgagtagcgaggattcttcgatccatcggagtccatctttggacagcaaggactcggactttgccaagccgtccacctccggccgcccgttcggccgcggcttcacggccggcgccttctacggcaccgcgggctcccggggccagagccgcgccgaggccggcgttaagaccgacaagtgcaatgcacccaaaggcagcaagtacgtggtgttttacctggacctgtcctttgtgttcctcctagaatttaagaagtgcaacatggccaggggctgcctctgctgcttgaagtacatgatgttcct

SEQ ID NO: 146 - DNA, 781 bp, Homo sapiens
cctaccccacggcgtaggcagcaaagctttataaatcccccttctctgagagactagaagcagcatgcatctgacaattgtcaatttcaaaacaaacacgctccgggacttgaacgcagcggggcattcagtagcgaatgctgtctccttgagttagggcaaagcctgcgtgcccgccgtcccctcaccacttcctcttccccagcccccacctgagagcagacattcggaatgatgtgtagtgcgaggcggctagcctcccagcagaaagccatccttaccattcccctcaccctccgccctctgatcgcccacccgccgaaagggtttctaaaaatagcccagggcttcaaggccgcgcttctgtgaagtgtggagcgagcgggcacgtagcggtctctgccaggtggctggagccctggaagcgagaaggcgcttcctccctgcatttccacctcaccccacccccggctcatttttctaagaaaaagtttttgcggttccctttgcctcctacccccgctgccgcgcggggtctgggtgcagacccctgccaggttccgcagtgtgcagcggcggctgctgcgctctcccagcctcggcgagggttaaaggcgtccggagcaggcagagcgccgcgcgccagtctatttttacttgcttcccccgccgctccgcgctcccccttctcagcagttgcacatgccagctctgctgaaggcatcaatgaaaacagcagtaggggcggccgggctcctgcgaacaacaacaaaacaaacaa

SEQ ID NO: 147 - DNA, 241 bp, Homo sapiens
cccaccctctgcctcgctgagctccctgctgcgagggcctcgggtgcaagggggaggcaggtctctatctcatggagctgtcagatgagacatcgcgatcggagtcctcagcctcgcttggcggcggcggcgggtcgctaagcgggaccgcagtgaaagcaggagactttctagaaaaaaacaccagttgtcaaccttggggcaggcaggaatcctgaagacggacggcactcctcctcct

SEQ ID NO: 148 - DNA, 601 bp, Homo sapiens
ggggcagttttgatggctaacccctctttccatcctttgggggaaaattgctcatctccctataggtggaactctaaagacaatgtattcctaaaaggggccatctgggcggtgtcctcttttcccagcgccctgatttctattcttagatctggagataggcggctttcatttttcctgctcccagttcccagaccttccgtggggccgcaggatccccggctggcgggtcgcggagggtggccggccgggctgcgcactgcgcgcctccgctgcggggctccgggcctgtggactcagcggagtccgctgagtcagtttcttcccgcgcgactcccggccgcgccgccgctgcggtggaatctggtcccaggaggcggcgtccgcccggggtccggtctaggcgtgcgtgggggccacggtcacggtcatcccagccaggcccggctccagcagccccacggccgccgccagagttctgcgcggcccgtcgcctcggcggagcctctggcaggcccctgagctcgtttttggggcctgagtgggggaggaggaagccgagcaggagggctccggagagggagggcaacgcggggcgggg

SEQ ID NO: 149 - DNA, 661 bp, Homo sapiens
ctctgcgatccctccagtgggcgtctcccggagcagcgtcccgcctgcccactgagcagctctcagcagggtgagctggcccctctccctgctctgccttttttcaacttcggcgaggtcgggaaggtgagctccgagcttccggaagcactgggttcccaactcaagtatttatgcggtgcttgtttccttgggacgcgctccctcccgccctattgccggaagactgctggttgcctactccccgctccctggagttttattttttcctctccctacgtcggtgtttgtcctctgcatcactgtggagggggtggagctgggagactcgcagattcctcctcacagtaggtgggatcgtggcgctttcccgcttttcccttccaaaaacttggacaactggacgagtcatgccttttctgggctcgtagccgtttccacaagcttccctcactagccttcctcgctagcctccttaaccatgcatttgacttcaacaggcacgctaagcgcggtacctggaaacctccagtccacgcaccggcgtccacgcatctagctcctgcacctgaacctggctctcgacctcacctcctccagtccgggtttcttccttctcaccgagctcacccgtgcagcagtctggcaaattttattcccc

SEQ ID NO: 150 - DNA, 1225 bp, Homo sapiens
ctcgctccctgggggtttggggcaacttccccgctacgtcgcccagggattttaaataattgccagccaccagaaaccccctaacccttaattcttccctccgagacccagcccgctgcttgccacttccctctccaaacgctggcgggggtgggtggcagcaccgaggcgattttcttcgtctttttttcctccgggttttgtcatggaaacgctgacacaacctccagacggcggccgagcccggccggggactgagggcttttgggaccctgcgggagcgcggcgcgcacaccgcactccccgggcaacagctggacgcgaccatatcccgggtaggggcggggggagcgcgacgctccgccccggcgctagggtccctccctcctcccggctctccgcaggcgccctcccctcgccgggggccgcgagttgcatttggtaaaacccagccccggaatatatagatcgttggagcgcaatgaagtagcctttggagagaagggagagggcccgtcggacagccacagcggccagcgcagcggcagcggcggcggcaccaccatcaccgctcgcaccccagccgcccggcccgcgaccaggcagcggcggccgccggcgggatcggaggaggcggcggagcggcgaggaggaggagcaggagcgcgcagccagcgggtccacgcatctcagcacttccagaccaactccggcaccttccacacccctgcccgggctgggggctccgagagcggccgcgaagcgactccgatcctccctctgagccttgctcagctctgccccgcgcctcccgggctccggtccgcgcggcggggtccctgctcctgcgccccgggcgcgcttcccggacaccccggtccccgcagccaggacaaagccatgaagccagcgctgctggaagtgatgaggatgaacagaatctgccggatggtgctggccacttgcttgggatcctttatcctggtcatcttctatttccaaagtatgttgcacccaggtagggggcgcgttagcgtggttttgttggatattttcttctctctcgcgctctagctcgctccgcctgatttctgcctcttccaaccctacctctccgccttcggcctcttcggggctcctggctgcccagagctcctggctgcccagatctacccgggtcaccgcgtcgggatggggaggagaagggaaggtgtgcttcgccctc

SEQ ID NO: 151 - DNA, 181 bp, Homo sapiens
cttctcaggaagccaagctccctcaccctgtggcgacgccgcgggcggaatgcgcatgcgcgccacgagccacaatcgtagggttgggcgcgccctgccggccaccaggggcagcgcaggagctgagcgcaccccatcagcgaaagaagcgcgcctccccgctcttttctgaaccgtatct

SEQ ID NO: 152 - DNA, 181 bp, Homo sapiens
tttctatattgagaacacagaccacatgagtgagagggctcggtaatgctagcgagacggcactggcaagacctgggtggaggaagcggacgtgcgggtgctccctcccagggttcctgcacccatggccttgagcaggggcgtgttcattcccaccgggagtgcagccagcacgaacggg

SEQ ID NO: 153 - DNA, 361 bp, Homo sapiens
ggcaaaatacacgccatatgattggatccttaagggcagcacatcctacccggaaagctgcctacttaacaataccaaaggcttactcaaagaggcacgtgaatctttcgcatggaatacttttggaacccagaccgaagtgcccaggggttaatcacggcgccggtcttacagcaccctcagcggcttcagccctgagactctgcaggtgaaggctcggggggtgtggacgggaccccacaccgcgccgcccgccgactcacttcttgcggacttcttccagcaactgctgtttcaggcggttggtgctcacaccgtcgaagttgtagtttctctcttccttcatagtgtcaggccagag

SEQ ID NO: 154 - DNA, 181 bp, Homo sapiens
atggtttccatagcaacaacagcacaagctgccgggtcccagagacgccctagggtcagaggtcatctccgtggcaacggaaacttcccgcgctacggcggctccaacgggccgcttccgccgcattgcgtagcgaagcccccggcgagccgaggctgggagcgcggtgatggccggtccc

SEQ ID NO: 155 - DNA, 541 bp, Homo sapiens
gccataggttcttttttgacgcatggagcagaggcctcttcttgcctctaagaaggatgaacacttgctctgtccttttccaggctcagcggagcggagaaaaaggtggaggttagcgtccagaggaggtgagagaagagcaagtcaccttggcggcacccccgcctcccctcccgctgttccaacaactgcccagaggctccggcctccgaggaactgcaggcgaggccagacgttttctcatcatcgccctccagctgcaggggcacacgcgttcacgcccctccggggactattcggctttccgatctcctctcctctcccttccgtccaccctttagaagagctcacggagctgcggggcttcccggtgcctgctcagaggccaggcagggcatctccccgccgtgcccgtgcctccccccgggctcctgggagaccccccatctggccttcctttctcattcagacactgtcgggggacgctcggggtttgatgagggagtgaggctagaactttcgtaactagcccaccctgctt

SEQ ID NO: 156 - DNA, 181 bp, Homo sapiens
agggccggggactgtggcgctgcaggctcgagatagcttggacgggaatcccatcggggagacaagctagatactcagccggagcagcagcggcgtctcaggctcgcgtccctcagctcggatgccacactcacctagcttccgggccgggctccgcgctccttccctccctccctcctcc

SEQ ID NO: 157 - DNA, 421 bp, Homo sapiens
ctttcaagtgtccaggccataaattcttctcaattccctctctctctccttgtcggaattaatgagatcagatctgatcagggcgctgatgtgttcagcgccaaatcacacaacagcgcgcgcaccgtaatggaatttgcatctaatgcatacataaatcaaacatctttctggacattttcatatgcataatgtcatttcatccagttctctctgtgcagagggggagatttttctctctgagagaatgactttctttaatgctttcattttattttcgctgactgcagtccgggagaatgcgctcggtcggagaatctttcggggcgcggttgacagttctttttccaagaggggtccttcacatttatcatgcctcttcctcgggggctttgttatgcaaatgtggctgaaattgata

SEQ ID NO: 158 - DNA, 241 bp, Homo sapiens
tccgccctccgcccgcctgcgcccgccctcagcccaagatttctagggcattggccgcgctgctgggtgatccctccgggctcaagttgcaagggggcgggccgggccggaggtggagtctcccgccaattgaagcctccgctataaattgaactccctgcactgctgaagcccagatgcctcgccaggccacgtcgcggttggtggtcggagagggcgaggggtcccagggggcttcggg

SEQ ID NO: 159 - DNA, 181 bp, Homo sapiens
cagggaagaccctcggccggagagccaagtgctgctgggaggtggccgggcgtggccgggctgtgctgtgggaaccgctgggtgggggcgcgctgggttgcccacgctcctggcgcgctgccggcctggagacgccgccgccgccctcttgcaccccgagggcccgcacctcgaaactccg

SEQ ID NO: 160 - DNA, 841 bp, Homo sapiens
ctgcccagaccggagctggagaggggcgagaggctctggcccatgccggccacgtccttgtggtagggggtatagaggttattcatggaggccagcccgcgctcatcccgcatgagcgtgaagctaccgctcacgttgcccgccaggcgctggtggtggtgcgggtggtggtggtgatggtggtggtggtgatggtgggggaacttgtccgagactgtggagatgggaggcagcggctgcagaggggtcaaggtggtgtaggtggtgggcatgctcatacctgggggagtctcgcaggccatggtcatggtgggatgcagggggccggccaggctgtgctcaggggcccggtggtggtggtggtaatctccgccgccgctgccgccgtccagcagggacgccatgcccatggagcgcgggtgcgcggggggcaggtggctgccgcggtgcgccacggagctgcgcgcgtgggggctgccgcccagcaggtcggcaggggcgggcaccggctcatggctcaccccgtgcagctcgccgatcgcttccatggtcagctgcgcgttcatcgtgatccgggcgagcaggcggcggacacaacatcgatgtggccaggcagaggcggcgaggggcgcacggagtccggtcttcacatcggctgctggcgactgttgccttccttcctctcactgtggggctctgtctctctctctctctctctccgtgtgtgtgtgtccgtgtgtgcgtgtgcgtgtgtgtgtgtgtgtgtgtctcgccttccctcttaccccccaccttcccctctgcgtcctcggcttttttttttttaatattaatttccaaa

SEQ ID NO: 161 - DNA, 421 bp, Homo sapiens
cgaggagctagcgcagaccgctctccgccctcagctgcggcgaggcaagggctggcagcgctcggacgcctccgtcttgcccttcccatgcctaagcgcggggaattacacgttcccggtgtagaacagacgatcggggctattagggctgggcggtgggagtgggggttgggagcaccatttttggctggacgtgtgtccagactcatcgtctctggtccttaggaccccatcttcctctgcatctccaggtgtcggcccctctgtacccgcctcccacggggctcgtccggcgaagggcagccgcagcccacatctactccccgccctcaatccctgccccctctgcccgccgcagtcactcgcctggctgggagcaagcctcccctctcgctgagggtgcagagagcgcctagggcgc

SEQ ID NO: 162 - DNA, 901 bp, Homo sapiens
caccagcgttatatcccgtcgctgcttcacatatattatttacctggcccgggtggcattttactttgcatccttgattgggagtctcaggggctacgaacaaacgttttatccccgggtagccggcgggtgcggagcgagtattcgtggggcgggataagtgcggaagtcgctgcgccctcgtcccttcatctccgggggacggccactctcagggttcccgaggagcccgctccgtgcacctaggccctaggtcggctcccaagccctggcccgccgctacaccagcggtttcttacccgcaagtacaaatgtgacacagacaccagctcctcgtgctcttggctcccagggtttctttcaccgcgcctcagcacctgcagcttctccactcttacagcgcccgccgtcgtcaaggcaacagagggatgcccggtgacagactcggcgccggcttccggcgccgtaagagaagcgtccgcgcgggcgttctggacccgcagagttctcggcgtttccgaagctcttggtgtggccgggacccgggagaaggagcagggctggtggggctgctgcagccggtgagtgtgtgctggcgctgggggctggaacctcctaggccagtctctgggcggtgccgcaggaccctgctcgctgcggctctgaggcggaaacaggggctggggccgagcgcgggctggaagctttggtccctggagtgtcgcttccagtctggggccgaggcggtcgcctgtgtagacccgggatcctcaaatagaacgaatccgggaccctgcagaaatgaagggcatgtagtgtagaggtttttcctttttatttagaaaggaatgaaagaccgacagtgcacctgcttggatagtaagcacgtgacccaaaactt

SEQ ID NO: 163 - DNA, 361 bp, Homo sapiens
ctcaaggtctctctctctcagcaccctcgccggccggcgtctgacgcgggtgccagggtctccgggcacctttcagtgtccattccctcagccagccaggactccgcaacccagcagttgccgctgcggccacagcccgaggggacctgcggacaggacgccggcaggaggaggggtgcgcagcgcccgcgcagagcgtctccctcgctacgcagcgagacccgggcctcccggccccaggagcccccagctgcctcgccaggtgtgtgggactgaagttcttggagaagggagtccaactcttcaaggtaactgtctccttccctccagagcgaggctctcccagggcgcccggcgagcc

SEQ ID NO: 164 - DNA, 181 bp, Homo sapiens
gcgcctcttggggtatccttccacggggtggggtatccttccacggggtgaaggctgcggagagtcgcagctgcaggcatggcctccggtcggcggacgctggtgacctggcgtcgtgcagggtgtcactttctcctttaattttttttgatgtttcagtggtttacgaaggtatttgttt

SEQ ID NO: 165 - DNA, 388 bp, Homo sapiens
aggtcaaaggatgagtggcctggctgaacagcccctgctgcctacagccggacgctggtgggcactgaagctgcaggtctggagggagtccgaggagcgaggctgcgtgggattactgctggtgctagggcaggcacctgccatctggacgggagtggaaggaagtcgcggggcagtaatagggggcagcaggcgctttgaggcgccttggggtaagtgccgcagagacccagcgggaatgcaggatggcagggcggcctcggggcggcagcaggcactgcgcggtggcccaggaagacgcagcgcggccgggctggggcgcagggcggcttcggggcgccagggggcgttgtgaagtcgtggcccgctccgggcggtctcaggtgcc

SEQ ID NO: 166 - DNA, 181 bp, Homo sapiens
aggcttgagcgcccagcgacagacaagtgtcctaagaattggtgcctcttctagggaaaaggaggcctgggctccaaggccttaaagactcgcctaattttccgcacggatgagtagacccaggcccagttcggatccgtctttatcttatcgtctgtgtcagagaaatatgtcatatttc

SEQ ID NO: 167 - DNA, 361 bp, Homo sapiens
tcactgttgttacctgcatttttccctgggccagctctgccaccgagtggaagtgggccaacaagtctgtgcccatcgggcctcagtttctctttctgtacaacagaagggttgacgaaagcaaccttgcgcttgttaagaggtggggggcgcggggagcactcggcccggcgggcggagacttttctctgcattgcgatggtggttggcaggccctggggaattacggtacttcgccttcggggacgcccagctgttttggggctttctctctattgggggtaggatgtttgtggtcttgactggaaagccgggacaggcgtctggaggactccccactacatcctgtaccctggaaggc

SEQ ID NO: 168 - DNA, 361 bp, Homo sapiens
gcccgcaggttcctgggtctctccttcaagaccacatcccccagagaccggcggagtttcgcacagccttctgggacttatagttctttaaggacgcggagtgggctcacgccgcgggtaggcaaacagagcgggactgcatttcccagagtgcactgaagacacggaggcgcggagcagggcgggaggaccgtttccatagcaaagacgaccagccgaggatggctggcggaggcgtggggcaggccgcaggaccctcgaaggatcgtgtgagaccccgggcagcctcttgggaggccatttcgaggagaaaaccttgatttctgcctcaggaccctgggcctcagttttcctatctgag

SEQ ID NO: 169 - DNA, 241 bp, Homo sapiens
agtgagccaccggcggggctgggattcgaacccagtggaatcagaaccgtgcaggtcccataacccacctagaccctagcaactccaggctagagggtcaccgcgtctatgcgaggccgggtgggcgggccgtcagctccgccctggggaggggtccgcgctgctgattggctgtggccggcaggtgaaccctcagccaatcagcggtacggggggcggtgcctccggggctcacctggct

SEQ ID NO: 170 - DNA, 181 bp, Homo sapiens
acgccaggcagtggtacgagccgccgccgccgccgccgccgccaccgccgccgccgccgccactgccaccgccgccgccgccggtggggacgtgaagcaccatctcttgcaggttcaccacagactggccgaagaagcagagggacttcaggtggctcctcgctgcctcctcgtcgctgaa

SEQ ID NO: 171 - DNA, 181 bp, Homo sapiens
ggaaagaaacaagcatcgaaagctacatgaagggggtgcagcgctgttctaaaacacaaaatgccgagccccgttttccctttccctccccgctcggtcctgcgcccaccccgtcccgcgctggccactcaggcaagctgtaaatggatataggtaaagatgcaggaggtgatggagaagg

SEQ ID NO: 172 - DNA, 241 bp, Homo sapiens
ttgagagctgggaattgatttctaagcctggtttgagctgagggccacagagccagtgcaggaggagaccctgccccagaaataggccagtgcttgttatgcaggccttggcggttccccgtttccttacgtaacctcagtgttcacgctgtttccttttgttgattccctccgtgtgactgtttttctgtcaatctccttagctaatgagctccttataaggagaatggatggatcagag

SEQ ID NO: 173 - DNA, 781 bp, Homo sapiens
tgcagagtcaggaaagatttcctgagcctggactgagaggccaaggtgggtttgcggaggcaggagagagctccagatcaggaggcagtgtgggccaagccggggggcggcaggatgtgagcacagagagggcagcaacccttctacagaccagttcaattccagtaaccccagcctgccgtaggggtgggggacagcctggctgcagcggggcccacctgccagtgtgtgccttgcctgcgctccaccttccccctcgggcactgcggctttcttgggacagcaggaccccagttaaacagccctgtttcctgcccagccgtggctgccgcctcttctcggaggatttttttttcccacaactcaacaaccactaccacttgcagctaagcagaagggaagttaggactcgcattttgcctctgtagcgcctgtaatcagccccacacagcccccgccgcaggcgcccatcagtgccacttccggagactacttgagatacacctgctcacgctaaaaggagaagcagtaatccatcaaaacaaccccaggcgccggggcgggagaggctgagactcagtttcccctcccatggaacagggcagtgttgggcatctgaagtccccacgggtcctggcattctggaagaacacgactcagtagctttccccttctgggcctcggtttccctgtctgccaaaggtgcagggagatgagctcccagctcatgcctctgggcctcctacctcgcccccaccctcatctctccctttccagagac

SEQ ID NO: 174 - DNA, 334 bp, Homo sapiens
gccccaagtccttcctgaacctctctgggtcgcactctccccagcccctccccccacgccccatcgcatggccccgacactggcagaaggcggccgcccagcctgagcaccttgtgcaggtctgcggccagcgcgcccaccagctcctgctcctgctcctggatcaggcgctgcagcgcctccagctgctggatccggaactgcagcggacgggtcctgcccgagctgaaggcggcgcgggcgcgcttcacggcctcgctgatcttgctcatggcgcctggggacagagagcacctgcagctggctgaggggcacgagcgcgccctgcctccca

SEQ ID NO: 175 - DNA, 181 bp, Homo sapiens
gccttgaaggccgcagcgccagccggctccctccgccggggaaaggagtgcggccagggcttggcgcccgcagctgggcagatcctcggccgctcctgaggcggggacgaagggcgcgacccgctgcggccacagcgggttacgggctgcgggctccgttctgggcctggggagcagattc

SEQ ID NO: 176 - DNA, 301 bp, Homo sapiens
ccatttgcgatcggcacctggaggggcgcgccgtgcacaatgagggcggggccgtggggctccgggtgcgggcggcggccgagtgcccacgtgggtgcaggctaggccgggctgatttccctggaaccccgcgccgcgtgcttccctgtaatgagctcccagggcccgaggtgagcttcctcggctgctcacacggcagccgcgtggcagcaaagaacacggggacttttttcttccgtgcctgacagctcattagaagaattaatttactctagcgtttgcagtttaaaggacattattt

SEQ ID NO: 177 - DNA, 324 bp, Homo sapiens
cgcccggtttggccccggaaaggcaggaagggggcggggaagggatggcgagctcggggtgcaccgcctgtttcttttctggttaggtatcgtccttggagaagatggaagcggagaggcggccggcgccgggctcgccctccgagggcctgtttgcggacgggcacctgatcttgtggacgctgtgctcggtcctgctgccggtgttcatcaccttctggtgtagcctccagcggtcgcgccggcagctgcaccgcagggacatcttccgcaagagcaagcacgggtggcgcgacacggacctgttcagccagcccacctact

SEQ ID NO: 178 - DNA, 721 bp, Homo sapiens
cacccgggggctcgccggccggctccgcgcatcccgccctctcaatggactttcttacctcttaatgtagttcctgccatacaggatctgttgcagcaaggtcaccaaggcaaaggcgcagatgaagatgaagagcaaagttcggctccccaacaaatcccggttggccgaggggtccgcgtagcgcatcctggctaccgggcgccgcgggcgcggggtacggggcggccaggcaatgactcgcggggttccggggccccggggggcgcgcggccgacttggcgcctcacggtgcggtcaggcaggcgggggacttcgaggggcaaagtttctggttggcgcggccggagctgggggcatccaagcgtcgcaggcgctggggcggcaagcaggacagggccggtggcagggagctctgccgcggccaggggccttccccacccccgggtacctttacctccaggcgccggtgccgggtagccgccgatttccccgcggaggggagacgccaggtgccacgagccggaggcggcccctcccgccgaggtggcggccaatggggagcaagacccgggctccgtcccctgtgcgccccagcgcgccgcgcatcgacccctccagtccggcgccggatcgcggttgcccagcgcgctgtgccctgccgggggcgggccacgtttgatctccgggcccgcagcaagggatcgcgaaggttggcctc

SEQ ID NO: 179 - DNA, 421 bp, Homo sapiens
ctgcttctgaccacgcccccgcgcccaccctcttcccaccctcctcccacccagggctctccagacgcgcatgcgcacccgttgtgcatctgccgcgtggtgaccgacacgccgtcggcgccgtccccgctgggccgcagcagcaggttcccgcactcggggtagcgctccaggagcagttgtgcctccagccggctcaccttcaggaagcacctgtggcgggccgcgtcacccactcgggaccccggagaccaagtccgctcttctgcacgtaaaccctgcctcctctgagacccagccccatccccatcccctaggcccaggagaccctgccctgctctccagacccaggcccctcccacggagacccagtccggccttccaggctcctagtttttgtggggttttttgtttttttttt

SEQ ID NO: 180 - DNA, 421 bp, Homo sapiens
gggtcgaagggggcgtgtcttccataaccacgccccctccatgcagcaagcgattctccgcgtccgaggccagtttcctggagggagaggccagtccccctttgggcgcccgccgccgtttctcggcgctgctggagcccagccgcttcagcgccccccaagaggacgaggatgaggcccggctgcgcaggcctccccggcccagctccgaccccgcgggatccctggatgcacgggcccccaaagaggagactcaaggggaaggcacctccagcgccggggactccgaggccagtgagtgccctatcgtgctgccttccccaatcttccccaatgtcctactggtcatatagtgagcatcccacgagcctggtgctgtttatgaaagatctcaggtcctattcacattgcaatttgggat

SEQ ID NO: 181 - DNA, 181 bp, Homo sapiens
gtgcggcggaagccggagctcatactgcgcacggagaacgggctctggctcaaggtggagccgctgcctccgcgggcctgagcgtgggcgcgcccctgcggctcccgagggtccaggccccgcccccaaaggaccaggactcgccccaaagatcccgagggcataggccacccccctcgaa

SEQ ID NO: 182 - DNA, 181 bp, Homo sapiens
tggagacccggttcgaggcccgacaacccagagccaccgtggccatcgggtccccgcctggcggaagtggccaggcgtccacgagcgcggcgcgtataggttcacctcgctcgctccgcagcccccaggggctcatggctgcctatcccccctttacaagaggacaatgaggctacacatg

SEQ ID NO: 183 - DNA, 344 bp, Homo sapiens
cgttccgtttgaaccccatacatcccttcgtcctcgggacccccctccagccctcctcaagcgcccctcgtcagtctggcctccacgccccgtcccctcagcccgccaacctcactgccacgaccctgcgtggcccctgccgagcccgcgggcagcacctggcctgtgcctcgtccaggctctggtcggtgatggccatgatctgctgcaggacgtcgctcgtgtcgaggcgccgcggggcggggggcgatggcgcggggcgcggcggggcggccatgagcggcagggccgggcgggcgctgtgagggtgccgtcgagcctggagcactaccactggcgccgca

SEQ ID NO: 184 - DNA, 181 bp, Homo sapiens
gggccacagaggctgggcctccaggagaataggacacagaccagtgaagacgagacctgaaacgccggctgcagctagagacaaaggccgcgccaaaagcggaaagccgtcctcgtcgctccagctgcgtgcctgattggacggtttccagcccagcgtctctgattggataatgctttag

SEQ ID NO: 185 - DNA, 181 bp, Homo sapiens
agcagagaacacagagcagtgaacaagagatctggagctccagcggcagcaagagacaaaggccgcgccataccagaaagccgtcctcttcgctccagctgcctgcctgattggagggtttccagaccagcctccctgattggattatgcttaaggctctgccccctcagtacctgagtga

SEQ ID NO: 186 - DNA, 181 bp, Homo sapiens
ctgcttgtctctgggacggtgtgtgtgtgtgtgtgcgcgccgctgtgattgtatgtcagcgcgcttcgctgggtgtcgggggaaggtgcgcgtgtctccaggcctcctgcccgagaacagcggcgctgctctctgattggccgcggccgcgccagtgagaagctcccgaatcctgcggtaa

SEQ ID NO: 187 - DNA, 541 bp, Homo sapiens
agaagctggagcggcagctggccctgcccgccacggagcaggccgccacccaggtgagccccgcacctgcccactccctcccctccccgggcctcctacccacccctgacactgcaccccgcctccccaggagtccacattccaggagctgtgcgaggggctgctggaggagtcggatggtgagggggagccaggccagggcgaggggccggaggctggggatgccgaggtctgtcccacgcccgcccgcctggccaccacagagaagaagacggagcagcagcggcggcgggagaaggctgtgcacaggctggtgagcgcctgggccagcggggcctgcctctgatgcctcgcccccttccttccttcctcccaccatgggctgccctgggtgctgcgggcagcctgcacaccccaagccccgcatgtggcctgtggtttgggctgtttgggatcctcacagctgagactcatttcccagcctcttccaggcagggctcgggctggggtgggacagggtccctggcgcttctgtttgagg

SEQ ID NO: 188 - DNA, 361 bp, Homo sapiens
gttcccccatctctccgattttctcctcctctgtccctctgtcccctctgtccctctgtccctccgctgcagctgtgggtgggcatgcctgcctggtatgtggccgcctgccgggccaatgtcaagagcggtgccatcatggccaacctgtcagacacggagatccagcgcgagatcggcatcagcaacccgctgcaccgactcaagctacgcctcgccatccaggagatggtctcgctcacctcgccctcagcccccgcctcctcccgcactgtgagtgtccggcggccaattccagccttcgcttcctcagagccccgcctcttgccctcagtctagccaatcctgggcctgctcactc

SEQ ID NO: 189 - DNA, 356 bp, Homo sapiens
cctctctgagcctcagtttcttcagtggactcaagaatgatactcagtgtaaggattctcaaaacgagcatcagcaggttccgcccacgccggcctcctgggttcagttctctaataaccacctcccttccccgcctactccagccaatccttgtgctgactcggctcctggccacgccctaaccccacccccgctgcctctaaacccgtccccacccctgcagcctcacaggctgccgtcagattctcaagcccctattcctctcggtggcctaaatccccaactgctcggggccacttttcaggccaaaatgggcccaaaatggggagggcaagtgatgaatgtcactagacag

SEQ ID NO: 190 - DNA, 421 bp, Homo sapiens
cagagaagagttttaagcagagaaacgacgcggtgggcggtcggtgtccacactgacctaaagcaaaaaggtcggggccagtacccacttcagaacgattttaatccgaaatggacgcagatctctagaccctctcggagcgacgggactgggaacgtcttagggccacgccgcgagaggaatgagcaggttcggggttttaacctacagggcgaccccaaaacccgacagcggagcgtgggaacctgtggcccgcgaggcgcaggcttgaacccgaaagacggagactcacccgagagcgccagtagccccgcgagatccgcttccgggtcggcaggaacctgcgcgtacgcgagtgcactggggcggcgcaaggggcaagggcaggggcagggcgcggacaactgtggggatgggcggg

SEQ ID NO: 191 - DNA, 181 bp, Homo sapiens
gctgagcatccgcagccgccaccaggccccgcccagcggccgcagccagccaggccgcgcccgggacgactgcagagcgcggtgagtgaacgcggccagagggagggactcaggcgtcccaggtccccgccctgcccctccccgggggcccgacatcccgaccctcagctccctctttttc

SEQ ID NO: 192 - DNA, 181 bp, Homo sapiens
cgaggagaagaaaaaccactactcgtacggctggtccttctacttcggcgggctgtcgttcatcctggccgaggtgataggcgtgctggccgtcaacatctacatcgagcgcagccgcgaggcgcactgccagtctcgctcggacctgctcaaggccggcgggggcgcgggcggcagtggc

SEQ ID NO: 193 - DNA, 181 bp, Homo sapiens
agcggagacagcgacgcacaacgggccgcagaggggagccccattgaggtcgagccgtgcccacctgctatagctggtgttgttgtctcccgtaacccactggaagccgcgcaggggcccgaggcgcttggggtcgccgcagccgggtggcagctgcaggccgatccagaggcgccggcgg

SEQ ID NO: 194 - DNA, 1981 bp, Homo sapiens
agatctgactggcattgaggaaggtcgcggggcccgggtagagcgcgaagcagtcgtgctcgacgcactggctgccacccggctgcggctctgcgggtgcggggaaccccaggccggccagggccagcgcgccaaggaccaggaccccaagcatgttacccaggcgcgccgcgtgcaggcgccggggaaagcgcgggcactgcgacagggccgtgccggagcagaggggcacaggacgccgatggcgacagcctctcctgtccgtcccagcccagacacttcttgccgctgcgcgcagcccctgcgaggcagcctctgacatgcggatcggccagggctcgagtttataagtgcccggccctccctccctggacgttcgggaaaaggaaggaagtgcctggtgggaagggctgatgccgcatactcggattgctgggttctctggccgcccttgcgcccgccctcgcgcatgggatcacctcgccgggatgagtaaaccctgccctggcgcagggaggttctcgggcggggccgacaggggcaggcgccagggaaggccagcacccctgtaacaagacgactgtccccgcccaccactcgggcccccacgcgtgcagccctctttcatctcttggtcctcctttctttcttttcatacatgttacagccacttccaaggaaagcctggattgcaagagctctgggaaccggagacttcagagaagagggctttgaatggggagtgggggaggtggtgcacaggacctgcaagacgctgggaggggtgatcggcaccaagggcactttgggaggacctgcctaggacgtggacttccccgaagacaggatcgcaaggagagacagctggatcctgtccgcggccaaggtgcctggctcaggaaaccagcggagcgcgcttggcctcacaggacagtgggtgtggctggggtgacggggcagggtggggaagactggcctaacaccagcgccctctgccccatggctggccagggacccgcgagtccctggacacgcactggccaacgccagaccccatctcatcgggtggggaagtcgcggggacactgtcagggcgccgaagtccggacccggctcagaggcggtggcaggtgaattgctgcggcgccgggtaggggcgggcgcgtgggagcgagtcagcctggccagtttcggcccagcttccgaaggatggtgcttcttgcaccccaacagagtggctggcaaccccccaggggagcgcgcaggatcccagctgatcccacccgggtcggctaaggaggtttccatttcgtccagagtccgaattgatacccacgtgcatagaaacgccacttgctcggcaaagggcactgaagagccaccgtcctgtggatgggcagggtggggggggggctggaggaggacatgggaatccgtcactttcgacctcttccggtggttcacttaccgggaatgcggaagagtgggtctccccctcgggtcgcccccataatggtgagaggcaaactgtttaaaaacacccttgcctctctcctctactgtcctcacaacgagcgccagggggcggcgctgtcgagctctaaacaaagccaaggaagttggagaagtttcgggctaaaaagggttaaggtgtaggagcacagagtcctccttctggggttggaagctccgttcccgggcagctcagcgtggattccgctgcgttcacctcttgcctccagggcccagtagatcctgggctttaaacaagaacagagagtatggcgtctgccacgtgcgacagacacgcaccggtggggtgggccgggctggactggactgacctgcagtgaccaaacgggtggggcgtggacactctgaaagtgaaaaaggcaagcacgactgtcccgccgcacactccccagcgccttggggcagagagcctccaaacgtcccgctgagttgagctcttcgctgggaa

SEQ ID NO: 195 - DNA, 661 bp, Homo sapiens
ctccagcacccgccaacgtgcctttaggagcacggcaggcaccacccccccgcccccgctccccctactctggggaactacctctgctcaccgccttcccgtggccaaacccaaatatgagttccccgaacttttcaggagcggacgcgctcacgggtcaaatccactcccctccaagggccttaacacgggcgcccagctacctcggagaaaagccagcgggtagggcggaggtattgctctcggtcatcaacgcaaacatcccctcgggtgcctacagcggcctgcttaggggagcagcgtgttcagagcaaatggagagcttcctgtatctccgaggaaaaaagaaaagccgccgccccggcagcctcggcctgctggggacctgtcctccccactaaaagcgcgcgctgcccgaggagctgcccgggagagaacgctccaccccgggcgtcggtgccgctcctcgtctcgccgccccaaacactcaagtggcagattccgacaagtgggaggcagcaagtggaaatattcgcaacaaccgcggaaagttactccagcccggggggccggcaggaaactgaagcggggaacttcgccaaacgcgggctgccgagggacgcgaggggccgggctcgctggccggggcgcgcggggacac

SEQ ID NO: 196 - DNA, 361 bp, Homo sapiens
gtcggaagctcgggggtcgggcgggagcctccggaagggccccgcggagccgggagtccgaggccgcgcgcacgccgaaccgagcgtaccaactccgcgcccggacgcgtggcgcccccccaacccgcagtcaccgcgggctacgccactcccacccggcacacgcgacacccgccgcgcgcaggctcctgcttgcaggtccggccgctgctcgggccaagtaaacaccgggctgggaaagctcgctgcggagccgctcgggggcaagccagccccgccacgcgcgcctccgcggccccgggaagtcaggggcgaccgctgcctgggcagtgacggcccctctctgggcagtgacggcccc

SEQ ID NO: 197 - DNA, 181 bp, Homo sapiens
ctcggcgcacaggtgtctgcgcccaggccgcgcgctaaacacgtttctaattagcatttctttaaacaatgctgatcacaatcttgccaccgtaatccactccaaatgcatcgttgagattgcagcacggaaagcgagagaggaaattcgctgcgaatctcaaactttcttttgtttatat

SEQ ID NO: 198 - DNA, 1861 bp, Homo sapiens
cccgggaaagacctcccaagcaggttctgcgaaggggccccaccgccttcagcccgcctgggtcagccttataagggggaaaggggacagaagtctgcagaacagagatcctagcgtagccgctcagggtaccttcccaggtcaccattgctcctctgccctctccacatccgccctcccgtgagcgcaggatgcacgcacaggcagcggttacaaaactcagcgcaacgttgcaacccgcacaaaaggcgcacacaaaatcattaaaaagaaatacacagagtggaaagaactcgcacaagctccaactcgctaaaggtggaaggagtcaggttacaaactctccctccccggcctaaatgctttgctttagtttgcagaaaatcgtttgtcagtttttttcttggttattcattattcgggcaaatgcaagtatgttttctagctgagttcaccaatccaaacctcaaaccacattcctccactccaggcctccgttctgtccgcggacttatgatcctgcctgccagcaggagtctaccctgaagtcgcgtgggatagataaagtgaggagaggaggatgaatggacagacaaacgagagcaattcttctacctgtgggctgtcctacgccttgcagtgccgggtcctgcggcgaccactgagccccttcgtcctcgccctcagtcccttcgtcctcgtcttcggtctccgctttcccagtcggccggggctcgtcgtccacgaccccgcacgtgccgccgacgtcgccctgccgattccgccgcaggaggtggaactgtagtggtgccggcggcttctcccctggggcggcggtggcgaggcgctcgctggcggcgggcagcggctggatgaaatacgcctcccccagcaggtagaaggcgccgcgcacgccctcgcagaggctgagggcggcagccgagctgggatcgccattcacggtgccggagtagaagcagtgcgccaggtcggtttccggaagcggcgtctcggacccggatttgcgccccacgttctggagcgtgaagccgggcgccaaaaagctgctgtcgggccgcagctccagatccagctgctggtcaaaggcgtgcaggcggaggcgcgtggtcccgtgtcccggggcgcgctccagctccggcaccactagctcctcgtcctcctcggaggggcgcccgagtgcgtccgacacggccagtagcgccgcggcgagcagcagcagcgtgggtactggcccaaagctccgagaccccggagcccgctccgcgttccccatgtcgctgcccagcttgcgccttccgaacccctcgggcacagctcgctgcattggagccccaggagacaccgctcgtagcagcgcacggagcgagggacctttagttcgggtcgggagagcaaagcctcgttggcctgctctggattgttaaaattaacaatttctattattcgttggaagggcgcgcagagccggctacagccgaagctcccggagtcactaaaaggaggcgctgcagttctgccggcgcgcgggaagtttttcttccagcgcaaagttggagacactgagaggcaggcgcaggcagagtggctctgctgggacaagaagcgctctggggcgcctccggggctgaggcaacgcggagattggtgcctggcgcccctcttcggcctccgccttggctgcgatgttgctcactctgctcagggctctcccctctccgtccggtagcgcaccctggctttgcaatagcccctggctcggagccgctttccagcgagtgcaagaaccgggcagccgagcggtccttttatagtggaccagtgaaacccccacccccacccc

SEQ ID NO: 199 - DNA, 781 bp, Homo sapiens
gcgtctgggagagcgaggccgagcaaggaaagcatttcgaaccttccagtccagaggaagggactgtcgggcacccccttccccgcccccacccctgggacgttaaagtgaccagagcggatgttcgatggcgcctcggggcagtttggggttctgggtcggttccagcggctttaggcagaaagtgctcgctctcacccagcacatctctctccttgtccctggagttgcgcgcttcgcggggccgatgtagaacttagggcgccttgccgtggttggcgcgccccgggtgcagcgagaggccatccccgagcgctacctccccggagcggagcacgccggctcccagtactaggggctgcgctcgagcagtggcgggggcggaggggtggttcttttccttctcctccgccagaggccacgggcgcccttgttcccgccggccaggtcctatcaaaggaggctgccggaactcaagaggcagaaaaagaccagttaggcggtgcagacggtctgggacgtggcagacggacggaccctcggcggacaggtggtcggcgtcggggtgcggtgggtaggggcgaggacaacgcagggtgcgctgggttgggacgtgggtccacttttgtagaccagctgtttggagagctgtatttaagactcgcgtatccagtgttttgtcgcagagagttttcgctcttaaatcctgggggtttcttagaaagcaacttagaactcgagattcacctttcgtttccctttccccaaaagtagcgtaacc

SEQ ID NO: 200 - DNA, 361 bp, Homo sapiens
gagaggggcttgtcacacgggcccctgcctgcagtgtgacccttctcagcttctctcagcagccctgcctgcagagtgtcaccaccaccatgatcatttccctgacactgcgagggtcgggggacgtcctgggtagagacagggcccgtggcagcagcaggctcaggggcgccctacactggtgggctggggacctggtggagaccacgccaagggctggacaaggggacgagcctccaccctggcctctccgcaggcctcagcagcccctcccacaggcagaagggttgacactgggttctgccctcactgcaagagctgcaagtgccacgtgctgttctgcccaatctggtgtctgcag

SEQ ID NO: 201 - DNA, 421 bp, Homo sapiens
caacacccaaactaaaacctctcacctgagtgtaagggcgtgctgaccttcttaagcagagagctcttccatcagggggctccctaagggcatctctgttcctagcggcgaagccctcaccccactttgctctgcttagcctgagacacgcaactttctccagcctttactcttcgctgaattctcacggcgggcttgcgggtacgttcaggagcgaggttgggggcccggcccgctgggcgctgttcacaggtagcttggaccagagcaggggcttcatcattacctgcggggacaggtgggacacatgcatttccggggtcatcccagacctcctggaggatgctgattgatgctgtcccgtttgagaactactgtgtccaggtagcagaggcctccccgatgccccttgagtagtggg

SEQ ID NO: 202 - DNA, 541 bp, Homo sapiens
ctaacactgtagactgtagcgcatcgaatcattagacaatgaccattcactttagggaaattaattctaaaattaccgacctcttttgggagagtcgaactgattatcacgtctggcaaaatccattctcacgtgagtgtcgtcgtcgttgtcagaatcttctctctccgggggtcttggcacccggcgactgcgaggtggtggttccggagcggcagctgcagcggcagccccgccagcctggttatcacctctggcaaggtttgcagatgggttgtgggctccagggttcgagccaccggcaacgtcttgggctccccttactgcttcggcatcagcagcattagcaacaggttgaaaccagcgggcagaggcggagtcaaatccagcagctgcggctgctgcgccgatgcccggggctgcggcgagcgcggaggccgcagctacaacttggctgagggctaaagtcggctctgcagccgaagcgacagccggggctgaggatggggaaaggtctctctcgaggctgtctgttggaaaa

SEQ ID NO: 203 - DNA, 421 bp, Homo sapiens
aaggcaagactaagcattccacattcatagagtaaggggacacttggggagtttttaaagatgagtgcttaattatttaaagagaagacatacgttttctcttccatatttataaattactgttcgctaccaaagcatttctaaagatgcgagcgttgtgcagtcggtggacttggcagcgctgtcgcagccacctgtgcggcatcatacagcagcattcaacagatgcttcaagaaaactgcgatgggtttttgcttttcgaaacagaacttgggtgccgacagtatgttcactgccaaattaaatttcaaagcctgaattcagtggcgatggagggaatcagaggattcccaaaatgccccttttggaatagactggacagctcctttcacaaatatggaaacagaggcacagagagaa

SEQ ID NO: 204 - DNA, 601 bp, Homo sapiens
aataagcttaacacagaaagataatgacactcccacggactggcacagaaggccgcgctccgaatgacatcgcgatcacagaggcacagacagcgtcacaaagccccacgcgtactcacaccgaaggctcagccgtcgcgcgtttccctcccaggccccaggaactagtaactagggacgcttctggtctctaggcgaggagagggggagagcgcaatctttgcgcctgcgcacactcctgctcttacccgccggaaccctgggccacgcccggctcgcgtaatcacgcactgcgcaggcaccgcccgctctgctctaaggtccctctcactccttcagcagcccgaggacaatcccctcaacactaggccacgccttgtctccgcccctctcgtccgacccctggagagaggctggcgcctgcgcgatggggggttccagcgtcgactcacggagtccttcggatgagagcgtctgggtgccagacgaggccgggggtttgttttgggtggtttgggagtccgagctcgagggctgggccaggaagggcaggcgaggcgggcggctccgacgcgggtcgcgaaggcccagccgcgtcctc

SEQ ID NO: 205 - DNA, 541 bp, Homo sapiens
ggcgttcggggcggcttggggcggcgggaccactggagtgagctgtgggagagatgggggtgtgcctgtgtgtaaaagatctgtcagagtgtgaggctccgtgagagggtgtggtttctgtgtgtgtgtgtgtgtgtgtgtgacagaccgagagtccagtgtgagaccagggtatgttcgtgtgtgacagagcgagacgggccagtgtgagagaccagtgagtgtgagagagatagggatgtgcctgcatttgaaagagagcgtgtgaagctcagtgagaggttgcgaggtgtgtgggtgtgtaagtgtgtaacagaccaggtgtccagagcgtgagaccaggatgtattcgtgtgagagagtgagacgggctggatggagtgtgagagaccagtgagtgtgagagatgggcgtgtgcctgtgtgtgaaaggccggtcggtcggtgggtgaggctcaatgagaggccggtgtgtgttcgagagagagaagaatcaccatgtatgcgagactagactgtgcaagaacagagtgtgagactgt

SEQ ID NO: 206 - DNA, 1141 bp, Homo sapiens
ctcgtgatcctcctgcctcggcctcccaaacacaacctccacctttcaggccgctccgcccgcaggggcccaaggcgccagctccccatcggtcttcggtatcctcacctaagccctttccagtcatcccggatgggaacttgcagacctgagccagttctcctggggaccaaaatatctcacctcccagatctaagggtcccgccaggagtgacgaaacgttcgaattcctgcgagaaaagtggcaggccaccaggccctctgggaaatgtagtccagagcgggacccacgccgattcctgtcagctcctcgcctgggcccacccgaaacggctgctccctcaactctcaacatccagccgagcctcggagttgcgggtcgccgtagcgctgcgcaatggagatgagcctcccggggaacccggcccaagcctcaccctcacacaggaaagcagatgtgttctggccggaagttgagtggggccgcggggcctgctgggaggtgttgtcctcggaaacgtcgctggcgcggagggatggttcggcgctttaggcgtctgtcacagacctatctgcgggtcgccttcacccagcatctcagaaactgcgcgcgggatgaacattcgggtgtttccggcaggtgacgctgccgagtccccgcagcagggggcgagcaagggactcgcggttgacgggacacggatcctctaaggcccagagtgtcccgagtagcggcagtggggagtgctcagggtacgctaatggtgagtggttgcagttgatgggacaaaaaactgtgatgggagttagtgtgggtgtgtggttgtgtgtgtgagtgtgacggcacgaataatctgatggggtgattgtgatatttggttgcgcgggattatgatgaaatgtgtgatatgtgtgtgattatgattaaggctgtagcgagtgtgaacgtggcgaagtgtgcgtgattgtaatatgtctagtagttcttgtcttgagctggcttttctgtagcatttggcacagttggtaacggcttgaaaaacacttatttgttttctactgatcctccctccttgttggccactcctctgtagtcttctttgctgtcttttttaccctagtagcccttggccctttgtaa

SEQ ID NO: 207 - DNA, 901 bp, Homo sapiens
ccccctggagacaaggtaggggggagcagaggaggcaggcgccgcggaggaccctggccgacctctagtccctccgccgccgccaccggagcggtgcgtcccggggctcgagcgcagccgagtacccgccgaaggctgtccccatcagtgcgtgtctgctgccgggcagcggcagcatccaacctgctttattcctcctgcctgcagcgccacagcgagcgagcgagcgaggagggggagagagggagtctgtctgcaaagtgctgctccctggtgctcagaggcggctgctccagctccaactctcattcatttcgccggttaacatgagagatcatggccgccttcgggcttctcagctatgagcagagaccgctgaagcgcccccggctcgggccgcccgacgtctacccacaggaccccaagcagaaggaggtaagggcgccggcggcctccccggcaaccggggccgcgctctgcagcactgacccggggccaagttggcccagcgggcatcgccggcgctgcggtggaagaggtcggggagggggattagaggcgggggccaggctgggggtgctgggcgaccccccggcggcggagaccgagcggctgtcagtccccgcgctccactggggcgctcgctttccatgtgccggtcgctttcccgttgccgggccttgcacggcgccgccgggcgcttctcgggcttcttccctgccgaaaccttgctcgctctcacccgtttctgcctgctttatttttcttcttgccgcttcggtaaatcgtcgtaaactttttgaaaaatgttggaatgcagtgcatcctacactgaggtcttgcgttttgcttttgctggccagggacgaaggtgagggggaagcttttcaaattttccagt

SEQ ID NO: 208 - DNA, 841 bp, Homo sapiens
aaagttagcccgccacgttgaacccctgtccaagcggcgctatgccaagctctccggcagcctctcccctacccaatacagttaatcttctcctctttgtaaaccccccaagtgacgcggagcaaaacttaatcggtccagggaacccagacacgtcttccgcgccgcacggacttcccagaaggagcctggaggcaggcgctggatccctctaggcacctccgtccccgccggctcccctcccccgcgcccgctgggccactcacccgcgtggggcatggtgatggtctcgttggtgttggagcccacgttgaagatgaccacggctgaggcgttctgcaggaacgcgttccggatcttatccctgtacgtgcagttgcccttggggatgagggctatccagttcttgccgcgggtcggggcggcgaacttggtgttggggtcgcaggccaggcggtcgtgggccgagctggccatgaccacctccccgcgggcgtcctgcttgggcgagtgctctccgtagcgcccgcactccgtcttctccgtgtgcagctccgcgccgccgccgcccgccgccccggccccggggtccggcgcgggctcggcgtaggtgatgttcacgaaggcggtgtaccattcctccttctcggccacggtaaagtccaggcagagcagatgcacgaaacaaaaggaaagcagccatgttgagagagccagactgcagcacgcttggatgagagacattgccatctttatccgccggggccccctccccgcccccgcgccctccctccgtcccgtccctcctccccagccccggccaaccccgggccgctgcctc

SEQ ID NO: 209 - DNA, 421 bp, Homo sapiens
gctttttcagatttgggatcctccccggggaggacctcctggcgccccctggcagtttcccgccgcctagggccgacttttccacctccagctcccgggcgggggaggccccgtacggccgcttagacgggctggggcgggaagattgcagcggctttgggtttactccttgtttcttcataatccctagtggagctgggtcaatttcaggcacagcccatccgagtcaggcgaggtccagaaaggcctgactcgcctggcagcctcaacggacttgtccccgcagccgttgactagccgttgacgagcggacctcccggtcgtcatggcgactgtgaaatgtagggtggagcgcatgcgttcgaagccattcgcgcgggcagtccctgcgtgtccccctgcgtgtccccccacgtgctcc

SEQ ID NO: 210 - DNA, 950 bp, Homo sapiens; identical to SEQ ID NO: 99

SEQ ID NO: 211 - DNA, 661 bp, Homo sapiens
cccatttgccgccctggcggggcagggcgatagggagactcaggccgtcccaccgattggcgcgtgagctgaggcaagaccggagactggtctcccgggctgaactttctgtgctggaaaatgaatgctctgagctttggaagctctcagggtacaaattctcagatcatcagtcctcacctgagggaccttccgcggcatctatgcgggcatggttactgcctctggtgccccccgcagccgcgcgcaggtaccgtgcgacatcgcgatggcccagctcctcagccaggtccacgggcagacggccccaggcatcgcgcacgtccagccgcgccccggcccggtgcagcaccaccagcgtgtccaggaagccctcccgggcagcgtcgtgcacgggtcgggtgagagtggcggggtcggcgcagttgggctccgcgccgtggagcagcagcagctccgccactcgggcgctgcccatcatcatgacctgccagagagaacagaatggtcagagccagggtgggggccggcatgacggaaaggaagcttgtgtagagccccctcaccgccaagcagacccccacacaagccccaggtgtctaattacccctacatttgcttccagtttccaatttccttcttgagttctctatccattctt

SEQ ID NO: 212 - DNA, 661 bp, Homo sapiens
cacagggctgatggtgacgaagtcgcggggccgcgggcccagcagctgcgctcgggcggaggccggcccgggacccggggccgcagccagcttgaggcgcaatgtgcgcaggaagcggcgcaggcggtctggggggcagtccgagagcagcagctgcactgcgccggccccgggggtgtcgtgggcggggagccgcagggtgctgcgcccggcctcggcgaaacgcgtgaagaggcgcgcggcgcgcagaggaaagcagcgcggccgccccgcgggccctggcgcttgcagccgcagcatcaactcgcggcgctcgttgcgacccaggctcagctccgcggtgcgcagggcctggcgccttcgcggctgcccgcccgggctcagctcctccacagccacgcggcaccgcagctccgagtcctcatattcccctgccgccgcctctatgcccgagagcatcgtcaccgcctctgctggtctgcgaagacaccggagcacaggggtcatgaggattcatgagacgtaatgggtgctataggggacgtaatgggtgctataaaggacgtgacagggagcagggtcaaggctacacaagatcacgaggactgtcactggtaacacaaagaggtcacaaagacggagaaagggctttgggctaacc

SEQ ID NO: 213 - DNA, 421 bp, Homo sapiens; identical to SEQ ID NO: 161

SEQ ID NO: 214 - DNA, 601 bp, Homo sapiens
atcctgcagagggcaggagcatgagggagagtgccatccctcagctgaaggccactgtgccttgtatttctggtttgggcaagtgaggagcctgccagcccctggcaggaagtgcacgtgaccggcggctggccaggggcacagagacgcactccacacagaaacccaggctggcggggtgggcggccggggagccagccctgcagatgttactaagtgaaacctgatgtggtgacatgagaatccacagaacgtctcacaaacaacctgccccgggatgttttggattgagttttgtggttatgacgtgaagaaacctcacatgtcaggataaaaataaccctggcttcagtacataacgcgagttacagttcaacagaaccagatgtgaaaacgtcagccacccagttcaggcccagcagggtccctgctccactccggcctccctccctgctggggttggggtccatgtgcccggacagcccgttgtgggctcaagatctgctgcctggaggatacaagggaagggccagaggccgctcaggggaggcagcaccaccttctccgaggccagctcctcttctgtgaaccaggcagggct

SEQ ID NO: 215 - DNA, 1021 bp, Homo sapiens
ggtcgggagccacagcttctgaatattccttcggaacttttttctcacttgattcccaagcctgtcatggggttctttttcaatggcactgacctgcaattacccaacgagcagcgggacagccccgggcaggacgcatcctgggtgggtgacgtgatcccgcagtctcctccccgaccccatatcccatacaatgatcctcgcttacagaagtcaagggggaaagatgacgctttcaaagcccgaatctctttaccctggagccagaaccagcgtcgccgccgtcccctgcagctcagccggcaacgcgcgccgagcctcggggcgcagcttggagacgcgcttgctcgttctgggaaggggcacgggacgcacggttccccggccccagctgcacagctcagctcggggctctcacctatcctcgttcagagccacattcggctgcctcccctgaccacccgacacaaagagattcgccggtggaaagaatcgatttcaaaattcaagctcaccgctgctcaacaaggcgcgcacgtttctccccgtctggcttcacatgtcccaaacttccagtaacagaaatgaggaagcagcagccttccccggctgctggcggaggcagtgggtgtaacttgtgaagtttcgtgctatgatgaatctggtcacttgggtgtgttggagagggttggtcgctcctcccttcctcctcccaccatcacctccctcctctccgcctccctctccaatttaattcttccctctggcattcgccggctgtcactcagaatcccagcaccctccccaccacatccttgggggcaatgtatttcgaaaaggtcttaaccattttacggatgaacctggtcaccctgcacaaagcgtgagtgcttgtcaaataattttctacagcacgtggcaaaaaagcagcgcctcttaaaagatataaaaggccagcaatgttacataagcgccccccaccagcccttcaaggacagaaacgtgggtagttcattcagtg

SEQ ID NO: 216 - DNA, 241 bp, Homo sapiens
gcaagaaacggctcccggctcgcgtgtacgccgacacctcggcccaacgcaggactcgaggtggtttctagtgcccgggtggctgcaagtctgccctccgagggaggctggacaagcggcgcccccaggtcgagcggcctctcgctgcctggcagtgcctggcagcccccacctctgccagtgcttcggaaacccgcctggccaggttcgcccgcggtgaaaaatgaaagcaaattcccca

SEQ ID NO: 217 - DNA, 1021 bp, Homo sapiens
agccggaactttcctcgacgaaggctccctcctgcgcctgtgtctggagaacccccagagcgctgcaagttagcaagagagattcgatggcggctctggaaggcgcacgaagggtggggcgggggagcaaagaggccactgggtgacccagcctggtccggggtgaaacgctagagaaggcgcctcgccttccttatttcaatgcaactcctcggccccagacggtaaaaatagtttccaagctgccgcggacgcccaggatgtgtttgcagagatcaaactggggaggaggcagctttgtaaaagttgcagaaagattagccgagaagcgtccgcccggcggggctcaagaaagcttggggacagctccatgttccttggggcggaatggcccaagaattggcctgggtaaccccctgcccagttctctgtcctcacttcgagccagtgcttaaataacttcccgccgcctgccctgcaaacttcccggcgcggcgccgttgaggccaggacacagcaaaggctagcaaaaccccgccgcggcgcgctcggccccggccctgagaggctgcgcgggtgggaggaccagtgtggtttctgctcccactcggctgcccagaccctcaagaccgatcccccaactcctgggagcgggtgcttccctctgggagccgagatcttgcggggccagcgagggcgcaaagtgcgcgcgctggcccgcgcgggggcggccgcgcgtctctccgcggggcctgtcgccaggccggccgcggcgcgtgagtgatgagggcagagaagggcgcccataaatcgcgggtgtcagggcgaaaaactctctttattgtctgcgtgatggatgggcccggggacgagacaccaaatacttcgtatcgcctttaaatgggaacacattttccgcggccataattcatgttttttaaatagaaagtttgaaatgttgcctatatttcaccagccctgacatatttatgaatcgctccctgcatgcaaatatcattac

SEQ ID NO: 218 - DNA, 181 bp, Homo sapiens; identical to SEQ ID NO: 126

SEQ ID NO: 219 - DNA, 301 bp, Homo sapiens; identical to SEQ ID NO: 11

SEQ ID NO: 220 - DNA, 361 bp, Homo sapiens
ggcgagactgacctggagatgataaggccagttgaagagacactggagaagagaagacagtttgttttacacattgcaggaaatcagattagacagttagggtgtggacacaaaagcgaggaccttgcaggcactggggagaagtgaccccattcaatagtccttggtctccttctgccctgcggctgcgcttcctcggctctcacggcaccagcagaattccatgtgagagggagcttgtcgagcgtggcctcttcccacttggggctgctttctgcatccctgtgcctggctgtgggcctccatttgccctctactgtcttcccttaggacatcatttatgcagagaaaggttcgtgtg

SEQ ID NO: 221 - DNA, 241 bp, Homo sapiens
gggattacaggcgtgagccgccgcgcccagccccctcctcactctctttctcttcctgtaacttctacagctgggcaagagctgggtctccagcggttgcacggagaagtgtgtctgcacgggaggagccattcagtgcggggacttccgatgcccctctgggtcccactgccagctcacttccgacaacagcaacagcaattgtgtctcagacagtaaggggagcgaccggggaggttgg

SEQ ID NO: 222 - DNA, 361 bp, Homo sapiens
tagatggggctgagggcagaggaaggaaaaagaaaacctccgaggtcagtgcggggcgaggtgagcccctcccagggccctctggcccaggaggatgaagcgcgccggcttcgctcttgcacgccggcttgccatccgggtaagcgcgggaaaggcggccacagggcgcggcggcagcgcagcgcgtgggatctcacgacccatccgttaacccaccgttcccaggagctccgaggcgcagcggcgacagaggttcgccccggcctgctagcattggcattgcggttgactgagcttcgcctaacaggcttggggagggtgggctgggctgggctgggctgggctgggtgctgcccggctg

SEQ ID NO: 223 - DNA, 781 bp, Homo sapiens
ctgtcctatcttttttttttttttttttttttttttttcagaaaagatagcctaaaagggttaagaatcccagcaagacacaacatagatgggctgaaaactcgtggcaggatggaagggtataaagacgccggggaagtggctggggaataataaaataagagggaagctaaaccagtgacccttgtcggcagtgaaaagcgggagattagaaaatgtttcatgctaatttccatggagatttctttaatttagcgaagactgcttcccgggctccgcctggcccgcgccggcccgcgtcctcggtggtctgggcgccccggctgagccgctagcgggtcactcgggcggctccgacgtctctatcagccgcgcccgcgccgcccgcctccccgcgctgctgcccggctctcgggctctcgctttttttttttttttttctttccgcggcagtcttaggattcttgtcacatgatggcttcatcgggcccttctcctcctgatcctttcaagctctttctcctgcctggcatatcaaaggagatttgtgggtcaccgagccgggacgcagcatataaagtcatcagcctggccggcaccacctcgatcatttgccgcattgttcttgcaaggagcccaggatggctgtggctttttaataactagcttagtagttagccgaaaaatcttagtttttaaaaatacaaaaaaaaaaaaaaaaaaaaaagagacagtctgatagtttatttgtttttccatacactcttaattgaaactcagt

SEQ ID NO: 224 - DNA, 241 bp, Homo sapiens; identical to SEQ ID NO: 172

SEQ ID NO: 225 - DNA, 301 bp, Homo sapiens
cagggcgccgggacactgcttggcgcgtcctgggagtgaagcgcattgaacccagctcaggctggtggtgggggagtcttggcaatgctctctctccaaaggcgagttgatcacagacgctggcagtgagtcagcggcaccgccagggctgctgagaaatccctcctgctgtccgatcgcattcctggaagggtgggccgctcagggccccccagctccagtcccactcaggccccagaatcccagcagcccaccactcacttctttgcgctcactcttccttctggtccccacacaccgc

SEQ ID NO: 226 - DNA, 349 bp, Homo sapiens
ggcagcgcgcacgggagggagcggcggggggcgggccgggagcggaacagctcgcggctctggaatgccaggcatccaggtcacccgcggctgcaagattaatggctccagcgaggagccaagaacagctcggcgctcactcgctccccggggagcggaaacgcctcccggccggcccccctcttctcacccactagcaagctcccagaaacccgccccatggcttcctttctttggcagagtcaggctccagaagtccgccttcctccacaggcaccctaatctgccgtgcccttgcagcttctcctccccagactcctcagggaaaccccagggctgccccctcccc

SEQ ID NO: 227 - DNA, 412 bp, Homo sapiens
tggatcccaacaacaggaaactacctaaatcaccgaccagttctggtgctgcccgcgaagggctgcctcgcccgccgccgccgccgcctccgccgctgccgccgccgccaaggagagaaccctgccatcgcgcctggcccggcccagcccagcccctaggcaacctgcgcccgccagtgcaacagagtgccccaggcggccgcaaatgcgtcaaggaaggggaagccacaggccccagtaaggtattcctgggagggagagggaggaaaagagagggaggaaaggcagggagagaggaataaaggcggggagcaggcgagacgagagcagctccgagaagcagtgtgcgcgccgctttcccaaatcttgcagcccagcgagccggcgccaagaggcggtagccgtggaaggc

SEQ ID NO: 228 - DNA, 181 bp, Homo sapiens; identical to SEQ ID NO: 2

SEQ ID NO: 229 - DNA, 181 bp, Homo sapiens
ccgccccccagctgcgcggccgtccctcggctccgccccacagctgtgtgaccgccctgcggctccgcccgcagctgcacgttcgtccctcggctccgcccccagttgctcgtcggttccctcggctccgccccctcggctgtgcgtctggccctcagctccacccccagctgcgcgtccg

SEQ ID NO: 230 - DNA, 181 bp, Homo sapiens
gcgggctctgtttattctgtgaccagattccttctaaaagaaggaaggccatgtctgcctgaagcctattggctgggcctactctggacccgcccctcttttttttttcatgacacacaccacagcgaagtctgtgcggaatcctaaaccagcccaatttacatccattcatgaatctgtg

SEQ ID NO: 231 - DNA, 601 bp, Homo sapiens; identical to SEQ ID NO: 50

SEQ ID NO: 232 - DNA, 361 bp, Homo sapiens
aaaaatgatggcgaggaatgcagagggccctaaatggaccctaagatgaagtacgggtggtggctggagagctgggactggaaggtggggctgggggagacgggtaagcagcttgctttggtgaggagctcccacgctgagaacggtgggaggagggaatgatggggaaacctttgtttaatgaggaaacctaattattgcgcatctggaagtcttagtccctactaccagacgaaggcgggtacctgagggatgcagtgcgcatgcccgagccgtcggatttgcatgataaggctcgcacgtgagccaactccggcgcagcccaggctgtgccgcggccggccgccaatggaatcttgct

SEQ ID NO: 233 - DNA, 1321 bp, Homo sapiens; identical to SEQ ID NO: 92

SEQ ID NO: 234 - DNA, 421 bp, Homo sapiens
cctaccttcactgaaggctctcggcagcacctgatggcttgtgagtgtgtttgtctttggtgtatataggttttgccttagtttagaattctctcctgaagtcccccgcaatgtcactgtagccactaacccttggtcacacggagtgtggagccagctgtcagtttctgggcaggctctggccgggaacgcatacaacgtcaaagcagtgaataagcgatttctgcagttcccgtagctgccagcctgtgcagtcctctgtgatgcttggggaccggctcctcggtcacaccccagtcctgctctgaaggttgccgttttccaaacagaaggatggtagctagaggggagatagcaagattctggagtctggaaagccttcacttgggtatgtgtgcaaagaatggattgttgtactgtg

SEQ ID NO: 235 - DNA, 181 bp, Homo sapiens; identical to SEQ ID NO: 152

SEQ ID NO: 236 - DNA, 181 bp, Homo sapiens
tgaccgggggcgggagcagggtcgtggcgtccgaacctccgggctgcagggggcgcggagcgggcgggctggcccagaaaacaaatcctgcggtgtcgcatttcctgcaacgtgagccaggtcgggcggggtgaagggtctgaggccaccgcagggacgcatgggctggagagtggggcag

SEQ ID NO: 237 - DNA, 181 bp, Homo sapiens
ccaacagcacggacttgaaccgggtcgcatgccggagcggacgggatgaggtgcaccgcagaactggggactcctggtgccgggacgcggcgggctggggcgccccactctcggggcaagtctgcaatgcccggtgcccacaaaaaggacacatccatctttgtcaccccgaggcctggca

SEQ ID NO: 238 - DNA, 481 bp, Homo sapiens
aggccggacagggaaagtggcctggggcgaacagaggcggggaggcggggctgagcgagcgagggggatcccccaggagcaggaggagctgggcaaggggggcggttgcggggaggggtggatggttcggaatgggcgtggtcttgccgaatgggagggtctaacgcgagtggttggcgtcccgcgcggggcccaaagtgtgacacgggtgggcttggaaccgggaccttagctactggtggggctgaagcccaccctgccattgttctgccacggtcagtggggcttgctcctccctatgggaagcacttacggccgggagcgggaatcccgtcaccaccgcggtggggaagccgcacggaaatccacggggtgcggacggtgccatctcctggaagttggccagagaaccccactctgtccgcaaatcgctcttatttaataacaactatcatcgattgtgatcctaacctgggcctcc

SEQ ID NO: 239 - DNA, 721 bp, Homo sapiens
gtgcccttaccccttaccctcacaaagggccccaccgccggaagccgcccgcgctcccacaccttgtgcaggtctcccctgaaatgaattttaatttccgctgagggcaggcggcgtcgtgagtcctgagcccgtggcggcggcggcggcgcgggtgtggggccgcgcggccgggagcgggcggaagagagcgcgaatttgaatttcaaaggcatctggaacccaagtgcttctgcgttgcccgattgtgtgtgtggcgcttttgtgtgtccgcgaatgcgcgcgtgcgtgtgtggcgtgtgtctgggtgttttatgactgtcctccgtgaggccgtgtgtgagcccttgcgtgggccgtgagtgcggcagggagcgcggtgtccgggggccgcctgtcggtgtgtctgtgcgtgcttgtgcgctagcctttgcctctgcgagtgcgtatttttaggaccgagtctgtctatatgagcctgtgtctgtgtgtgtgcgctcccggccctgcgtgtgtctgtgagcgtctgccggggcgcgtgtgtgctcggaaccccgcggtggtgtgcgggtgtgtccgtgtgtctgtgcacgtgcaggcgagcgttcccatctgtgtgtgtgcatctgagtctgggctatgtgtgactcagggaccagtctatgagcctgcctgtgcctttgagccgatacctgtgtgtgactcagggacgagtctatga

SEQ ID NO: 240 - DNA, 181 bp, Homo sapiens
gcctgtcacctgcaccaggagctgctggatgaggccgagctggagctggagctggagcccggggccggcctagccctggccccgctgctgcggcacctgggcctcacgcgcatgaacatcagcgcccggcgcttcaccctctgctgaggaacacctgtgccccccgactccccgccccctc

SEQ ID NO: 241 - DNA, 241 bp, Homo sapiens
ctcccggcgctcctccagcgctggctgttcgcgggcagggtgggctggggctcctgaatatgcggggggcggggcgggggccggcgtgagctgtcacctgagaggaccggcggggttgccgggagggaggccggcgccaggcatccagctccgccccgctcggtccagcctcctgcgcccaccctctgtcctcgaggggcgaccggggtgcgggtcggagatgatggtccagtttctttgt

SEQ ID NO: 242 - DNA, 364 bp, Homo sapiens
aggaagggcagtgggccccgccgccgcctcccaatggcgaggctgcgggattgcctgccccgcctgatgctcacgctccggtccctgctcttctggtccctggtctactgctactgcgggctctgcgcctccatccacctgctcaaacttttgtggagcctcggcaaggggccggcgcagaccttccggcggcccgcccgggagcaccctcccgcgtgcctgagcgacccctccttgggcacccactgctacgtgcggatcaaggtgaagggccgcgcgggcctggcgggagcgggagggagcgtgaccgccgcgagggtggggggctccgggcttctccttccgagacgctggctcagcgtcc

SEQ ID NO: 243 - DNA, 481 bp, Homo sapiens
cctcgccccccgccccctgcgcgaacccattttccagtcctggtcaccagaggcgcagcgcacagcctttccggtggaaccagtgcgaaaacacccgaggaaatgaaaagaacaagaaagtgctaccttggcaaccacgggcgtttagtggccagctggtgggctggggagggcggccgctgcccccctgccgctggtactctcctcgactacgcgtattcttaagcaataacaacgtaatccgtattatccacccaagaatacccgtcaccgaagagagtcagaggaccaagctgccgctgccgctgctaccgctgccgctgctaccgctgccgctgctactgccgccgccgccgccaccagaactcttgctgctcgctgagcccgcccctgcctggggatgggctgagcttgaccgggaccataaatccataactcgatttccctaaagaaggatccaaagctgtgctcggctgcttcc

SEQ ID NO: 244 - DNA, 901 bp, Homo sapiens
ttcttccgaacccctcttgggaatactgaatggaaaagggggagcgtgagcaagtgcttggtagagtgtagacattgtgggatttgactgtggtaccatcgctttgacgtcctagtgctgatttttacacctgcattctgcttagggcaccggcaacagttttccgtttgtgcctactccacctgctgtctttgttgggtcagcgaacatcgcctccctctaccgctcaatcagcaaaagggaccgcccttgaggacctcacccgccgctcactcccctcccaaattcgcgggcatcgcctccggtcgcctcttccgaaggcctaacgagcatgttagctgcgaacggaggtgaggaggctccgctgactgaccggtgcccatgtccagggcacgcacaaacgccatgacttggcttggcctctctcttagttattcacagctcagcccgataggcacctccggggcggcgacggcaaagagggtgagcttattaagtgcagctccacggggactggcctctctgcacggctgtgtacacctgagcgagacgctcagtcgctctctaaagccgcttctgcggatgacagacacggagataaacgtgagaggtggcccaccacgacttgccctcctttgcccgggtttgcccctcgctgaggaggctgttctacatctgacccttggagcaggccggctgacagcgtagtaaaggaagatttctgcgggagggcggccagtgcaaaacaattccctgaccgggaatcgaacccgggccgtgacgctttcagcaccgaatcctagccactagacaaccatgcagatgcggaaagctgctttctctcccttcttcgacctgaagcgacactttcctgtgctctaggaggacttgggtcttgtga

SEQ ID NO: 245 - DNA, 361 bp, Homo sapiens
ccttggattcctcgccaagttagtaaggtgtgaggtctcttttccttcccctgacgcgcctggttgcgggagcaaaagggaagagctgacagcctagactaacgacattgccgtgactcggattcgaaccgaggttgctgcggccacaacgcagagtactaaccactatacgatcacggcgagccacaggctaagccgcgatggcggagcttgctctagcccttttgacgtcaatggatttcgattattaggcggattcgttcccagacagccacaggggactcgcgcttttctttcatgcccgctctgcttttccctcccttcctcccaatcttcatacgtgatgagaacaattctcatc

SEQ ID NO: 246 - DNA, 301 bp, Homo sapiens
aaacacattttctctgctgtatcctcagcctacctggggagcaggaccatttgggtttggtaagagaaaaaaggagggcgaaaaccccggacactcctcctgtctcccgacgctcgttctggccgtctggccctcagtactaagcaggccctgacctacttgtcttactcttgctgcttcttcccgccgggcctcttgccccttctccgaccatgctgcaggtcctgccccaactttaggacttcagaactcctccaccgtgccgtggaggaacagcccttcttccacctcacgcacaccc

SEQ ID NO: 247 - DNA, 721 bp, Homo sapiens; identical to SEQ ID NO: 12

SEQ ID NO: 248 - DNA, 181 bp, Homo sapiens; identical to SEQ ID NO: 13

SEQ ID NO: 249 - DNA, 661 bp, Homo sapiens
cctcccgcctcgccacctccccggcccccagacagcgacactgctcgccctgcctggaggctcccgctcagtcccctcggaggaggggaggcagacgcagtctcacggttttcttggcgggctcctttttcctcttcttctccgagttgctgtggtagggcaggtcgcggccgcggtaggacgggccgcgggtcagctccagctcgctgtagggcggcagcgcgtcgtcggacgcgtcctcctggtcgtcctgcgacgagccggccttgtaggtgccgggcggcgaccaagcgtagtaggaggcgctgcgcgggccgagctgcgcgctccgcttggatggcgtctccaggctgccaccgcggctggcgccctcgggccgcgcctggcgctcccgcgcgctgcccaggtacgagtggtcgtatttgggtgcggtgcctggcgtgcggctcaccagccgcggcaggtgcgcgtcctcggcgggtctgcggcgcgcggggctgaaggcccagccgcggtcagcatcggtcaggggctcgcggctgcggctgcgctgaccgtagtactcctccaaggagtcgtcctggtagaagccgctgtgcgcccgcgactccgagcgctcgaagcggctcccgccccgcgcctcgtgactgttgccgtctgc

SEQ ID NO: 250 - DNA, 781 bp, Homo sapiens
tggcctaagaaggggggaagctcgaggggttgtggggcacacccttgggccttccgggacagtaggctcttaaaccctagaggaggggagacaaaagaaacgctctcccacaggggtccctccagtcgccaactagaagggtttccctctcaacacagacatgtttgcctcttcatcacatggagtcaccacgaatggagcacttggggacgcaggtctaggtgtccccaagctcggtgcctctagtgccctcccctctaggggcattttagaagaagtgatttaaatccagcttatttcggcggcagctggactattcctttgcttatttggggatgggtgaggggcataccctttaggaaaacgtttccaaatgatgtaataatttctctctcatctctggtcttgctccagacttggcctcttcctcgccactctgtcccggcctcccgcccccgcaggctcccgtgcggacttagcagttcgcgccgtagccctcctggttttttaccgcgccttggtcgcgcggcccccggtgcgggcctcgtcgctccgacagccctacagctgtccctacggcccgcaccgacagctcgtccccgccacctccctccgggctgtagggacgtcgagatccgaatcctcacagcgcctgacccggggccgtgttgggtacgggtacggcgagagccttccgagccgcctccaaaactctccccgcggacctcagcagtccctccacgcgtcggggccctgctggccggccatgccctctgaggag

SEQ ID NO: 251 - DNA, 241 bp, Homo sapiens; identical to SEQ ID NO: 14

SEQ ID NO: 252 - DNA, 181 bp, Homo sapiens
cctttatttctgcagagctgagggcaggcggcgcaacaaatctcaggtaaaagagcatcagatttcagaagagctgtattctagacttggcgcaggcccctttggggagaagagcccaggggctatagagaacagaggtttgaaggaagcaaaagctggcgagaggttttttttttgtcgc

SEQ ID NO: 253 - DNA, 301 bp, Homo sapiens
attgggtgatcacggggagctcacctgagcgctcccgaggcttgggctctggtccctgctaatccccagagccgataaaaactggtcataggataaagaagcagctaagtttgcagcgggcagaggggaggcaggaactggagaggacgcgagtggcgggtggcgggggcggtgtgtaggggtgacgtccacccggcagagagggttccttgtcccctggagccgaacacaggaaaatcagctggtgagtcaatgggactttgttaggatagtcacagggcgcagctggcgccggcttaag

SEQ ID NO: 254 - DNA, 181 bp, Homo sapiens
ccgctttcgccgcggcctcccatcgtggaggctcagagtgcagctattcctgcagccggccttcctattttcagtaatctgattaggggtcgatgttggtgggctcggggacggcttctccgtgaggtcgttatttagcgcgcaccgggtcgcctgagcccggggtcgcggccaaaggggt

SEQ ID NO: 255 - DNA, 301 bp, Homo sapiens
aaaccacgactgcagacccaggcctcctgctctgtgagcaggcaaaagccctgccctcctgagcagggctataactgcccaaactgcagctgtgcatcagagcctccctgtgctcttgcgggagggctgggagcgggcaggatctgccttcccgggtgcagctgccctcccaggtgcaggacccgggtgtctctgcagcctgaacccttgggtgccccaggaaggacccccacacttctcctgcagagcagagagaagccaagcagcaggagcagacaccctggagcctggtcacggtggg

SEQ ID NO: 256 - DNA, 661 bp, Homo sapiens
catcaattgtcttaatacaaggttggtggcaaaaaacggctcacaagtatgcatacaaaggggccaaacacattgagcagcaaaacccccaaagcagacaccgcccgagacccgctggagcgcttccgcaaatctcgcgagatagcaggcagcgatgccttttgctccggtttctcgtgagaccccggggcttcagcttctcgtttgcggagcccgcggcggcgtttcctggggcaacagcaatggcggcctcgctgtccgagcggctcttctcgctggagctgctggtggactgggtgcgtttggaagcccggctgctgccgtcccccgctgccgcagtggagcaggaggaggaagaggaggaaaaggagcagggggaggcctcgtcgccgcgcggtctgtgccccgccgtggccttccgcctgctggacttccccacgctgttggtttaccctcctgacggccccggcgctcccgccgccgaaccgtggcccggtgtcatccgcttcggtcgcggcaagtcctgcctcttccgcctgcagcctgctaccctgcactgccggctcctgcggaccccgcttgccaccttgctgctgcagctgccccctgggcgcccgacgcccaccccacagctcctgggggcctgcgacatttcgctggc

SEQ ID NO: 257 - DNA, 301 bp, Homo sapiens
cttatttgtttggtctgtaacgtcagtctttgagtttcttgttttcagatactgaaattcttcacatccttcaaaaaaccatgcagacaaaggacacgatgaccacaggacatggagaaatggatttcagcaggacgttcatcacgggctgagtctgtggtttccagcttctgattaggaaaccaaacaagccctctgcacggacgtgcacaaaggaggaagtggcaagtgattctttattagcccctgagttttcagaggggccttggaactaaacctaaagttgtgcccccaccctgga

SEQ ID NO: 258 - DNA, 554 bp, Homo sapiens
ctccccatctctagacttccctgtctgctcatcccctctcttccgtgcccccctgaacaacacctttgcctgtaaggttaagaggctcccgtttggagccctagggatccgcagtggtaataccactgcgatggacacttcggtttccttttttgtctttaaccctgaacagtgactggtttatgtatatgtgtgtctgtgtatctttgtgtgcacccaccgggccccagacaagtggatgaggggcgaaatagttgcgaaaaagaaaataactataatagagcatactactacccagaattggacctagatcaaggattctttgtcacttaattttagatttgctgactgtttttttttttttttgagggggtaaggggagagtgggggacccattctgcctttgaaatggtcactgggcacggttgtgctgcaaataacacatcgcgcttttgccattcaccacagactactttgcggacttgccttatttcctagtggactggagtatttcattgcaaaatttgggtttagtggagatctccagtcagttt

SEQ ID NO: 259 - DNA, 781 bp, Homo sapiens
cccaagcagagaattgtgtctgagggaccctaagggagggagtgatgttggtttggggttccggggaggcagcggtcattgtgtatttgcacccgagtgttgagacccggggaacgggaaatattacagctctgaggctctgtgagggcgggtccttcccaccccaaagccagaggccaggagggaggccttcggttagggtggggaaagacattctcttctcttcttgcaccctaagcgatctcagcacccagagacgctgtctcagcacccagagactctgggatttctcacgggcggttttctgccttcaggcttaggttcttcgtaaactcacagcactttagcggtgaggagtgggaaggctgagaccctatccctgaggcggaggagaaaagtaggaaaatcaatacatggtggggcggaggcagacctaaccgggagagaggacgttgctccacacatctcagccctgtcatcctaataagacggggtggtaggagggggacacgctggcgtccagcagagaaacctggtcctctcaaagagaggacccaaccggtttcctgcgtttaggagggaaattacccatcctgcaatgcctgtaaaataaccgtttatttaatagttaaaaaaaaaaaaaactccagtgataaatgtccgttaccgatggtcagcataaagtgccaatcgcaatataacgcccggctcttggctggctgctccctcgcagtgtcgcggcagcggaggccgggccccctgcagaccccaggcccgaggt

SEQ ID NO: 260 - DNA, 481 bp, Homo sapiens
cccgcgacgggctggaagcggccgccgtgctgcgagcggcgggggctgggccggtccggagcccagggggcggcggcggcggcggcggcggcgggcggactcttgcccaggctgcgggcgccgcggctgtcccggccgccgcggttccccgggcccgcgccgcgcgccgcgccgcgggctccggcttcaggaacggctcggtggtgccgcaccacttcatgatgtcgctttaccggagcctggccgggagggctccggccggggcagccgctgtctccgcctcgggccatggtcgcgcggacacgatcaccggcttcacagaccaggcgacccaaggtacttacgcctcttctgtgcccgcccatcccgtcaggtcctgggctgagaccagccccggagccgtgccgcagctccgttacatttggagccgcggccccatgcggcccaccctcaggtgatagaaagaaacttcgccgaggcc

SEQ ID NO: 261 - DNA, 781 bp, Homo sapiens
tcagggtaggctgggccgctgctagctcttgatttagtctcatgtccgcctttgtgccggcctctccgatttgtgggtccttccaagaaagagtcctctagggcagctagggtcgtctcttgggtctggcgaggcggcaggccttcttcggacctatccccagaggtgtaacggagactttctccactgcagggcggcctggggcgggcatctgccaggcgagggagctgccctgccgccgagattgtggggaaacggcgtggaagacaccccatcggagggcacccaatctgcctctgcactcgattccatcctgcaacccaggagaaaccatttccgagttccagccgcagaggcacccgcggagttgccaaaagagactcccgcgaggtcgctcggaaccttgaccctgacacctggacgcgaggtctttcaggaccagtctcggctcggtagcctggtccccgaccaccgcgaccaggagttccttcttcccttcctgctcaccagccggccgccggcagcggctccaggaaggagcaccaacccgcgctgggggcggaggttcaggcggcaggaatggagaggctgatcctcctctagccccggcgcattcacttaggtgcgggagccctgaggttcagcctgactttcccgactccgccgggcgcttggtgggctcctgggcttctgggctcacccttacacctgtgtactaaagggctgctaccctcccgaggtgtacgtccgccgcctcggcgctcatcggggtgttttttca

SEQ ID NO: 262 - DNA, 661 bp, Homo sapiens; identical to SEQ ID NO: 20

SEQ ID NO: 263 - DNA, 361 bp, Homo sapiens
ccgcagagggatggcctcccggcagggactcctcggctcccctctgttctgagactgctgctgggaccggggtccgactctaaagagaaaactcaaacagcaaaaaaaggaatatcgactcagttccgagggcgggggccggggctcgttctcacccgcgcgcggcccctcgacctctcggacccgggccaccagctctgcgcccctcacgcctccctcggggtctctgtgtctctctcccgctcccggactccctcctccttctgactgctgttatttgggctgttgtccctccccgctccctggtacctcagctcggaccttagcctgtgcctgcagcccggagtcccctcctgccctg

SEQ ID NO: 264 - DNA, 541 bp, Homo sapiens; identical to SEQ ID NO: 25

SEQ ID NO: 265 - DNA, 601 bp, Homo sapiens
ctggtaacgtcccttcctgtcgcatggattcaaggccgacctgccccagcaccaccaccagcagccttctgctggggccggcacagctgggagcaacctcctactctcaggcagacgcgcagcaccaagcagagaggcccggtgcaggatcccagcgccgaaccagcgccggctcagtggacgcggaaggggccggcggccgcggccggtcccatcccccactgcagacccccagcctgtggcggtggtccagttccgccaggaaaccgccgcctggagctgtgggtcgcgcacattaacgcatccagcggaaaaatgaaggagacccaaattcaaagttaaagtaatggtgacccgagaggtgccttgatgagaaggtttggggtcccggttactgatggttatcattcttacgagatgctggtcacctacgaagggagaaaggcacgaggagcgcctgaccaaagtggttttgccctgcttcccgcaagaggtggcacccacggctggaacgcaggagtcagacccacagtccccagctctggacgcccgcagcggggcctcgaagaggttcagggcggtgcccgcggcgctcgggccg

SEQ ID NO: 266 - DNA, 421 bp, Homo sapiens; identical to SEQ ID NO: 27

SEQ ID NO: 267 - DNA, 181 bp, Homo sapiens; identical to SEQ ID NO: 31

SEQ ID NO: 268 - DNA, 421 bp, Homo sapiens
ccgctcggctccgcggccggtggcggaggctggggccgcgttgttgccgccgcgctccgcccctgggggcaggtgcgggcggcagggacccgccccaaggcccgggcgcgggagccggcgcaccgaggcggacgagagggaggaaccagcgtgaggacccacaggcggccctggcagagcttggctagggcgtagcggggacccgccccacctgcgccgcgggatggtgcccagaggggacccctcccactggattcctctggggtccgcgaagcccgcggccgcgcgtgggtagcagacagcgcccctaatttggcatctttctcttctggagctgcacaggcttcagaggctgtacagggtcttcgcctgggcctccattctcactgctcatccagggaaaaagggttcatctgtcccc

SEQ ID NO: 269 - DNA, 181 bp, Homo sapiens; identical to SEQ ID NO: 36

SEQ ID NO: 270 - DNA, 481 bp, Homo sapiens
gggaggagagagcgagcggtcaggcaaagctccatgcacgccttcccctctcctccacttgagaagagtcggcctctgggactggtgggtttcgagaggttgaggtgaccttaaggctttactgaggtagaagaagccggttgacgggcgacttccgaagactggtgtaaagcgaagaaggttctagagtcaaactctgactctcggggcctgactcgcaaaactcgggggctcccgagaagccgcggacgccgctctgcacctgttgccgccgtcactcatcccgccaggcgggcggggccgcgcgggtggcttggtcaggacctgccattcagcccagtcgggctccggtgctcgccccggacggcgccccaagcgggtcccggccccgctgagcacctccagcagtggcacagcctctggaggggtccgggacgaagccacccgcgcggtagggggcgacttagcggtttcagcctcc

SEQ ID NO: 271 - DNA, 481 bp, Homo sapiens
tctctgaaggacggtggcagcaggggtcagggcactaccaggagctacagaggatttgggtggggggtcttctggagggagaaaccaggactgcgagaatcttctgcttcgggcaggaaaaggtgaggccgggtttgcttcgcaggcacggagcgcgcaggcgcagagaggtgtttcactccttcccgtcgcgacccagagactcgcgaacctcacttcggccactcaggtgggcgcgacgcggccctagcaacggaaacgccgcgcctgcgcattgccttccgcctgccccctccccccccccgccccccgcattccgcgcctgcgccaccgcgggaggcctgggtgggcgcagctgtgggagccggtcggagtccgagcgctccgtcgcggggcccggccgcttggcgagcctgctccgggccccagcacttagcctgtggtcctccaggccgtcttcccgctttcctgctggccccat

SEQ ID NO: 272 - DNA, 301 bp, Homo sapiens; identical to SEQ ID NO: 40

SEQ ID NO: 273 - DNA, 301 bp, Homo sapiens
aaaggaacccttaaaggaactatatggttctaaaaaaaccctaaatgtatattgcaacaggatgcctcctaccacacacagcaatggccgggagagaaagacgcagaaaaccctaccgttaatatctgcattaccttttgcctagtgaaccaagagagatctggggaaatgaccgccatactaacgctctctttgtttcaaaatagcccacacagctgcattttgcaggtggtgaacagcttttactacttttagttgagacagctctaagctgaggaaacgggcatgaactgcagttccc

SEQ ID NO: 274 - DNA, 550 bp, Homo sapiens; identical to SEQ ID NO: 41

SEQ ID NO: 275 - DNA, 312 bp, Homo sapiens
tctcgcggaggaacccgccatctgccagaagccccaaagacgccccgccccacttcccacagcttcctggcccgccccgccgctgcctcccgccccaccgcggctcccaggccgctggccctaccggcaccccccctttggcgagtcggcagccacgtccttgtcctcacccgcagcgcagtgacgccgacccatccaacggtcatcgcatgcgcgtgccccgcgcaggccccaaacccccacggattaggttgaaggtcagacaaaaaatcccggacccatacgtccggttccttaaggccttgcccacac

SEQ ID NO: 276 - DNA, 241 bp, Homo sapiens
gcccactcgcccagccacgggccaagagcgcacggacccaggcgggcggcagcccacccgccaccacgcagctccacttcgctgttccacagccaccaaccgcacagccggcacagtcccgcccgcgcagctggcccaatcgggcctgggctgcaaaagcccagggaatatgagggctccctacttccaagtttctttaataaaaatattacatttaatgatgcttgtcaatatcctcacc

SEQ ID NO: 277 - DNA, 421 bp, Homo sapiens
cgcaagcgaggggaggagacgcaaagccggggagtgagtgattaaagaaaagaaagaagggcttcttgcagctccgggctgtgttttttcctgcgcgccctggcgcagtccccggctcggaaaggcaggagcacgtgagcggtttgcagagcagcccggcccagccgcgcgcccgtggccggaggctccatttaccctccgcggagggcgctgtgcggcggcacttaagcggcagcttcctctctcccaggcggcctttgtggctgtggccgggacagggaaaagctgcccaggccaagagggcgggggcgtcaggggcagccagcgccgcctttgcgcaactgaagcggatgaagccgcctgctctcaggtcttctaaggagaaggtctttttatcactcccattttacagatgaggaaa

SEQ ID NO: 278 - DNA, 1201 bp, Homo sapiens; identical to SEQ ID NO: 49

SEQ ID NO: 279 - DNA, 661 bp, Homo sapiens
tggggcaatcacggggctgcgcgttgccacgggactgcgcgttgccacgggacgccggtgccactgcggggaagcgacggcagccatgggggagagggtcgggttcgctgacctcgttcgggggagcaatgggcgccccccggcgggcaggcccttgtggcaaggaggccaaggtgccgggggacccggggacccgggtcgggcgcgcgttacctcctccgcgctgcagcagcgagctcgggttcgcctgctggtctgagagcgtaccctgtgcggcgcgccgcttctccgagtgcacgatcagcagcatgtcgatagatacagcgttgatgtccttcttcagctccatgatgccgcctcctttccgacctgggcgccgcggccgcacgctaggctgcttgcgctgcaaatggccccgtgcgcgcagctgccccacacgggagagggcgagggcgcggaagagggcgctcccccgccgctggagccgcagggcgctgcttttcgctgactctgccaaacacgccattagggcccgcctgggagggcgctaccctaatgaagcggctctaagtcacctttgaaaggaaatccccgggcccaagccttgacctgcaccggggccatagtcagcaggggcggccggtccagagcctccctccct

SEQ ID NO: 280 - DNA, 361 bp, Homo sapiens
cattttaatatatagtcaatggctctttgtggaagggacaaaaagaaactacgcgcagttgttgaatagactttgcgctaggcaaagacaggttaatcgagggccgcatcgcgaaaacaagcgagtgttgtatgtttgcactgaatccaaatgtctgcattttcctaactaaatcaaagggagtgttatttctttttctgctcactcatctgaaggtaagtaaattttctctggcgatcaaaagcctggtcggcaacaaagaccgcgcccgctttttccaccgtcctggtgtggcgagttgcggaatttcaataactgtgacaagggtgactgatttgtgaactagaaaaggtttgaatgt

SEQ ID NO: 281 - DNA, 301 bp, Homo sapiens
catgttaactgggagcgcagaattcctttaaagtcaaactttgcgaacaagaataatcttgaaaaagaccctttaggcgcaaatcaacgctcaagaacgttgccaatcacttgtaacctccttaggcatttcacggatgtgttatttatgctcaaggaggggtctcctttcagcccggcaacccaaatctttgctctgtgcttcggactcagtgggggcttgtcggatgagccactgggaaaatatgcgtcccctcacttctccttaatcaactaaggtcaccttgacggagcgcttccct

SEQ ID NO: 282 - DNA, 181 bp, Homo sapiens
ccagggccgcggccggaagcccctggctgcacgcgcgggcccaggcggcccccagccctgtgagctcgcatggcgcgccctctgggtcctcgcggtcaccttgcattccgagcacggccgtgttatgtatgcctttagttgatgctggccaaaattagacaacttagtggcagacgtcgag

SEQ ID NO: 283 - DNA, 421 bp, Homo sapiens
ctctcctcgccgctcctccccgcctccccgcggagggttgacccttcaattcggagtcccggcctgtgggcgggcgggggagcgccgcggctgtaagccgaggatcaggcggcggcgcggagagcgcgcccgggcggccagcgccgagcgcgcggagctggcgtggggagacacggcaggaaaggcgagtcggagtgggtgatgagaggccgggagagcccgtccgagccggagagaccggagagaagggagcgagcgactgtgcggcgctcacgctgccagagcccgggcggagtgcagtcgcctccaaagccttagagcggcgccccagtcactgcagctcttcaccctagagctgtgccctgggaccacagagaccaagagcatggaaatcggctgagaggtacaaaagaaataagga

SEQ ID NO: 284 - DNA, 481 bp, Homo sapiens
atcgatccgcagggctgatacacacttaattaaactcattttgtgtagtgtacaaactagttaaggccatttaatttatttcggcgtatattaccccccaattaccgccggcgcagggccagccaattgccgggcatttaataacaggcccggcggtggggccggagccggccgagagaatggggcttgggggacccaaatcctatgccctggccccgaccctacctcaagcctccaggccctgagcttcggtcgcgagggtcagccccggctcccctgcccgcgcctcggcccctgcgcagagttgccgcgggtagggccctgctcggcctcaccaggagggctgggcgggcgtgcaggtcggagtggctccccgcggcctaaaggcccggtcggccgagtctgaacagcagctccgcatcctccaagcagaggccctgaagtgactgcattttgagtctctgaaatttggaagaaagca

SEQ ID NO: 285 - DNA, 181 bp, Homo sapiens
ctgcgctcagattaacggaaaaagacacccctctagagtccggcagcagcgggcgggcaccggcgccttctccacacaggagaatctcggcgatttacacccccaggctacgcagaaaaagcggcttcggaatccgccgcaagtcccctcctcgggtcgccggggaagtctggcctcccgc

SEQ ID NO: 286 - DNA, 181 bp, Homo sapiens
aagaaatcaagaagctccgggcagtagggccctgctccctccaatcagagcccagcccggggccagagcaggaagcgcggcggtgggacgcgcggtgacagccccgcgccccccggggcccgccggccaggggagaggacggtgcggccgctgcgcgacagctccgggcccgcgcctctcg

SEQ ID NO: 287 - DNA, 181 bp, Homo sapiens
gggcttgcggggtcccgcgggaggacccgcctcaaagagccggcccgatcatcgcctcctagaatacccagctcaacgtctacctggagtcggctctacaggacgcgctcatctcaaacccagagctcaggcttttagggcagagagcgagagaaaggcttgctttacagaaagggaaact

SEQ ID NO: 288 - DNA, 901 bp, Homo sapiens
gaaagggagggagggaggggagggatcgagagagagcggggagagagaggctgcaatctcctccctgaatcgcgcacagcgctgcagatcccactgctccgacatgcgggccgaatgcaggtgagaaaaggcacggactctgcggctgcgaacccaaacttgggcaccgcacggtgcgcactgctcagccttcgcccccgtgggcgaaaggctgctgcggtttcaggcggctgcttcgtgactaatgaccttgcgcagagttgttaagaaaaaagagaaacccgcgctctccggggtgagaagggactgactctgggcgtctctgaagatggctcgggcttctctttggcgcgccggggggaccctgacactgaccgctctgtgacgcgagtagtctcccctgcaccgtgcccgaagcgacgtgccgggggatttttcattctcgatctgttgactggctcccccgctgcatgagcagagtcggagttgagactggcttgttgctggccccagcgcctggtgcaggaagcgactcacgtttgtctgggtggccggagccggagcagagcctgggtttggagtgagtgcctggaacgtgaattggactcaactcgagtagcagcaaagaccagcgggctggcaggcgggggaggctgcaggctcattccccacctcttcccagccccactgcccgtctgccggagcggttctggccccttccgacagagcggggactagagccggggattctccgcccgctgaggggatgactctgggttgggggagcgccgaacccgcggcgcgcagtgtcccgtgaactgtgagtactgcgactgaacggcggcaggcgagcgggcgattagcacccattgcatgaattatgaaacaataactttcggaa

SEQ ID NO: 289 - DNA, 421 bp, Homo sapiens
ccagcgtgcgaattccgccccgggatgcgaaggagttcgaacgcatggagtggaaaacaggcaggcgtgatgtggccatagtgggagtcaagactgcggaaatggagcgacctgcaggctagaggagagatccacgtgcgggatccactttgacctcggcttcatctctgatgctcttactgtgttcgcttcggctttggagtccaagatatgtgcggtccccactacgaaaccagctgcctgcacccggattccagagcctaggcccttacctatgggaaatcctatagctccagatgctggaatccgagctctgataggaaaacgccctaatgctggcatctctcgcttagcacataggcaagaaaatggggcacgacccccaaatccactcccttccagcctccgaaaaatgcaccca

SEQ ID NO: 290 - DNA, 301 bp, Homo sapiens
aggcgagagagagaatcgcccaggcggcttaggcagccagtgggccagtgggcctgcgcgccggggtcaggatggcagggcagtgtgtccatcctggcgggacagtaattgccccgggtctgacacgacgccgggggctcagggcgcctccatccatctccatccagttagcgacgcgccccccgaccgggcgggtggccgggcttgggcctcagctccgaataatgagaacaattgtctccccgcctggcatagccctccgccgctcctccgggttcgctgcccctctcatttctctagc

SEQ ID NO: 291 - DNA, 721 bp, Homo sapiens
aagaatgaacccgtcgttagcccccggtgccctggctcttgtttaaatccttagatcgagaaggacttgaaggagatcccaggctcccagctctgcgcccctgggccagtttcctctcgggacgcggactgaggagggatgcagggggaggggcattgggccgggctttccagctgcaaacacgtctggcgccgaggcgggcccattttgtgcctcctggggacggaccgtgggcggcgcgcagcggcgggacgcgttttggggacgtggtggccagcgccttcctgcagaccccacagggaagtactccctttgacctccggggagctgcgaccaggttatacgttgctggtggaaaagtgacaattctaggaaaagagctaaaagccggatcggtgaccgaaaggtgtgggtctcagggttccccgggtctaactcgccgggtccaaccgcagcatcagccttggggcggcagataatctttcggtctcgcctggggcgcaagatgcaggatcgggggcaaatggcttctcccaacttccccctaattcgggttctgccagatggttgtcgtttgctgaagtggctcggcggcatttccttttgttttaaactgatcaatgagcgaacctgggatgggctgaaaaagtagattgtaggagggaataatgggaaacccgacttggggcgcctccttccctgcctcctactgcagtttctc

SEQ ID NO: 292 - DNA, 181 bp, Homo sapiens
ttagaaactgacatgttctaccccagggcctccgcgaacgacagcaggcgagaatccttgctctggacacggggaacagggtcagcatctcgtctcctatctccaccgacctgtctctggcttttcttagtccccagatgcgcccagaaggtcctggagagtggtgcgtccccttggcaac

SEQ ID NO: 293 - DNA, 541 bp, Homo sapiens
tccttacctgccctccgcccacccgtgggcccctagccaacttctccctgcgactgggggtaacaggcagtgcttgccctctctactgtcccggcggcatccacatgtttccggacacctgagcaccccggtcccgccgaggagcctccgggtggggagaagagcaccggtgcccctagccccgcacatcagcgcggaccgcggctgcctaacctctgggtcccgtcccctccttttcctccgggggaggaggatggggttgggaacgctttccccgaggatgctcgtgtggctggtggcctcggggattgttttctacggggagctatgggtctgcgctggcctcgattatgattacacttttgatgggaacgaagaggataaaacagagactatagattacaaggacccgtgtaaagccggtaagtggctctccaggttgggacggtggcgcgccgggggccgctgcgctgggtttcccatgggtggcggtgggagctcacctgtttccttccctcccgcgtcagcccctccgccgccc

SEQ ID NO: 294 - DNA, 241 bp, Homo sapiens
ggtgcgggagcccggcgaggtcgagctgggcggcggcgggggccgcgccgagggaggaggggaaggcggaggcgcggggagcgtgtttggggcgccgcggcggggagggtggcggccgctggtgcgcgcggggcgctgtgtatgcgcgctcccccgctcggggaggaagatggcccaaaagggaaagttggggtgacgcgcgcggtccccggaggctcggcggggggcaccgcggccagcc

SEQ ID NO: 295 - DNA, 361 bp, Homo sapiens
ctggaggcagggctatgagcacaagtggggcgccctgtgggtgtgcaaccgcggtcggggagcacaggcttccgaagagaaactgagctctaagtgccactcaggccggacgagttccagagggggacagcgccctcctcgaaaagccttggtttctccccgccccctcttgtgacagaaagttggcaaggatgccccgtaggagtgcgagccgctcccctcctccgaaaagccgcgggcttccgctgctccgggcatcaccaccaacagcttcccactcccacccctgggactaggacaggggacttcaccctcctccttccttccggaggagcccgcggcttcgcctgaggcctcgcgg

SEQ ID NO: 296 - DNA, 181 bp, Homo sapiens; identical to SEQ ID NO: 62

SEQ ID NO: 297 - DNA, 961 bp, Homo sapiens; identical to SEQ ID NO: 63

SEQ ID NO: 298 - DNA, 601 bp, Homo sapiens
gcactccaggcgcgtccagcacgttgcttttctcatttgctgctgctccgggatctttggcagcagcaaaaccccattcttttaagggctgcgcagagttgtgccgcccatgcccggctggtttgaaggtgccccatgggcgggcgcggacgtgtggttgctccagtgtttcctagagcactctcagccacgcccccgccaccccagcggcgctgcaggaaccagcccgccgccagcgcgaaggtgagaccgggcgccacgtgcttacccggcggcctccggaaccagccctgcccgccggctgtgcgcggatgcctgcagacgccgagctgctgcccccgtgtggcctggtgcgggggctcctcctgctcactgggggcgcgtcccggtaaaccagaacctcagcccatcaactcactcgtggggttactgaggaggagaatctttggttctcaccgtcatggctcacccagtggctgaatcccgctcgcacgtgccgcatccaggcagctgtggaaactggttgaaaccaggatggtcagctgctaccctgtgtttgggggactatgtgacagtgcctgctgtgtccctattctggtgc

SEQ ID NO: 299 - DNA, 181 bp, Homo sapiens; identical to SEQ ID NO: 64

SEQ ID NO: 300 - DNA, 181 bp, Homo sapiens
attcaaggtaataaacaaacaaacaaacaaacaaacaaacagacagaaagccttttgcctgggaggtctcgcgattcccacgcttgggggcgacaagagttggctggagcagggtcggtcgaggctagttaacaggtgggagcaactttattctgccggtgtttaactgctgtcttaaccg

SEQ ID NO: 301 - DNA, 541 bp, Homo sapiens
tctgatccagtgtaatcgcgaaggtaacaccatggtcccaacagagcggcctaaaacctgctcatggcaaaggaacaaaagggtcttgcagctatcctggaagttaagtccagacgtataaaaatgaaaaagaaaacttaacccccccctttttgttcttttcttaaaaaaaaaaaaaagagtatttgaggcttccgttgacttcttttatcttgtaacttgccttgcctttccttcccttaacttccgactggcccgaaggcagctgctgtgctgggctgccctagcctcctgtgccatgttttatgcatgaagatgatggggcggtaatttattcaagcagagacgatcaccgggctcctgtgtctgccctcgcgtcagaggagccgtgcaatggcagggggagggcaggtgtgtctgactgcacgcaggaatgggctgaaatgggaatccctctctgtaggcagaaatgaagagcagagctttgctgctagagctgaatcagagcaacaccccttaccttttagggcgtatgatttat

SEQ ID NO: 302 - DNA, 489 bp, Homo sapiens
ccaacgactgtttttacttagggaaactactgaactgccccccgattccttaccgcatctctgcattgtcccaagttggaagttgagactaaagcaccaagatacaagagacgcggcatcccaaaaggagatttttgtgtattctgcgaaatacacaaaagggctagccaaagaaagtcctcacacacgtgcatggtataaaagcaccagctttaaaaagagaagtgtttttgtttttttgtttgagaagcataattgaagtgagcagttttagaatcagtgcagcaaatttagagatttcaaaagagatcaatatagaagggatcaaatccacacaatcatgggaacgctatgaactcactggcaaaatgcagtcactgaaggaaaaacgtcagtgtcaaaatgctactatttcacctctttgtgtacgatttctgagagaactgccacgtttggagatgctaaatttacccaatgccttcgtagcct

SEQ ID NO: 303 - DNA, 181 bp, Homo sapiens
cgtttgccgtcatcctggcctcctacggtgccgtggcccgagctgtctgttgcatgcggttcagcggaggccggaggagggcggtgggcacgtgtgggtcccacctgacagccgtctgcctgttctacggctcggccatctacacctacctgcagcccgcgcagcgctacaaccaggcacg

SEQ ID NO: 304 - DNA, 601 bp, Homo sapiens; identical to SEQ ID NO: 70

SEQ ID NO: 305 - DNA, 421 bp, Homo sapiens; identical to SEQ ID NO: 72

SEQ ID NO: 306 - DNA, 241 bp, Homo sapiens; identical to SEQ ID NO: 74

SEQ ID NO: 307 - DNA, 391 bp, Homo sapiens
ctggtgatgctggaggaggtaccggggaggagcgtgtgtggccccggcctctcactagcagcggcggctcccgacgctagcctgctcgagcgcacccagcaccctccccaagaccatggcccgcacctggacccgcggttaacttagcccgccgcggagagagccaggcaatgcctgggtggtgtcgtgctcaccagctcctttccgcagacctgatgccgatcagatttactccctgctgaattcaccccccagtcaggccggttttccttgtttcaccgtgttctctgaatacactgaattactccgagcatctatagttggcaatgccctgcgcattttccgcactccgatacactttacactgaacaccaattcggaagttgtgtgg

SEQ ID NO: 308 - DNA, 181 bp, Homo sapiens
gctgcagtgtgcctttctgcggacggccacggccacctggccaggaagcggctgctgcagcagtcattctgcggcatcttgcggccttggcgggcggtgctgtgccgcgttctgctgcccccaaggcaatgctggctttccctgtgtggggctggattgtttgtttcatttactcgcataa

SEQ ID NO: 309 - DNA, 421 bp, Homo sapiens
gggtgctggactagccacaacgtgcgttggggttattccctgggcgccgcacccaccggtgcccatctcccacctcagcagactttcctcctagcagcccgcaggcttcggggaatgcatcggatacccaagccctggctgcctccctcctcctcctcgcgctgctgcagcaaagggctcgtcctccctcagtcgcgaaggagattatcctagcgttgcgccatgttatgccctcgcctccccttccttcctcgccgccggctccaaagcctcgccgaggcccatcgcccgggccccttccccccggttccaaatccctgccgcaggggccgcccgggagctctgcggaggcgccggagtcttggggcgcctcacccttcctggctttggagaggagccgggctgacagcgaagcccagtc

SEQ ID NO: 310 - DNA, 541 bp, Homo sapiens
gccaaagacatagactaaccccacccgctagcgcccaccgaagttactgattaggaaggttcccctggcatcagcccatttgcttcacacactcttcctccttcccaaggggctaacggaaaagttgcacctaccagcggtaggagcacggggaatcgcgcacgcaggccctccgcgcggcttcccggagcggcctttggcgactgcgccgcccctacaaggccgcacacccctcgccagcactccggcagcctcgcacaagacggagcccacgcaggcttctagttttctaaaccaaaaactgcacgcgccggcgtgtgaatctgacggagagacttttagagttttgtttggttttcagttcagaccgctacgctgtcagagcaagcaactccgagccttgatgggaatgacttacaagccgcggtgcgggctgagcctgcctctctcggggttctttccccaagggagtgggagacaattgggcctggaacctaaaaggaagagagcctgtgctagccgcggggtagaggggaaggag

SEQ ID NO: 311 - DNA, 181 bp, Homo sapiens
ctgccacacaccgcaggcagcgctgacagactcggccttccgggagcgcaggcgggtggggggcgccgcccttgtcgctgtccggagccccgcaggcccgtggccccctgcctggttctcccgcctctgcaagcctagccttcaggactccgcctcgcccccctcttttctgttcggagac

SEQ ID NO: 312 - DNA, 301 bp, Homo sapiens; identical to SEQ ID NO: 81

SEQ ID NO: 313 - DNA, 301 bp, Homo sapiens
acaactgcacacagtccaaaactcacgctcacacacatcaaaacacaacttcgcacgtccaaaactcacacacacacacgacacaacttcacacaacgtccaaaactcacgctcacacacatcaaaacacaacttcacacagcgtccaaaactcacgctcacacacatcaaaacacaatgtccaaagctcacgctcacacgcgcgttgaaagcagccggaacaacacaatttcctccaaggggaaatgccgattcgaatgacagcgaatttctcatcggaaaccatgcaggccagaaggaa

SEQ ID NO: 314 - DNA, 301 bp, Homo sapiens
ctttttgaaatgaattgaggtaaaataaccgtttcaggtccatcccttacatggcaaagtaaaaagctggagtcagtacacagtgttggggtgggggcagcgtttgggggcgacgagttttgtgcaccgcgctggagtaccctgcacataaggtccgctcatgggcttctcagtacggactcgccggcgggaacaattaattgagcaaagcgcccctttctgggctggagcaaggttcgcggctgcagatatctcaagctgaaggcaagagcccaggcgaggcgcaggcaggccacgtggc

SEQ ID NO: 315 - DNA, 181 bp, Homo sapiens
ggtccagccgtctgagctgccccagacggtggaagtcgaaggccgtgatgttggttatgaagttgccgccgaggctgtaggtgagcacgtcgtgggggctcggcagcgagctggtcttgggcactacgcggagccccctgttggtgcacaggagatgctggggatgctggcagtcgcagcg

SEQ ID NO: 316 - DNA, 481 bp, Homo sapiens
aagaaagtagggaagcgctcagtagaatccggcgcctctgagccggcgccaactggccaggtccatactcggggcagatcccagggctgggactctcattcgatggtcccaaatttgatctctttgacagtggggctgagcaaatgcagccctgaaaaagataagcttagcgagagctgcgggcatttggcaaaggatgctgctctcagaaccgtggcttctgctcctcaccagtgcgtctctagcctggggctcctattttccctagagggaccctggaaaatgggacggctgccgaagagaaggcgaaggtcagggcgcggagctctacggtaaccacgcgacgcgtagtgggagagtgcgaaccttatggtagcgcccggactaagcggacacagacccctctggttttacaaaggcggctgtgacgaggacttcccacggccttgttggagggcgtcctgttagccctgctcagcct

SEQ ID NO: 317 - DNA, 301 bp, Homo sapiens
acatacatacatatatatataattagaatgaataagacagaatttgatagctcaacagggtgactatagtcaataatactttaattgtacattaaaaattaacttaggtcagcgcgagggagcccgggtggccgccattactgagcctggcgctgcggctggcgctgggagagcggggagggacggggccgcagctggtggcagagagggagggagggtgggtgagcaggctgcgggggccgtggggctcagggtttccgggcgtgtgtgtcggggagggcggagggaggtgcctgaaggg

SEQ ID NO: 318 - DNA, 181 bp, Homo sapiens
tcccctggctgcatttcttaaaaatttgggagcctgggagtgagttttctccgaggcgtgtgtgagaggcggcgggggtgttttcctgcgcgaggggcgggtgaagttcattgcccccacttttcccgcgacctttttcggacccgattttggatcgagttgaggggggcgcgggcgtttt

SEQ ID NO: 319 - DNA, 301 bp, Homo sapiens
ccttcagcaatggtacggggactgctgtggggcctgggtgagggtgacggctgaggagagtggtgggccctaggagcccctcaccagcaagcgccttcaatgattgagcccctgtgggggcctttgggagagtaggtgtggatgaattgggctttatctaaaggggtaatatgtgtattgaaaaatacacacgtagtgaacaccaaatcccgggagtagtgctagtggtgggtttgtcagctgtcaagggctctgcaaccctttctctgaatccaagtagttcttcctttggacagggaac

SEQ ID NO: 320 - DNA, 181 bp, Homo sapiens
aacgatggaaggctggagttggtaacattctgagacgggtgtagcctagggaagagtaaggtgtccggccgggctgtatctcgtgggtggcgagggaacattgcctgtctcggaaacagttcccaagacaacgcgcatcccagacgcccggcgaggctgccttcctacaggtcttttactt

SEQ ID NO: 321 - DNA, 181 bp, Homo sapiens
ggccgacgacacgtggtggaaaagtagctattatttacatgcgtgttgcagtttttgataatgcgattgctgctgctaatgtgactaacgcgatgccgatgaacatctcggcgttttttggtgcaggataagcgggtgtagactctgtctgtttagtcccagattctcctcctttaatgaa

SEQ ID NO: 322 - DNA, 181 bp, Homo sapiens
aaattcatcagttggggtggttgagattgggtgagtggttttgggggttttgttttgtttttgcaaccgttctttccaaacactccccgccgccccccaccaccgcagaaaaaagagcttttagcataaggcggatgctatctatccgcggtagaaactgggtcttctggtcccaaggaat

SEQ ID NO: 323 - DNA, 361 bp, Homo sapiens; identical to SEQ ID NO: 96

SEQ ID NO: 324 - DNA, 423 bp, Homo sapiens
cgccgccttctccacggccccggccggacttgggctgctttcgggaccttcaggttgtcgcaccttcgcgggcacctgcggctgctccagcgtggggaccaggcttcccacgggctccattgggagctctgccccggcttggcctccgggcgcagcctcccaagactcctccatcccgcgcgccccgccacccggagacgctgaggagcgcacctgggcccagtgcagaggagcttcgctctcctccgtccggattggtccagccgcgtcgccgaagttgtcaggccacgcccctccccgaaggaccccgctgtgattggctgtggctgaggttctgctgccccgacccccttcgggacacagccccggcctccaccaggcactgggagggagctgagaacggcagcggggccaggcgagggt

SEQ ID NO: 325 - DNA, 344 bp, Homo sapiens; identical to SEQ ID NO: 100

SEQ ID NO: 326 - DNA, 481 bp, Homo sapiens
agtgaggaagtcgctgtagagcagccggccctggtcgtccgccgccagcacgcggtccccggggctcaggtccttcaccagcttggtgccgccctgctccaggtgcaccgtggccgagcccgggaagcagcctcccgatttggccgccaccgagttctctgcgggtgaggagaagggaaagaagagaggacagggcattgagttccgagagggaggcgcgtctcggggaggagggcgcacgcttggtgcccgcgctcctaggccaggggtgcgcaaggcgcggggcggggcgattgattccaggcgggtcccgcacacacctccctcccccaaccccactgccccagggacaggattccgacacattccttaacgactctctaagtctgggctggcggtcacagaggttggctggcgtttcctgcagaggccggtgacactctttccttccgccttcctccaaccccacccccagctccgc

SEQ ID NO: 327 - DNA, 421 bp, Homo sapiens; identical to SEQ ID NO: 101

SEQ ID NO: 328 - DNA, 481 bp, Homo sapiens
aaggacttctgccggcttccttcagaaaaatcaagaatttaagaaaatacttgttatgcaaacaaacatttagcccacttaacattgagctacggtcgtccaaagctgcttagtgtccgcgaggaggccgtccggatgcgcgatgattcaggccttctccgccagctccacccgggacgcgagcacccggcgtggacctctgcgtcccgggcccacgacgcccgcgccgcggggtgcgcgcactgcgtccccgctctcctgggactgcgccccgagtaacacgtgcagggggcactgggtcccctgcaagcggcgagaacgccggcagccctggccagttaagcggggagtgggtccacgcggaccacagcggcaactcagcccaggacgagcctcgggtcaagttctccgactccgcactcgggcacctagcgggccgcgccccggagctacgcggccccaacctcacctgcccgcccaa

SEQ ID NO: 329 - DNA, 721 bp, Homo sapiens
cgcgtcccggactgggctggaggagtctccggatttacctggctggccttgtcccttcaattggggtcatcccatccttgccccctggcctgccagcgccgcttccagccggtctccttagggcaaggggaggctgggctcagaaaagtcggcccttggaataccggcgctcctgggctgcaggagaccctggcgtccccatccctctagaggcccctctcccacggcgccgtttgtgcagtgagctctgtgctgggtcccgcgtccttgcctctcctttgcctctcctggaagtaactcgagctttggctgtttctccattgacttcgcgcaaagattgcgaagaaagaaacgcggctggggaagcggggttccctcaccgcagcccacccgggcctccttccgcgacttccctcttagtcagggcctcagtacgcctttgctttgctggcagcgagcgctgcagcgccgcagcccgaccccaagcctcctacaagggggtcgcaagtcccagcagccgcgcgagcattggcgacccctccccaccgcagagatttcctgcgccgaccacgtgctcgcagctccacgcacgccgtggatttgagggtcgggcccccgcggccgccgcttcctttcctgtcccaaatccagcctaagagccgcttccctttccctgtcctcctgaccccagtggcaaccgtttctccaccgccccttgccc

SEQ ID NO: 330 - DNA, 181 bp, Homo sapiens; identical to SEQ ID NO: 103

SEQ ID NO: 331 - DNA, 181 bp, Homo sapiens
gctcacgggcgttggccgcgttccgctgcgactgcttgcactctgcggctgagcccttggccgggaggggcttcttgccaccaccgcccgcgctaccacctgcgccgccgcccccagccacacggggccgcttcctcttgcagccttccgcgctgccggctgtgcccagagcgcagcgctc

SEQ ID NO: 332 - DNA, 301 bp, Homo sapiens; identical to SEQ ID NO: 111

SEQ ID NO: 333 - DNA, 301 bp, Homo sapiens
atccatccttaaatccttggatgtgtttagacgcacaagcattcatcaactatttgttgagctcctactgtgtgccaagcacgcctctaagcgctggggacggcgatggaacaaaacacacttccggttctctggagtttacatatcggcgtgtatgtaggggctggggcgttcattatgcattgctggggggcttctagtacggccagcgctgcttttcattctgttcccagttacctgtcctgtttgaggctcagcctgtcttgtttccctggaagcctttgctacaaagcggtgccat

SEQ ID NO: 334 - DNA, 181 bp, Homo sapiens
agctcacagccgggatggcaggagagtgcggaagcggcacatggcagacacaaccggggatgacccagctcctcaccagagggcaggtaccggaaaccagcaaacacgatttgacaggacgcagagcaaacaccgcattaaacagctcctgcgttccaaggccaggtgcttagttcatcta

SEQ ID NO: 335 - DNA, 181 bp, Homo sapiens
ttgcgtgtcatgtacacatgtgcttgtgcgcgcacgtgtgggagtgcgcgtgtacgcgcacctgtgagcgctcggcgcaggcccgcgacacgcccgagcccctcccgccgcgccccgctctcgcccacctcctggtgctccacctccccgccgcccgggtgcgtggcctctcgggaagacc

SEQ ID NO: 336 - DNA, 301 bp, Homo sapiens; identical to SEQ ID NO: 114

SEQ ID NO: 337 - DNA, 313 bp, Homo sapiens
tgccctcccgcccttggaaacttgtggaccccagaatctcagctttccgcctaccaaaggtgccccgatcccctcccactgccctagcagcggcccagccccaacgcctttggctagagattgaaatcctctggaaccaaccactggacgctctggattggggcggaacgcgcttccactgtctcgaaagcagcaccttctcggatttgagcctttgcggcgcgcctgggctgagatctgagaaatgcgccctgggccacaggcagcagcggaggcggggaaggaacaactttccctccgccctctaaccaca

SEQ ID NO: 338 - DNA, 601 bp, Homo sapiens
gggcacgcaggccgtcctgtcctcgagatcaccgcgtcacgacttttggggagactcacccccaccaacaccgtccagagaggcctgagggagggattccatgctgccttctccggactctgcgtcgggtttcctcaccctgttcggccctttgtgactcttggcatccggagactttcccctcgacccagtggagccgtcaggccggagcctcagagccttgacacccaagcactgccacggaagtctccccctttgccaagcctcggggactggtttctaagacaaccgtgggaaccactgtgacgggagaaaccgcttgtgcttcgcgcatgcgcattggctgggccgactcgttctcccctcctggcagtcaggctgcgtcccctttaaagaacgccaccgctgagaactgaccctcacatctcccttcctgaatttctttagggaaagcaacaaccatccctgtaagccatgggttttcatgcggaggaaggagagggctagttgtctgagagggtaactgcttaaggctgcagactaggaaatgggattccaggtttaagatagctcctttctggacctcagtccttcacctagt

SEQ ID NO: 339 - DNA, 181 bp, Homo sapiens
tccccaggcgggaggtaggcgcggagtgggttggaggcaaaggacctggctggcctttgcctggaaagttctgaaaacctcagcagtgaccgcagactaagactgagtggaaaggttcccgctagcgtttgtggctctaagtggcaggaggaggcggagcatcttgaacctgcagccctgg

SEQ ID NO: 340 - DNA, 601 bp, Homo sapiens
ccaaggcggccctccttccagtgctgccaggagagggaaaaggcactcagggagtttttgctggagataagagcaatttttgaaaaaaaggtagtaaggcaggaggtggagtctgccacgggtctctttcaaacttgctactttccatcccgttaatacaatcccggccctgtttcccggccccgcggccattgcagagtcatgaagtcatcgcagctgcgcctgcagccaggcgggaacgggaacgggaactggctggccgcggtcccttctgtcccccgccagccggaaatgtccgcgcgctgaaaagcagacgctgcctgcccggggaacggcgagagagagcgagaaaaaaaaaagcctgaaggcggcgcggcagccagcgagaggggagaaacagattcacacccaggggcctccgggcagggcccacgggactcaggccgtgtcccgcttggaatgtggagcaggcgcggcctcggcgtcagcagagctcccctgcatctcctcctgggggtgtgggggccgagtgggagaactggcggacagaggaaaggggcctcgctcgcaaggcccgggcggggaggcctggcctcctgct

SEQ ID NO: 341 - DNA, 181 bp, Homo sapiens
ctttcccagggcccccagagacggcccccgcaggctctctccgcggccggggctgggcaggttgcgggcttagggcggcgttgtctcatccggcggcctgggcaggtgcggcagggccggcgctcacgcgggcctgtgtgtccttggcccacagagatggacggcgatggcggccgccgag

SEQ ID NO: 342 - DNA, 661 bp, Homo sapiens
gaaacgcgggaggcgaaggcgaggctgctcaggggcggctcgggccgcctccagggacggggacgagccgtgcgcgccgggggagggggaggcgctggcgctgcggcggccgcggggagggccaccttcccagcacacgcacacacgcgcccccggccctccgctgcgccagctgccgctgcccgccgaccgctgacctccaggcaccagagcgcccggggacagcgatctgggaaccgggaccgcgcgctggcacacgcagtggccgccgccgctccgccgagcgctgcctgtagcacctgcacggtggtttggaaccgcttctcggaggtctggccgggaaggtctgggcaggagaatgttccacgaaggcgtcccagaggcatctgcagcctacgctctcccgttcttttctggcgcccacgagcccctgaccgagtcccgggggtcgctgaagacgcccacgggtgctcgaacgcccgttggtgccaggctgcccggcctttagggccttggctgaggacacccctttcctccccaccagacggagcgaccgccctttgccaaccccaagcaaagctggggtcccaaccttacgtgcgctaccgccccctccaggcatttgacctccccgcgtccccattcttgatgggccccgccc

SEQ ID NO: 343 - DNA, 721 bp, Homo sapiens; identical to SEQ ID NO: 116

SEQ ID NO: 344 - DNA, 301 bp, Homo sapiens
tgcaccgctctctcagcgctgaccacactggtttgtaaatgtttcgtttctggctcttctcttccaccccttccaccttcccagagttggggtcccggggttgggtgtgggggaccaagaagatttgcctctgcgtccccagggcgggcacccctccacccgggggagcattcggaatcgcttgtgtgtgcacggaggaaacagtccggcaaaaaggctctggttacagcctgcctgccttggcaaattcaagcaactgtcagttgaaaaaaacagcgttgggttggactgagtgcaggag

SEQ ID NO: 345 - DNA, 316 bp, Homo sapiens
tggaaaaagcccctgaccagcgcactcaacctgcgggccgaagggctgctctccggccagcctgggcgccggggacagcagccggcgcggcgtcctacctggtgaagttcgtcctgccctcggcgtggacccaggccccggtcgccgcccgggagggcaccggcctcgctcgcttgctcgctcgcccgcccttgcccgctcgctccccgcccgccgcctccctcgcgcgcccgctccggtcctccggctcccactacagctcattccaatatggcatcctctctgtgcgcatgctcggcgctcttttttttttttt

SEQ ID NO: 346 - DNA, 181 bp, Homo sapiens
gcgggtgagactatggagcagcgtcttcggcggccgcggcggcagcagcagcagcagcttctgaacgcgcctcaatgagagcggcggtggcggcagccgggccgagagacggactcgggctgactccagccgctgggagcgcgaggccatgtaacccgctcggctccaggctgcgaggtgc

SEQ ID NO: 347 - DNA, 181 bp, Homo sapiens; identical to SEQ ID NO: 124

SEQ ID NO: 348 - DNA, 241 bp, Homo sapiens
cctgtctgtgcacgcacacacacattcccaagcataccagcctcccctgagcctggagcccctgaagccatgagcagcctgtgctcaggtggcccccaccctctccacacgggagcggctacagccaggtcacggatcccctccctccccagagagaaggggcaggctgggggatgaaacctaggctcagtgttccctcccccgcatcctctcctggcactctccagaggaggaaggggag

SEQ ID NO: 349 - DNA, 1561 bp, Homo sapiens; identical to SEQ ID NO: 129

SEQ ID NO: 350 - DNA, 301 bp, Homo sapiens
gccccagcccgccccgctaactggggctcaccttccctaagccttggcggggaagggcgaggcaggttctcctcacttcccaaactgggaaactgacgctccgggatggcgctcgccggaacccggcccctacccagcgctgggagcccgctctccccgccaccggagcggttcacctcccaattctttgcatggcttgccctagcgatgcaaagaattgggaggtgaacccagcctactcagcccgtaagtcactactgaaatgtcacctcctcaacgtgtcttcctcaaaaccacccgc

SEQ ID NO: 351 - DNA, 661 bp, Homo sapiens
ccaggggtgggaggacacttcgggcccagcgtagaggaggcctccgaggcccaagcgggcttcggctgctgcgagtccccagaggctccctcgggcctcactcgcggtgtctcctccagacgccaggggcaggccacgaagccgagggctccgcgtggccgtgggagaagcggggtgcacggagccttcccgcgcccagacgccgaggggatgcaaacaggggagccgggcctggtatggccaacctccaggatcgaggggccccagaatgtgcgtgtggccgggggcgggggcagctgcgggggccagaactagagtattccttcgctctcccctgggggccgggcccccacgagttgcagcagagcccgtctgtaattagggcctcctggtccggcaaagctgcggctgctcccagagagagttggggtcttctcagggcccgcgatgggggagtggtcgtggtcagacccccgtgagccccttcggaaggtcccagtccctgtccattcttctgtcccgcagctctctccgcgcaggcggggcagagccggggaagaagacgctggacgaggggtcttggggccgcctcgctggctgcggttggaagcacccgttttcccgcccgcccgcgcaggcgctgctctgtggccaccagcag

SEQ ID NO: 352 - DNA, 301 bp, Homo sapiens
gctcgcgtcgctcgcgtccctccggccccgcttagcgacgcgcgcggggaggcagcggctgggccagctccggggacgcccgcgcgctcgcttgctcgcgacgcggcggagccagccacagccacccggcttcgcgctcctccgatgtcctcatttactgcaattgtcttcggcgagatctcagagccagggccaggaggcgggggcggggcagaggagggagcaggagggaagtcctttccgctgctccaggtcccagctactccgcggagccgggcggccagaggcgagggcgccccaa

SEQ ID NO: 353 - DNA, 301 bp, Homo sapiens
cgcggtccggccattggccggcgccccccccccgcccgcgcgcccccgccggccgcgcactccatgaagggcccattagcgcggcaggtgcctcccgggctgtaaattcgccccgatttatctccccggggacgaaataaatccagcttggatgggagtgtagttaggcaaaggttttcatgcgaaatcaggaaaaaatacgagaacgtattttattaacggaaagaatgcagatttgaggacccgcccgcgcgctcggagcgccccactcggggaagagtcccggcccgcgtcccagtcg

SEQ ID NO: 354 - DNA, 181 bp, Homo sapiens
cacacctcattggtccctggctaattcaccaatttacaaacagcaggaaatagaaacttaagagaaatacacacttctgagaaactgaaacgacaggggaaaggaggtctcactgagcaccgtcccagcatccggacaccacagcggcccttcgctccacgcagaaaaccacacttctcaa

SEQ ID NO: 355 - DNA, 541 bp, Homo sapiens; identical to SEQ ID NO: 133

SEQ ID NO: 356 - DNA, 481 bp, Homo sapiens
gttcctgtcctgaggggcggggaggagaggagggggggggtacgaggccggctgggcggggggcgctaacgcggctctcggcgcccccaggggccttcctgctgtgctggacgcccttcttcgtggtgcacatcacgcaggcgctgtgtcctgcctgctccgtgcccccgcggctggtcagcgccgtcacctggctgggctacgtcaacagcgccctcaaccccgtcatctacactgtcttcaacgccgagttccgcaacgtcttccgcaaggccctgcgtgcctgctgctgagccgggcacccccggacgccccccggcctgatggccaggcctcagggaccaaggagatggggagggcgcttttgtacgttaattaaacaaattccttcccaaactcagctgtgaaggctcctgggggctgatggggagtggggaagaggggtttctgcctcagtggccccaggccccccagccagtta

SEQ ID NO: 357 - DNA, 181 bp, Homo sapiens
gtccacgccccgcgcggctccctcgcgtcccgcgtcccgcgtcccgcgtcccctgctcacccggtggcaaagccggcgaggaggcggcggcgctggtggggactgacccggcagtccgagaatccaccgcggccttttcacccaaccgccccctcctgcgtgggggccccgcatcccctgg

SEQ ID NO: 358 - DNA, 181 bp, Homo sapiens
gggcgcggccgcggtggcccgagcgcggctgtcagcctggcggggcggcagcaccgtgcctcgcgccccgcgcagccctggcacccagcccgctgccccccgcatccccgctccgctccaacgctcggagccctcggtgccgcgcctgttccagtgtgttacaactcgacccaggccctca

SEQ ID NO: 359 - DNA, 181 bp, Homo sapiens
cacgccctcctcttctgcctcagcgaccagctctaccgaaggcagccatctccttcactgcctgcccctgcgcccgcggcatcccaggcccgtcttctctggcctccaggcttgcaacagcccaccgaggttgggggtagggggaatgttcctcagtcccaccttggtctttccaagccaa

SEQ ID NO: 360 - DNA, 601 bp, Homo sapiens
cttccaaaggggcctcctcacttcggagatgcagtgacaagttaatatgggcgtccaagcctctgtttcccaggaggaaatttgcaagaggcggcagcccctgagcgcccagagctcttgaaaggccacccaggagaggtgtgagacccggcggcagcatccgtccaggtgggacccgctgagcgccgtggccagtcccccattcccatcccggcaccccaaaggcgcgctcgcccgattgcttcgagttccccgacctggggattttttttttagccgctggtggtgggcgcctcgtgggctaaggcccggcgcctgctctgctacccgcgctgcctttagcggtcgcccccgccgccgctgccagggacgtgctgggaaagcccaagccccgggagaagatgccggccatcctggtcgcctccaaaatgaagtcgggactgcccaaacccgtgcacagcgccgcgcccatcctgcacgtgcccccggcccgggcgggcccccagccctgctacctgaagttgggaagcaaggtggaggtgagcaagaccacctatcctagccagatccccctgaaatcgcaggtgctgcaggggctgca

SEQ ID NO: 361 - DNA, 2041 bp, Homo sapiens
cctccacctctcgcattttcaaaggattaagcagcaatctccaggaaagaaaatcaatcccctccccaccatcccatccccagccaagctacggctccgccaccacctccgaggcccgccgccgccgcctctctatccgcatcccggataggggcgccaccaccccgcgcgtgaccccgctttcccgcgggtacagataaaaatcccctcacccttccgtagatgccatggtctggggaacgccccctcctcttcagcactatccggcagctgtgggcgagggagaaagcggacgccggggtgagcgcgaagtgcggccgggagcggtatttaagaggagcctctgcccgcccttccacccgcctccggggtaagccctttagcgcctcaacgggcgcaggaggctcctgcgggcgctaatccgcgtcccggctctccacggcgcgcgacccgcgctcccctccgcccgcggggatggcgcttggcggggagctccgggggctccgagggtggcttccccgagagagcgatgcgcccagggctgcaggagggcgcacgccggcgatgcgcccctgcagccgctgccacctgtgctttgctgcggggctcgcgggcgcggcgagtggcgggagcagagagtggtggcagaggacggtgagcgtgcgtgcgcgtgtgcgggtgtgtgcgcgcctggggaggcggtggaggccgctgcgctctggctcggcgccggccagggagggattgcaaggtttagccccgccggagctggggatttgcaggcgatccctctctattttcgtcgagagctgacatcacccgcgccgccgcctcgggcaactcctttaaccgccgccccccgcccccatctccagtcgcggtccctcctctgccatccctccccccagcctctcgccataaattagccaaataagaaaagaggccccgccgctcgtccgggaaggcttgggcagccggtggcaggagcccaggatctaaggagtagctattgtttcccctgaagcccgcgtggccccaggtcaccccgtgcggggtgaagcgcaggcgaccgcgcggagacccgggatgcccctccgtctccgcctccctggagcagcccctggcgctccctcctcactccccggagcacccgcttcagctcacactcacccccaaactcacaggcaggcacacccaccccatcctcccacgtctgggggtcccaggtccagcggagtcgagcggctgaaacacgcgggtggtgcagcctaaacgcggcccagctgcgctccctcccccgccgaagctcgaataaatctctggccttcaattattcagcgagattaatattaatgcagctccctgggggcggcgggcggggtgcaggggaggccgggattttttttttttttttttaggccgagagaggtcggcctcgtgggtgccggctgagaaggcgcggagagttggccgaggggtgagtggcgggggacggttctccacccactcggcgctgctcgccgcctgcttccgtgtcccgggggcggcgcacagagacagatgggcttgtgcaagggagagttcgagccttccggacgcctttgcataaaaatgacgagacctgtgcagctttgattatctctggaatactgcaggaacctagggtcccactacttgccgaccctgtgagcgcagagcaggcaaagcctcactttcctcgtctaggcaatggaacccaaaagaactcacttggagggccacaggagaattaaacagactctctttttccccggggtagacgatcttcggatttgcgctgtgctggaccttgttagacgatggaacgcgaccggccacgtgcaaactctctgagtaggtcccggggatggtgccagaggagccggagtcccagcaggaccgattggtagttaaatgccaggcgctgatatccgaaggcttgagttcttcaccaccttctagctgagtaacctggggcaaattcctccatctctctcttcatcccacctgtaaaatgggacta

SEQ ID NO: 362 - DNA, 541 bp, Homo sapiens
tgcggagaagcagctccactccccagccccaagtcttgcgggcagttcccgaagaaaagatgggtttggggcggtcgcgaaagcggcgcctcgcgtgttttcctgccgttcccgggtccttatagcccggccggagactccgctgagttgactcggcgcccggggtcctgccaggggtagtgaatgctgggaactgagataacgcaacgtggcgtttcggactccccgctggaccgggccgtggagaggagctgcgttcccacagggcatccctaagcgtcctctgtccccgcctatgaggacacaacctggaagtccaggccactggttgccgccttggagttggatgtaccgtgaaagtgcggccccgacgcaggaagcaggcaccttcccccgcactatggaagctcgcgcccctcgcttctcgaaacacctgattcacggcgtcgaccctgcttcgctgggtctgcggacattgggctcctcagctttccgccacagggtgtacgcgcccgggcccaggcgggtgtaggtcccacgt

SEQ ID NO: 363 - DNA, 478 bp, Homo sapiens; identical to SEQ ID NO: 137

SEQ ID NO: 364 - DNA, 346 bp, Homo sapiens; identical to SEQ ID NO: 141

SEQ ID NO: 365 - DNA, 301 bp, Homo sapiens
ggcagagagggtgggaatgggggagaagcatgaaccagtaggaagggggggcagacagagagaaaagtcacagttacaatgacaggaacagaaacacggacagtcaccaagggccagacacacagcgggggtcagggctgcaaaccgagaaggcagaacaagaagaaatcgagaagaagagcagtcagacaaggaaggaagggctcgctggggctgcagtcagatgtgcatgatggctcaagaggaaatttttttctaaaaaaagtctttttgattaaatgactcaactaaaaaaaaaaaa

SEQ ID NO: 366 - DNA, 661 bp, Homo sapiens
aggctgattcgtcacaggccgtcagcgcgggccacgcctatttcctctccaggttctaattaggtcaggggccctacagcctcttgggtagtttgcaagtgcgtcgcggagccggcctcggaaatatggcgacagcttcagctttcagtgtgagggagccgagggcccagccaaaccctgcgggaggcaattcctgggtacccttcccatattttcggtctttgggctgcgccgtggtaacctcagagcctggttgcgtgctcaccagcgacaagtgtctttcattgggacatgaaaggggactgggaagtgccgtgcagtttcagggtggtttctggttaattacattttcatgggttttcgcagagtctgggggcaatttgtgtcctccagagaccagggaccagggccgaagctacggcaggggagacgcggccagggccgtggcttctagtgcgagctcggttcgcgtccgttcccgtctggcgcccgggcctccgggagcccagggccttgaatgagacagtgctcgtccttgaaaaagcagttctaggtcactcggcctgctttgccagcattccgggccccagctcaccttccgccatccatgttgacaacaccagttctacgacgaagcgggcgattcctcttgcctggaatt

SEQ ID NO: 367 - DNA, 181 bp, Homo sapiens
cctcctcggctcagcctgggcccctccccatccaacatccactccagtcctcattcaacttcctcttcctgcgaaagaggggcgctgccccgtgacctacacagactgagacacgatcgccatgaatggagacctctggaaaagctcaggagccgaggcccacggggcccagcagaggcct

SEQ ID NO: 368 - DNA, 1225 bp, Homo sapiens; identical to SEQ ID NO: 150

SEQ ID NO: 369 - DNA, 721 bp, Homo sapiens
gtgatgaacataagacacaaatagagccaagatcgactttcttaggaagggggagaggagggaactcttcacgaagggaggtgggagtccacctcagacctctattggaaggaaatcgagttgttccgggggactgaggtctcttgcataaggcatgggatccttattattattattattatttttaaatcccccgcggaggagctctgggcaaatgaataccgaggcgccgctctagctggttaggcttgggatgcgataactcagtgccctcttgcagacttgcatagaaataattactgggttgtcgtggaggggacacgagacagagggagttctccgtaatgtgccttgcggagagaaaggtccaagaatgcaattcgtcccagagtggcccggcaggggcggggtgcgagtgggtggtggagtaggggtgggagtggagagaggtggtttctgtagagaataattattgtaccagggcccgccgaggcacgaggcactctattttgttttgtaatcacgacgactattatttttagtctgatcaatgggcacaatttctaagcagcgcagtggtggatgctcgcaaacttttgcgcaccgctggaaacccactaggttgagttgcaaaacgtaccgcgtagacgcccctggtggcgccgagagaagagctaggcctgcccagcacagagccggagagcgtcgggccttccggaag

SEQ ID NO: 370 - DNA, 701 bp, Homo sapiens
aatttatgttgaagggtcctgcaaataacaaaaatagataaaacaggaaaatgaatttaaatctcaccctttccaaaactttgctacaactcataataacaagggtaataaatgcttacgaagcagaggtcaaacgggaaacattagcaaacgaggagaggcgcaggagcccaggatcatgcctcgatgcccaccaagttgggcattaggtcactatcagagagaaatgcagccagccacttcagctatggcttcagctgaggcaaaagctgtgctgccaagttgctgaacctgctctttctccgttcctttgagattcattaaagaaagttcagaaacacaactacatgaggtgaggataagggcatatgcagacccccttcaataaaacttactttcatctactcccatccatatccaaatccctcagcttgggtggacaaactttccagagagggtgactgaaaataagatactccttctagaaacaactggccgaaggggcaccagaaaactttctatgctccaagttgaggtaagctaccaaattgggccccacagagggtggcctgaagtctcagaaacacagctgcacaaggaggaacgcgtcagccagaaggcagggagagccagaggaacatggtgtccagcgtctcctaaccaggatctagccgagcagagaaaacattcagcctcctccc

SEQ ID NO: 371 - DNA, 901 bp, Homo sapiens
attagtaagcaaatcaccacccacaactaaggggacagcggaagccagcctcagatgactgaaacccccaagtcagtagctctcctcaaaatttccggcgggttattatagataatgacttttcccaccgccctaagcagccgaagcttgactcagtgatgattctctctatcccgtaactgcgaggaagtgggcgatcagcaaattgcccttttgcaggaggctggggacgcccctggaagttcgctttcattctccaggttttctgccttttcccttcccccttcctgcaacgcccccgcgcctcctcagcctggggatttcctggcgcttcgccggccctctccgcaaccccctgataaatcggttcagaaccagtctggctgggaggcccgagggctgacagcagcggagcggccccggccggggtctcacggactctcggggtctggccgacacggccgctcccgtcactgcagcgcgggctgagctcacggccgcgcgcccgccgccgccgccgccgccgccttcatgctgcagcgcagggctcagttccacgcggccaggaggccgccgttgcccacacgcgacgctttgggaagcccagctcccgggtccgccccggccgcggccgcagccccggacctcggctgcttgcctcgcgcctgaactgcggactcgccccagcgcggtggccagcgggcggggcgctgtgttccgcggcgcgcagggaggcggtgagcgtgtgcagagctgcccgaacggaggactatgtatgtgtgtgcgcgtgtttgcgtgtgtttgagcgtgtttttccttcttcccttgaggatgtgaattgtttagcagctggctgctcccttaggatccttgactttggggagctctggctgtgaacaca

SEQ ID NO: 372 - DNA, 241 bp, Homo sapiens
ggtgtctggccggcgcggggctcgcccagcctggtccggggagaggactggctgggcaggggcgccgccccgcctcgggagaggcgggccgggcggggctgggagtatttgaggctcggagccaccgccccgccggcgcccgcagcacctcctcgccagcagccgtccggagccagccaacgagcggtgagctgcgcggggcgcgggggacgcggctccggccgggcaggggagagggcgc

SEQ ID NO: 373 - DNA, 421 bp, Homo sapiens
agtcagggaggaacctcatttacataacggccgcccctctgtctcctggcgggggccggagtcccgcccctcgtccaacttgaaatctgttgggtcacgggccagtcactccgacctaggcaagcctgtggtggagctggaagagtttgtgagggcggtcccgggagcggattgggtctgggagttcccagaggcggctataagaaccgggaactgggcgcggggagctgagttgctggtagtgcccgtggtgcttggttcgaggtggccgttagttgactccgcggagttcatctccctggttttcccgtcctaacgtcgctcgcctttcagtcaggatgtctgcccgtggcccggctatcggcatcgacctgggcaccacctattcgtgcgtcggggtcttccaacatggcaaggtgga

SEQ ID NO: 374 - DNA, 421 bp, Homo sapiens; identical to SEQ ID NO: 157

SEQ ID NO: 375 - DNA, 181 bp, Homo sapiens; identical to SEQ ID NO: 159

SEQ ID NO: 376 - DNA, 319 bp, Homo sapiens
cgggtgtggtgggcgtcccgggtgcgcggtgggcggcggcccgggggtgtggtgggcggtgtcccgggtgcacggtgggcgtcccgggtgcgcggtgggcggtgtcccgggtgcgcggtgggcggtgtcccgggtgcgcggtgggcggcgtcccgggtgcgcggtgggcggcgtcccgggtgcgcggtgggtggcggcccgggtgcgcggtgggcggtggcctgggtgcgcggtgggcggcaccatccaggcttgctgcgatgttggcaagaggacgaggtctcctcaccatgcatgtctcagaacatacctctgtcgt

SEQ ID NO: 377 - DNA, 841 bp, Homo sapiens; identical to SEQ ID NO: 160

SEQ ID NO: 378 - DNA, 181 bp, Homo sapiens
gccagtggcctctagcccgctgccgaggcgccaccttcagtactgcggccaggagagtggcgctcccctcttataccgtaggctgagtcccgcccagccgccagcggcccaacccggaggtgctgcacagcccgccttcccgccaccctctcccacgacgccgggaggtctgcatgcactg

SEQ ID NO: 379 - DNA, 241 bp, Homo sapiens
caaggtcagaccctttggctgcaacacgtccgtcaagaagccaggcaaatctagcatgcaaactaggatcattttcgggcgttggggcccccccgcttgaaatctggtttccatgttcacaaaacgcagcccgactggtggaactcgcgactccagacgcagagaagctgtgggcagaggcggaggcagagggtgggaatgcagcctggcgttggagtggggagaaaggggagggaggaac

SEQ ID NO: 380 - DNA, 181 bp, Homo sapiens
gcaggcccgcactgggcttcatccccactcgggacaggcagtggctccattgacccggatgagctgcgcactgtgctgcagtcgtgtctgcgcgagagcgccatctcgctgcctgacgagaagctggaccagctgacgctggcgctcttcgaatcggccgacgcggacggcaacggggcca

SEQ ID NO: 381 - DNA, 301 bp, Homo sapiens
gcggcttgaggtcctgctcgtccaagccccgcgggatctgccccacgaagagcttgatggcgtcgtggtccttcatgggtacggcgggaccggggtttagcccgctcatgccgacgccgctgtccgcggtgctgaaacccaggcgcgggccggggccagcgggctgcgctgaccctcccggcgccgcggccatgtccccgccctgtcagccctcccgccggtcccactggtcccgcctgtcccgccgtcccctccctggaccggtggcgagggccagggggagggggcggagcccgggcgg

SEQ ID NO: 382 - DNA, 301 bp, Homo sapiens
agcggctgggccgcgccggacgggcgtcgggggtctgggccgcgaacccgccgcggggccgccggaacctccgcgaaggttctaggcctttgtggcgtcaccgtctccttgcggaagcttccgccggcgccgaataaaacccgccgcggaggagccggtggctctagtgcggtggagccaggcgtggaagtcggtccggcgcggggcggggggcgggcgggagctacaagcggcggcggcggcggcgaccgtgaccgtgacgcgcgagcgggcggcgggggcgcgggccaggggcgcgggc

SEQ ID NO: 383 - DNA, 181 bp, Homo sapiens
caagcccgggtcccgccgatgggcacgccctcctccctcaggctcacctgcccagccccatccctcccagtccgccacgcccccggggcccgccctgcgctcacttctccacgcccacgacgatgtagcggtcttgtaagaagtggaaccagccctgcatgagcagcgcccactggatgcc

SEQ ID NO: 384 - DNA, 241 bp, Homo sapiens
tatgcaggtggtgccgattaactttgaaaaaatcacgactgagccttcacgagtgaggcggggaaggaggaggcagcggaggttgtatggccccatcaccggggcaattcagaaaggctgtttctataaacaaatccttaaacgtctggtaagaaatgagtccgcgacggaacgagagcagatcgtggttcgcgtgtttactgccgagtgggacgcggactggggccggaccttccacaga

SEQ ID NO: 385 - DNA, 301 bp, Homo sapiens
ctgatctccccccgcaccccactgtctgaatacagaggccccctcctctctactggggagcccagacatctagcccttgccctgtgtggttctctccgggtgaggtgggagggacctgccgggagagacaacatccctgctgcttcactcacggtgtgaagccggaagggaccagactcagaccccctcccgggccagcctctccgtgaagcccctttctccagcaggagagtgtagctgcccctctgggtgctcaggggccttctcagcctcacctgaccctcaccttgggggtgggggg

SEQ ID NO: 386 - DNA, 361 bp, Homo sapiens
ggacctccaaggaggccagagctgtttctcccgtttggagagggagatcctagcctttctcaatactttttgatttctgggaaaggagaagttggaaggccgcctcgcctcctgtctcggtggcgttcaaggttatccagacagcggtctgcgggtttcatttgcaagtcactgcgcggcgcatgcagaagcagccgcgggccggcggggcgcgcagataaggtctgggggcgtgggtttcgggctgtacctgcattatcgcggcttccttaagctcggatgaatatgtaaatctctcgctgcagccttccggtgccgcagtcgcagccgtgggggccgcctccgctgtagcaattccgag

SEQ ID NO: 387 - DNA, 181 bp, Homo sapiens; identical to SEQ ID NO: 166

SEQ ID NO: 388 - DNA, 361 bp, Homo sapiens; identical to SEQ ID NO: 167

SEQ ID NO: 389 - DNA, 241 bp, Homo sapiens; identical to SEQ ID NO: 169

SEQ ID NO: 390 - DNA, 301 bp, Homo sapiens
taccaggagtttaacaaatatttatcgaatgaatgaattcattcatttacttattcaatcaagaagattgaaatcttacagtcagaagctgcagccacagaggcagcccaaagctcgtttattaaatgccggctgtggtggccgtgtcctgccagcatagtctggtgtggcctctatggcgccctcgggagggtggtgacaatatagcacaaggtgctcaagctcctgggatggcttcacctggaggctggggaggcagggtgggaaaggtgagcaccgtcattacatgagggtgactcct

SEQ ID NO: 391 - DNA, 334 bp, Homo sapiens; identical to SEQ ID NO: 174

SEQ ID NO: 392 - DNA, 181 bp, Homo sapiens
ggccaagaagtctttttctgggaggctggagctgcagcgccacctgcaggccaaggagtctttttctgggaggctggagctgcagcgcgacgtgcaggccaaggagtctttttctgggaggctggagctgcagttgcagtgaagtcacaggttccgtgacgtcacaggtgggcaggcgcac

SEQ ID NO: 393 - DNA, 181 bp, Homo sapiens
agtaaggaatcatgtcggggccaccgaggctgcaggtgcaagcgaggggcgccttcctcttgcgggccaacgtgctcagggtcatggggccggctcaaagtgcacaactccgcatcctggcctctgctctgctccggcacgaggcgcaggctgcgcgtgcacccggcggcggaggcgggcc

SEQ ID NO: 394 - DNA, 181 bp, Homo sapiens
aagatgacgtaaatgatgacttgtgagcagtggcctgcctctgttgccatgacaaccggagcttgactacttggcctttgcaaggttggccgaggcgggttcttcgttaactcgagattaaggaaggatatttaggggggagggtgtgtgtgtgtgcggcggattaaagacgaaaggagta

SEQ ID NO: 395 - DNA, 181 bp, Homo sapiens
ccaaaagctacatttttatccaagtgtgaagaatggggagagctgcaaagaaagcaacaagtggccccgggcggagccggggggtgggggcgccagcctcctcccgccggctgcgctgctgcgcctggcccccgcccccgcaggcatgcggggtgattcacctcgcccagactgcgcccag

SEQ ID NO: 396 - DNA, 241 bp, Homo sapiens
cataaccacctaaagaatggtgaaataaatgttcttggaaattcctacccggactggctagtccttgcggaagcagcgtccgggccctcgggtaacgtttgaagagctggcagcgtctcaggctgctgcgtggcgaaggggcggaccgggggacgggggggtgggcccttaggggctggggcgggacttccctgggcactgagtcaaagcttgaggggagtgttcgctcccgcattttcga

SEQ ID NO: 397 - DNA, 181 bp, Homo sapiens
gcaaacggcctcggccgagagcattcgctttccagatgagaatggcatcttcagggacccgctggtagtggggccaggtctccacagggccggtccagtccttcctacccacccgggccctgcggccaggcggggccgggaggggcggatgccggagggcgctgggggaggccgacccgcg

SEQ ID NO: 398 - DNA, 351 bp, Homo sapiens
caggcggagggtcctcagagtcgggggtggggggcctgtggggcggccccggcccacaccggggagtgcggcgaccagacggccagctgccgaatctgaggcctcggtgggtccgtcgcccgcctctcttggacaagtccaggcgatgtgagcacgcccagcctcctacatttcactcccgtctctcccaaacagacctagcgcaaaacgagcactgacacagcgggggcccacatcccggaggttctttagggagaggtcggggagtgcggttacctatggctccgaagtccccgctggcatcctgaaaggcatcgtatttctcgcttaaggcgttacccttgtggtagt

SEQ ID NO: 399 - DNA, 301 bp, Homo sapiens
ggagactctgtctgaaagaaaaaaaaaagaaatataagtacggtaaagggaaaaacaacaacttgctcgagataagccctgtttacttgggggcctcgcttttccatgtgtgtttgcccagctcatcctgaggctgcccacacggctgtgggtcctgctttatcacccagcagcagatgcctctgcggctttgtggccaaaccctggccctgcacagcctccttgtggcctgagcttattgcaggctgcacggtgcacattacaaatggtcagttggaggccaggcgcggtggctcacgcc

SEQ ID NO: 400 - DNA, 361 bp, Homo sapiens
tcagctcagggaggaagccctgcctgaaaaggctgcagcttaggctgttactctttcatcactcagcccagcatctgatcacatcctctgtcactcagggactgagtgggcggggccttaagcattatccaatcagagacgctgggctggaaaccgtccaatcaggcaggcagctggagcaaagaggacggcttccgggtttggcgcggcctttgtctctcgctgcatctggagctctaggtcgcctcttcgctactctgtgtcctctgctcctagaggcccaccctctgtggccctgtgtcctgtaggtattgggagatccacagccaagatgccgggaccccttagaagcctagaaatg

SEQ ID NO: 401 - DNA, 181 bp, Homo sapiens; identical to SEQ ID NO: 185

SEQ ID NO: 402 - DNA, 421 bp, Homo sapiens
tttggaccgtgattgtaaagaagctgttctaaacccgtcggggggcggtgtttgcagggagggaagtagcgtgaggcaggttggggaaggcgtgagaggcctaggagagccgaggggcggtggaggggtgtggcctagaatgttaggcggagcgggaggtgggccgggccttcggacgccctgtcccgcagacgttgacgagtgcagcgaggaggacctttgccagagcggcatctgtaccaacaccgacggctccttcgagtgcatctgtcctccgggacaccgcgctggcccggacctcgcctcctgcctcggtgagaggccccgccccggcctgatccctcctcccttcgactccccgactcgccgattggcctcccacctctgtctttcctcctccgcttctcccctccccttacct

SEQ ID NO: 403 - DNA, 541 bp, Homo sapiens
ctgttggctgcaggatgaacctccattctaaccttacgctttagcgccgccccgccctctctcggccgtttgcacctcattagctggagtctctattaggccccgcccccatttgcccgcctctaccatttacccgcccagcctggagcgtccgggccggcaagtccagcgccggggcctcactgtttccgcgtgtgaagcgttcgaagactgccatggacccgcggccagagaccgcatccgcctgtagcactaacgcgtcccgcagcgctgcgtagccgcacagccccaccgcagggcgcgggcccagccgcactgtgaacacccggccccagcggccggagagctacgggtagccggtgctcagcgggtgcccatagggttcctcatcggagccattgcccccagctccctcttccttcagacccaggagtcctcgtctcagaccctcattcctcaggcccaggaattcaaatccccagctccttcctccctgagatccaggagtccaggcccccacttccttcttcccttaggacct

SEQ ID NO: 404 - DNA, 361 bp, Homo sapiens; identical to SEQ ID NO: 188

SEQ ID NO: 405 - DNA, 356 bp, Homo sapiens; identical to SEQ ID NO: 189

SEQ ID NO: 406 - DNA, 181 bp, Homo sapiens
gaatagacttacgtggaccacttatgatagaaaccaaaatgatttcctcttaccaagttgaaaacggtttatgttaaaattgtttgccggcgggttggacccagtcctgctagggagtctgctgcagctcaggaacggggatctgggaatcggggatctcggtctgggaactgggatctta

SEQ ID NO: 407 - DNA, 181 bp, Homo sapiens
gccatgggggagcgcgcgcggggctgttcgctgggcgtggcgggcgggtgtggccaggggtgtgggtctgtgagggaccggtcggaagggcgtcgcgcggcctcgggtgacatgcggggggcggcgagcgcgagtgtccgcgagccgacgccgctcccgggtagaggcgccccccgcacaa

SEQ ID NO: 408 - DNA, 181 bp, Homo sapiens
tgctcccaacaggcacctgtggaccccagattccatccttctggctcagttcacttccaggcctttgcccgcgccagtccctgtacctgccggtctccccaccgcatcccacgggtgtcagaaatggggcccctcccgcaagcgcctcagtgtcccaacgccggcgtccgggctgcagagc

SEQ ID NO: 409 - DNA, 721 bp, Homo sapiens
cggctgcatcagctttctagacaacgggagaaaagagaaatggtggaggaggggaaatcctatgccctcctcctcgcggaaatcaaggccgacctccctgacgcccccccggaaggaagcgcgtggtcggctgccagccgagacccccatctgcgcctccagctgcagggcctttgctgggcggttcctcgcccgcaattcccccacgagccctggggagacccagcgctaaccaggggtgcccaagggaggagccgggagaggccctcctggaggtgggcacagcccaggcaaacatcagcagacggaaccagcacccgggacccagggaaacgtcacctgccaccaggagctccacagggtcgctgagctccgattcgaaggtgtggggcacccaggagcggtagcggcacctgtagttgccggcgtgctggggccccacgaagatcagctcgaggttcgccgcggccccgggggtgcggaccgtcttcacggccttcgtctcgccctcgcgcagcagctcgaaggtgacgtcggggatgggtccctcgcagcgcaggacggcatctcggcccgccaggaccgccccactccacgtcgcccggagctgaggcctgggagggggtcctgggcggagcgggcgggtggtcgggccaggccacgccccaggccacgccccaggccacaccccaggccacaccccaggccgcgcccgcgcctg

SEQ ID NO: 410 - DNA, 601 bp, Homo sapiens
caccaggaggggccgggggcttagcgccagggcccgggggatcgccgtggatgcgctggtgctgcagcagattggagcgctgccggaagctctggccgcactcagcgcaacggaaaggctgttcgcccgtgtgcactctccgatgctcttccaggcgcgcgctgcgcacgaagccctggccacagtcgccgcacacgaacggccgctcctcggtgtgcgtaagctggtggcgcagcaggtgcgagctgcggctgaagctgcggccgcactcgctgcacacgaatggtcgctcacccgtgtggatcttctggtgcctcagcaggttgctgcgttggctgaacaccttgccacatacatcgcaacggccgcccctaaccaccccgcccccagtgctggggcggccccggctccggcccctgggggagcgccagcgggtggtgatcagagcagggcccacaccccggcagggatcctcgtccgtggggtcctgttcactcctcagatcgctggggagcagaagcgcatgcgcaaagccaccttcgcgggagggtgattggatctggccagaaaggccagccatgccgaggtcccaggggacgtg

SEQ ID NO: 411 - DNA, 421 bp, Homo sapiens
gcaggggaggcactgcggggacgggcggggtgagcgggaggaggggagccgggagtcgaggggttggaggggaacgcagcgaggcggggatgctggggtccagggctcggagtgcgggcgggacaccggggctgcggctgcaggcacgctcgggcgccactgggcctcgaccgcggtcacgggcggggcgtccagatctgctcggcaccttggtttcttggatgacctctcggtgacagccctcagcgtcctcaccctcagctagggacgggtctcccgtggactacagcgtggggaacccttcctcgagcctcggggtcatcgctggtgggcgccactgttgcagctgccccaccctccaccactccagacccttcctccttcctcctcgccctgctgcggcttgagcccgggcccaccc

SEQ ID NO: 412 - DNA, 301 bp, Homo sapiens
actccccgagacagggacccggagacgtgggctttgtcagtttaacagattctgcctccgggaaccaactgccgggagattctgattggctcagccgcgtgcccacgtgaccgaccaaaaccggccaccagggtctcccaactgcctgtcaaacgcacagccctgttgggcccccggagaggaagagccgagaaggaggccaggccgggggtcaggtggcttcctctatgggccctttaatccacctcacttttttatcttcttttttttcccagcagctttattaagttataattcacac

SEQ ID NO: 413 - DNA, 301 bp, Homo sapiens
ccaggagccctgagccttggccctcaggccccaggagggaggtcaggagggaggcgtggacaagggtccggccgtagctggtcccgtcctggaagctgcttaagttcctggttcccaccggggccaagagtgatacctgatcctgggggattgtgaaatgacctcatgtggcagcccgcccgcggtgcccgcaaagccctccaccctccccttccccgctcggctccacccctaccccacgccccctcccgcgcgcgcggttaaatccccgcacctgagcatcggctcacacctgcacccc

SEQ ID NO: 414 - DNA, 421 bp, Homo sapiens
gcccctcgacccaggggacgggatcctgtaagtctcacctgcctatctccatcccaggcctcgggcacgagggtggttgtactatcctggttatggtagctccactcgagcaagctttattttaacatataagctattcgtttagtggaggcttcattaaactactcccctccaccaccacctcgggaagttgtggtcaaaacccaccagaccgactgtggtggaagttgatgcggaagctggagagcccgcggctctggaggggtgagccgccccggagaggggacccatcctcctttccgcgcccggaaagagcgggggagaagaggaagtccagttacaactcctttcctcagccccttaaaggaaaggtatcagctaaccacggggagctggcagcctaagagaaagtaggaaccta

SEQ ID NO: 415 - DNA, 601 bp, Homo sapiens
catcgggccttgcagcagcgccgcagatattctgcctcccattttgcccgcggggacgccgaggcccggcgccgcatcctgccgcccgttttgcccgcggggaagccgaggcccgatgccgtaccctgccgcccgttttgcccgcggggaagccgaggcccggcgccgcatcctgccgcccgttttgcccgcggggaagccgaggcccggcgccgtatcctgccgcccgttttacccgcgaggaagccgaggcccggcgccgtatcgtgccgcccgttttgcccgcggggaagccgaggcccggcgccgtatcctgtggccgttttacccgcgggaaagtcgaggcccggcgccgtatcctgccgcccgttttacccgcgaggaagccgaggcccggcgccgtatcctgccgcccgttttacccgcggagacgccgaggcccgatgccgtatcctgccgcccgttttacccgcgggaaagccgaggcccggtgctgtattctgccgcccattttacccgcggggaagctgaggcccagtgctgtttaatatcttactcatgttcacttgatgagaaagtgacagatctgagacaaacccag

SEQ ID NO: 416 - DNA, 361 bp, Homo sapiens
acgcgtcgccgaaaagccaggcccggaggtgcctaagtcagggaccgagacgcaaacatagacacaaggatgcacaagcacgccctccccgaagttgacaaaaatcagccgataaaatacaaagtgccgcggccgccgcaggtcagcgctgacctcctgctgccgagaggaccgaatgccgacgtccggacgctgtcatttccatccagcgaaggcacctgggctgcacggtctcgtctccctccttcgcgcgagggatgcctcctcctgcctctcctccccgcatctccccacctcccaagtgtgtgaacacgaaaacaatacgtggaaagcccgatcggggggagctaggacccgccgg

SEQ ID NO: 417 - DNA, 181 bp, Homo sapiens
aggatccccctcccccaacctgcttcaagggtagccctgttcctgtctgccctccccgcccccacagaaatagagatgagaaggggcaggcgaagaactaggagtgtctgcgagaccatcccaggaccctgagccccccaactctctgcatcccagggctgacttcgacatgaagcgcctc

SEQ ID NO: 418 - DNA, 181 bp, Homo sapiens
gcccccaccccagccttggatagggtagtatacgatagggggcgtaaagaagggtcatgggctccggtggtcgcaggtcccaccggcaaccgccagggcgggggcagcaggagcaggaacctgctcgcctccgcatctcgtcggctcccctctcccgccagactcctgtctctgcgccagg

SEQ ID NO: 419 - DNA, 181 bp, Homo sapiens
cctccccttcaaaagccaccttggcaaggcattagctaaacatcttctcggtcccagaaggcttcccctgtgaagtctgcagcgttcaaacgacaaccagcaaatccccagagacaggtccctgggaattagctgcgccgggcgggatgaaagccgctctgatgttctggagcgagagagt

SEQ ID NO: 420 - DNA, 241 bp, Homo sapiens
ccgtctcaaaataaataaataaatacatacatacataaagtaaaataatgaataaataaaataagaaatggggaaatggatcagcaagaaagtgcccgccccaggcatgggtgccgtgcgggacggggacgcggcccagccgggaatcggggtgcccagggtgcgatgtgcgaggggctcctgagcgcgtgtgctccgcccgaccccgccctgtccccccgacacacaggtggacccaggg

SEQ ID NO: 421 - DNA, 181 bp, Homo sapiens
agcgcgcccctatcctgcacgcatccgcggccccgggccctttccgcagccccacgcggtctcctcccgggttaaatctatccactcgcgcgttccttggcagccgtgatcacaggcgtgaccacggtccccaagccctcgcgcctccgtccacgctattgcggccgcccctgcgcgcctg

SEQ ID NO: 422 - DNA, 808 bp, Homo sapiens
tgatccatctgggccctccaggtgcaacacctgacaacatccatcggcaacttcgtccatgaacacatcacgccggggactcaagcacgttaaactgctccaattggtagctaaacgagagattgcaaaacatgcctctactcaacggcttaatgtctgagcacttacctcccccgctgctctgccgttgggagcactggtctctgggtgagggacttccagcaagaagtattcacaaatgaaacaaaagctcagcaaacttgagctgaaggcaggggaaggagagctgcttcctgaatatcaatgaggggaggaatcgggtggatcgtagaaatgtttcgtgttggttgtgtaaaccactgcctcggagctgtcagaacccaactaggaaaggaaggggccctgcctgtgccactcgccacagagctcgggtctctcagaagaaagaagcgtccctaagaatagaatcccaccaagtacacattctgagcaggctctgtttctgaaacgtaactgtttactcgaaggtcttctacatctttccaagtagcctttttccatcccccacagccacacggtgggaacctccttcacacggtcacataagcattcacgcactcggcttagctgtgtggccttgggcggctccggattcggccctgtggtttgcgtgggcagcccggatggctggtgggcccggtcctgctgccccctttatctctgctcaccaagcagagaaaaaccacagtaatgtgtgtcgcccagagacactggcaccctgacaactacagcaacgggttctttgtgc

SEQ ID NO: 423 - DNA, 421 bp, Homo sapiens
agtcaggagcgggcgagctgtatttttatgctaaaatttacacaaagggacggccccaggctctccctcctttacaagctgtggtcagtcacgccgtctggccgaggaatccggctttcacagggggaagcaaataataggacggggaaaccgcagggtccttgggcactcagagctgtcactcatcacaaatccataaaacaattcgtgtggaagtaatgatattgtttaaccactgtatttttgattaatgtataaataatttaactgagtatttcttgagttttcagcgtgtctgccattatttaccggccctgtcatgacggctgctggtgctctgccatataaaacatcctcaagtccgtccgaggaggctggtgggttgttaatggtcttagggggaaacggcattgcagctatt

SEQ ID NO: 424 - DNA, 241 bp, Homo sapiens
aatgaaaaaaatgcataacaacaaagaatatgaatatggatcacatctctaccagagttaatcaactgatgcaaactcttgcacaaatgctgaaagctgtaccatacctgtctggtcttggctgaggtttcaatgaatggaatcccgtaactcttggccagttcgtgggcttgttttgtatcaactgtccttgttggcaaatcacacttgtttcccactagcaccataggtacatcatccg

SEQ ID NO: 425 - DNA, 241 bp, Homo sapiens
tgctcctagtacctgtagaggttaatatccgcaaatgacttgctattattgatggcaaatacacagaggaagccttcgcctgtcctcatgtattggtctctcatggcactgtactcttcttgtccagctgtatccagtatgtccaacaaacaggtttcaccatctataaccacttgttttctgtaagaatcctgggggtgtggagggtaagggggcagggagggagggaagttcaattttt

SEQ ID NO: 426 - DNA, 241 bp, Homo sapiens
caagtgagagacaggatcaggtcagcgggctaccactgggcctcacctctatggtgggatcatattcatctacaaagtggttctggattagctggattgtcagtgcgcttttcccaacaccacctgctccaaccaccaccagtttgtactcagtcatttcacaccagcaagaacctgttggaaaccagtaatcagggttaattggcgagccacatctacagtactttaaagctttctataa

SEQ ID NO: 427 - DNA, 241 bp, Homo sapiens; identical to SEQ ID NO: 426

SEQ ID NO: 428 - DNA, 241 bp, Homo sapiens
ttgcagcaattcactgtaaagctggaaagggacgaactggtgtaatgatatgtgcatatttattacatcggggcaaatttttaaaggcacaagaggccctagatttctatggggaagtaaggaccagagacaaaaaggtaagttattttttgatgtttttcctttcctcttcctggatctgagaatttattggaaaacagattttgggtttctttttttccttcagttttattgaggtgta

SEQ ID NO: 429 - DNA, 301 bp, Homo sapiens
tatagcataattgagagaaaaactgatatattaaatgacataacagttatgattttgcagaaaacagatctgtatttatttcagtgttacttacctgtcttgtctttgctgatgtttcaataaaaggaattccataacttcttgctaagtcctgagcctgttttgtgtctactgttctagaaggcaaatcacatttatttcctactaggaccataggtacatcttcagagtccttaactcttttaatttgttctctgggaaagaaaaaaaagttatagcacagtcattagtaacacaaata

SEQ ID NO: 430 - DNA, 301 bp, Homo sapiens; identical to SEQ ID NO: 429

SEQ ID NO: 431 - DNA, 241 bp, Homo sapiens
atttaaacccacctataatggtgaatatcttcaaatgatttagtattatttatggcaaatacacaaagaaagccctccccagtcctcatgtactggtccctcattgcactgtactcctcttgacctgctgtgtcgagaatatccaagagacaggtttctccatcaattactacttgcttcctgtaggaatcctgagaagggagaaacacagtctggattattacagtgcaccttttacttc

SEQ ID NO: 432 - DNA, 241 bp, Homo sapiens
aagaatggtcctgcaccagtaatatgcatattaaaacaagatttacctctattgttggatcatattcgtccacaaaatgattctgaattagctgtatcgtcaaggcactcttgcctacgccaccagctccaactaccacaagtttatattcagtcattttcagcaggccttataataaaaataatgaaaatgtgactatattagaacatgtcacacataaggttaatacactatcaaatac

SEQ ID NO: 433 - DNA, 241 bp, Homo sapiens; identical to SEQ ID NO: 432

SEQ ID NO: 434 - DNA, 241 bp, Homo sapiens
tataagatattattttattttacagagtaacagactagctagagacaatgaattaagggaaaatgacaaagaacagctcaaagcaatttctacacgagatcctctctctgaaatcactgagcaggagaaagattttctatggagtcacaggtaagtgctaaaatggagattctctgtttctttttctttattacagaaaaaataactgaatttggctgatctcagcatgtttttaccatac

SEQ ID NO: 435 - DNA, 241 bp, Homo sapiens; identical to SEQ ID NO: 434

SEQ ID NO: 436 - DNA, 241 bp, Homo sapiens
gctctggaatgccagaactacaatcttttgatgacattgcatacattcgaaagaccctagccttagataaaactgagcaagaggctttggagtatttcatgaaacaaatgaatgatgcacatcatggtggctggacaacaaaaatggattggatcttccacacaattaaacagcatgcattgaactgaaaagataactgagaaaatgaaagctcactctggattccacactgcactgttaa

SEQ ID NO: 437 - DNA, 241 bp, Homo sapiens
ccctcaaggagataagtgatggagatgtgataatttcaggaaacaaaaatttgtgctatgcaaatacaataaactggaaaaaactgtttgggacctccggtcagaaaaccaaaattataagcaacagaggtgaaaacagctgcagtaagtcaccgctttctgtttagtttatggagttggttctaatgggtcctttatttgtatttagaatattgaagggctattcccatttaaattactt

SEQ ID NO: 438 - DNA, 241 bp, Homo sapiens
actcagcagcatctcagggccaaaaatttaatcagtggaaaaatagcctcaattcttaccatccacaaaatggatccagacaactgttcaaactgatgggacccactccatcgagatttcactgtagctagaccaaaatcacctatttttactgtgaggtcttcatgaagaaatatatctgaggtgtagtaagtaaaggaaaacagtagatctcattttcctatcagagcaagcattatga

SEQ ID NO: 439 - DNA, 241 bp, Homo sapiens
ctccggctgaagcaccagtgcccatcccaccgagcccagacaccaaggaccggtggcgcagcatgactgtggtgccgtacttggaggacctgcacggcgcggacgaggacgaggacctcttcgacatcgaggatgacatcatctacactcaggacttcacggtgcccggtgagtctggcgggggcccctgcccggctctgctgactcggccaggatgtcccacgggagcagggtgcctgcc

SEQ ID NO: 440 - DNA, 241 bp, Homo sapiens
aatgtgtaaaatcacttctttttccccccctttttttttttaactgtggaaaatctaaagtcttcaagaatccttgatgaattcaagttctgtcttataaatagtactaaccttgtttcataaattagcatctgaaattaaattaggcatccaataaatatttgctgaatgaagtagactttaaaatctaaatatgttaaatagtgtttcctgtttaagactattttctattataaaatta

SEQ ID NO: 441 - DNA, 241 bp, Homo sapiens
tgccaaagtttgtgattccacatttctcttccattgtagagcaaatccatccccacaccctgttcactcctttgctgattggtttcgtaatcgtagctggcatgatgtgcattattgtgatgattctgacctacaaatatttacaggtaaccatttatttgttctctctccagagtgctctaatgactgagacaataattattaaaaggtgatctatttttccctttctccccacagaaac

SEQ ID NO: 442 - DNA, 241 bp, Homo sapiens
ccagcctgaatgatgacattcttttcggggtgttcgcacaaagcaagccagattctgccgaaccaatggatcgatctgccatgtgtgcattccctatcaaatatgtcaacgacttcttcaacaagatcgtcaacaaaaacaatgtgagatgtctccagcatttttacggacccaatcatgagcactgctttaatagggtaagtcacatcagttccccacttataaactgtgaggtataaat

SEQ ID NO: 443 - protein, 6 aa, Homo sapiens
KPLRHH

SEQ ID NO: 444 - protein, 4 aa, Homo sapiens
CRAV

SEQ ID NO: 445 - protein, 4 aa, Homo sapiens
CRAV

SEQ ID NO: 446 - protein, 6 aa, Homo sapiens
KPLRHH

SEQ ID NO: 447 - protein, 4 aa, Homo sapiens
CRAV

SEQ ID NO: 448 - protein, 4 aa, Homo sapiens
CRAV

SEQ ID NO: 449 - protein, 4 aa, Homo sapiens
QAGV

SEQ ID NO: 450 - protein, 5 aa, Homo sapiens
EKLPR

SEQ ID NO: 451 - DNA, 63 bp, Homo sapiens
ctgaaagctgtaccatacctgtctggtcttggctgaggtttcaatgaatggaatcccgtaact

SEQ ID NO: 452 - DNA, 63 bp, Homo sapiens
gtattggtctctcatggcactgtactcttcttgtccagctgtatccagtatgtccaacaaaca

SEQ ID NO: 453 - DNA, 63 bp, Homo sapiens
tagctggattgtcagtgcgcttttcccaacaccacctgctccaaccaccaccagtttgtactc

SEQ ID NO: 454 - DNA, 63 bp, Homo sapiens
ctggattgtcagtgcgcttttcccaacaccacctgctccaaccaccaccagtttgtactcagt

SEQ ID NO: 455 - DNA, 63 bp, Homo sapiens
caagaggccctagatttctatggggaagtaaggaccagagacaaaaaggtaagttattttttg

SEQ ID NO: 456 - DNA, 62 bp, Homo sapiens
tatttcagtgttacttacctgtcttgtctttgctgatgtttcaataaaaggaattccataac

SEQ ID NO: 457 - DNA, 63 bp, Homo sapiens
tgtgtctactgttctagaaggcaaatcacatttatttcctactaggaccataggtacatcttc

SEQ ID NO: 458 - DNA, 63 bp, Homo sapiens
gtactggtccctcattgcactgtactcctcttgacctgctgtgtcgagaatatccaagagaca

SEQ ID NO: 459 - DNA, 63 bp, Homo sapiens
tagctgtatcgtcaaggcactcttgcctacgccaccagctccaactaccacaagtttatattc

SEQ ID NO: 460 - DNA, 63 bp, Homo sapiens
ctgtatcgtcaaggcactcttgcctacgccaccagctccaactaccacaagtttatattcagt

SEQ ID NO: 461 - DNA, 63 bp, Homo sapiens
tctacacgagatcctctctctgaaatcactgagcaggagaaagattttctatggagtcacagg

SEQ ID NO: 462 - DNA, 63 bp, Homo sapiens
acacgagatcctctctctgaaatcactgagcaggagaaagattttctatggagtcacaggtaa

SEQ ID NO: 463 - DNA, 63 bp, Homo sapiens
gagtatttcatgaaacaaatgaatgatgcacatcatggtggctggacaacaaaaatggattgg

SEQ ID NO: 464 - DNA, 63 bp, Homo sapiens
gggacctccggtcagaaaaccaaaattataagcaacagaggtgaaaacagctgcagtaagtca

SEQ ID NO: 465 - DNA, 63 bp, Homo sapiens
aaactgatgggacccactccatcgagatttcactgtagctagaccaaaatcacctatttttac

SEQ ID NO: 466 - DNA, 63 bp, Homo sapiens
ctgcacggcgcggacgaggacgaggacctcttcgacatcgaggatgacatcatctacactcag

SEQ ID NO: 467 - DNA, 63 bp, Homo sapiens
gcgccggtctctcccaggacaggcacaaacacgcacctcaaagctgttccgtcccagtagatt

SEQ ID NO: 468 - DNA, 63 bp, Homo sapiens
atcgtagctggcatgatgtgcattattgtgatgattctgacctacaaatatttacaggtaacc

SEQ ID NO: 469 - DNA, 63 bp, Homo sapiens
ttccctatcaaatatgtcaacgacttcttcaacaagatcgtcaacaaaaacaatgtgagatgt